European Patent Application EP 4 434 997 A2, published September 25, 2024. Title: DELIVERY OF NEGATIVELY CHARGED PROTEINS USING CATIONIC LIPIDS. Applicant: President and Fellows of Harvard College. The sequence listing filed with the application follows.

SEQUENCE LISTING (280 sequences)

SEQ ID NO: 1 - protein, 240 aa, synthetic construct
  REGION 1..240: note = Synthetic Polypeptide
GGASKGERLFRGKVPILVELKGDVNGHKFSVRGKGKGDATRGKLTLKFICTTGKLPVPWPTLVTTLTYGVQCFSRYPKHMKRHDFFKSAMPKGYVQERTISFKKDGKYKTRAEVKFEGRTLVNRIKLKGRDFKEKGNILGHKLRYNFNSHKVYITADKRKNGIKAKFKIRHNVKDGSVQLADHYQQNTPIGRGPVLLPRNHYLSTRSKLSKDPKEKRDHMVLLEFVTAAGIKHGRDERYK

SEQ ID NO: 2 - protein, 18 aa, synthetic construct
  REGION 1..18: note = Synthetic Polypeptide
GGSGGSGGSGGSGGSGGS

SEQ ID NO: 3 - protein, 16 aa, synthetic construct
  REGION 1..16: note = Synthetic Polypeptide
SGSETPGTSESATPES

SEQ ID NO: 4 - protein, 12 aa, synthetic construct
  REGION 1..12: note = Synthetic Polypeptide
SGSETPGTSESA

SEQ ID NO: 5 - protein, 21 aa, synthetic construct
  REGION 1..21: note = Synthetic Polypeptide
SGSETPGTSESATPEGGSGGS

SEQ ID NO: 6 - protein, 15 aa, synthetic construct
  REGION 1..15: note = Synthetic Polypeptide
VPFLLEPDNINGKTC

SEQ ID NO: 7 - protein, 12 aa, synthetic construct
  REGION 1..12: note = Synthetic Polypeptide
GSAGSAAGSGEF

SEQ ID NO: 8 - protein, 12 aa, synthetic construct
  REGION 1..12: note = Synthetic Polypeptide
SIVAQLSRPDPA

SEQ ID NO: 9 - protein, 10 aa, synthetic construct
  REGION 1..10: note = Synthetic Polypeptide
MKIIEQLPSA

SEQ ID NO: 10 - protein, 10 aa, synthetic construct
  REGION 1..10: note = Synthetic Polypeptide
VRHKLKRVGS

SEQ ID NO: 11 - protein, 12 aa, synthetic construct
  REGION 1..12: note = Synthetic Polypeptide
GHGTGSTGSGSS

SEQ ID NO: 12 - protein, 7 aa, synthetic construct
  REGION 1..7: note = Synthetic Polypeptide
MSRPDPA

SEQ ID NO: 13 - protein, 4 aa, synthetic construct
  REGION 1..4: note = Synthetic Polypeptide
GGSM

SEQ ID NO: 14 - protein, 238 aa, Aequorea victoria
MSKGEELFTGVVPILVELDGDVNGHKFSVSGEGEGDATYGKLTLKFICTTGKLPVPWPTLVTTFSYGVQCFSRYPDHMKQHDFFKSAMPEGYVQERTIFFKDDGNYKTRAEVKFEGDTLVNRIELKGIDFKEDGNILGHKLEYNYNSHNVYIMADKQKNGIKVNFKIRHNIEDGSVQLADHYQQNTPIGDGPVLLPDNHYLSTQSALSKDPNEKRDHMVLLEFVTAAGITHGMDELYK

SEQ ID NO: 15 - protein, 248 aa, synthetic construct
  REGION 1..248: note = Synthetic Polypeptide
MGHHHHHHGGASKGERLFTGVVPILVELDGDVNGHKFSVRGEGEGDATRGKLTLKFICTTGKLPVPWPTLVTTLTYGVQCFSRYPKHMKRHDFFKSAMPEGYVQERTISFKKDGTYKTRAEVKFEGRTLVNRIELKGRDFKEKGNILGHKLEYNFNSHNVYITADKRKNGIKANFKIRHNVKDGSVQLADHYQQNTPIGRGPVLLPRNHYLSTRSALSKDPKEKRDHMVLLEFVTAAGITHGMDELYK

SEQ ID NO: 16 - protein, 248 aa, synthetic construct
  REGION 1..248: note = Synthetic Polypeptide
MGHHHHHHGGASKGERLFTGVVPILVELDGDVNGHKFSVRGKGKGDATRGKLTLKFICTTGKLPVPWPTLVTTLTYGVQCFSRYPKHMKRHDFFKSAMPKGYVQERTISFKKDGTYKTRAEVKFEGRTLVNRIKLKGRDFKEKGNILGHKLRYNFNSHNVYITADKRKNGIKANFKIRHNVKDGSVQLADHYQQNTPIGRGPVLLPRNHYLSTRSALSKDPKEKRDHMVLLEFVTAAGITHGMDELYK

SEQ ID NO: 17 - protein, 248 aa, synthetic construct
  REGION 1..248: note = Synthetic Polypeptide
MGHHHHHHGGASKGERLFRGKVPILVELKGDVNGHKFSVRGKGKGDATRGKLTLKFICTTGKLPVPWPTLVTTLTYGVQCFSRYPKHMKRHDFFKSAMPKGYVQERTISFKKDGKYKTRAEVKFEGRTLVNRIKLKGRDFKEKGNILGHKLRYNFNSHKVYITADKRKNGIKAKFKIRHNVKDGSVQLADHYQQNTPIGRGPVLLPRNHYLSTRSKLSKDPKEKRDHMVLLEFVTAAGIKHGRDERYK

SEQ ID NO: 18 - protein, 248 aa, synthetic construct
  REGION 1..248: note = Synthetic Polypeptide
MGHHHHHHGGRSKGKRLFRGKVPILVELKGDVNGHKFSVRGKGKGDATRGKLTLKFICTTGKLPVPWPTLVTTLTYGVQCFSRYPKHMKRHDFFKSAMPKGYVQERTISFKKDGKYKTRAEVKFEGRTLVNRIKLKGRDFKEKGNILGHKLRYNFNSHKVYITADKRKNGIKAKFKIRHNVKDGSVQLADHYQQNTPIGRGPVLLPRKHYLSTRSKLSKDPKEKRDHMVLLEFVTAAGIKHGRKERYK

SEQ ID NO: 19 - protein, 248 aa, synthetic construct
  REGION 1..248: note = Synthetic Polypeptide
MGHHHHHHGGRSKGKRLFRGKVPILVKLKGDVNGHKFSVRGKGKGDATRGKLTLKFICTTGKLPVPWPTLVTTLTYGVQCFSRYPKHMKRHDFFKSAMPKGYVQERTISFKKDGKYKTRAEVKFKGRTLVNRIKLKGRDFKEKGNILGHKLRYNFNSHKVYITADKRKNGIKAKFKIRHNVKDGSVQLAKHYQQNTPIGRGPVLLPRKHYLSTRSKLSKDPKEKRDHMVLLEFVTAAGIKHGRKERYK

SEQ ID NO: 20 - protein, 248 aa, synthetic construct
  REGION 1..248: note = Synthetic Polypeptide
MGHHHHHHGGRSKGKRLFRGKVPILVKLKGDVNGHKFSVRGKGKGDATRGKLTLKFICTTGKLPVPWPTLVTTLTYGVQCFSRYPKHMKRHDFFKSAMPKGYVQERTISFKKDGKYKTRAEVKFKGRTLVNRIKLKGRDFKEKGNILGHKLRYNFNSHKVYITADKRKNGIKAKFKIRHNVKDGSVQLAKHYQQNTPIGRGPVLLPRKHYLSTRSKLSKDPKEKRDHMVLKEFVTAAGIKHGRKERYK

SEQ ID NO: 21 - protein, 248 aa, synthetic construct
  REGION 1..248: note = Synthetic Polypeptide
MGHHHHHHGGASKGEELFDGVVPILVELDGDVNGHEFSVRGEGEGDATEGELTLKFICTTGELPVPWPTLVTTLTYGVQCFSDYPDHMDQHDFFKSAMPEGYVQERTISFKDDGTYKTRAEVKFEGDTLVNRIELKGIDFKEDGNILGHKLEYNFNSHDVYITADKQENGIKAEFEIRHNVEDGSVQLADHYQQNTPIGDGPVLLPDDHYLSTESALSKDPNEDRDHMVLLEFVTAAGIDHGMDELYK

SEQ ID NO: 22 - protein, 280 aa, synthetic construct
  REGION 1..280: note = Synthetic Polypeptide
MGHHHHHHGGASKGERLFRGKVPILVELKGDVNGHKFSVRGKGKGDATRGKLTLKFICTTGKLPVPWPTLVTTLTYGVQCFSRYPKHMKRHDFFKSAMPKGYVQERTISFKKDGKYKTRAEVKFEGRTLVNRIKLKGRDFKEKGNILGHKLRYNFNSHKVYITADKRKNGIKAKFKIRHNVKDGSVQLADHYQQNTPIGRGPVLLPRNHYLSTRSKLSKDPKEKRDHMVLLEFVTAAGIKHGRDERYKGSAGSAAGSGEFGLFGAIAGFIENGWEGMIDG

SEQ ID NO: 23 - protein, 26 aa, synthetic construct
  REGION 1..26: note = Synthetic Polypeptide
GIGAVLKVLTTGLPALISWIKRKRQQ

SEQ ID NO: 24 - protein, 26 aa, synthetic construct
  REGION 1..26: note = Synthetic Polypeptide
CIGAVLKVLTTGLPALISWIKRKRQQ

SEQ ID NO: 25 - protein, 16 aa, synthetic construct
  REGION 1..16: note = Synthetic Polypeptide
RQIKIWFQNRRMKWKK

SEQ ID NO: 26 - protein, 30 aa, synthetic construct
  REGION 1..30: note = Synthetic Polypeptide
MVKSKIGSWILVLFVAMWSDVGLCKKRPKP

SEQ ID NO: 27 - protein, 24 aa, synthetic construct
  REGION 1..24: note = Synthetic Polypeptide
GALFLGWLGAAGSTMGAPKSKRKV

SEQ ID NO: 28 - protein, 21 aa, synthetic construct
  REGION 1..21: note = Synthetic Polypeptide
AGYLLGKINLKALAALAKKIL

SEQ ID NO: 29 - protein, 23 aa, synthetic construct
  REGION 1..23: note = Synthetic Polypeptide
LIRLWSHLIHIWFQNRRLKWKKK

SEQ ID NO: 30 - protein, 1653 aa, synthetic construct
  REGION 1..1653: note = Synthetic Polypeptide
MGASKGERLFRGKVPILVELKGDVNGHKFSVRGKGKGDATRGKLTLKFICTTGKLPVPWPTLVTTLTSGVQCFSRYPKHMKRHDFFKSAMPKGYVQERTISFKKDGKYKTRAEVKFEGRTLVNRIKLKGRDFKEKGNILGHKLRYNFNSHKVYITADKRKNGIKAKFKIRHNVKDGSVQLADHYQQNTPIGRGPVLLPRNHYLSTRSKLSKDPKEKRDHMVLLEFVTAAGIKHGRDERYKTGGSGGSGGSGGSGGSGGSGGSGGSGGTALALPKKKRKVMDKKYSIGLDIGTNSVGWAVITDEYKVPSKKFKVLGNTDRHSIKKNLIGALLFDSGETAEATRLKRTARRRYTRRKNRICYLQEIFSNEMAKVDDSFFHRLEESFLVEEDKKHERHPIFGNIVDEVAYHEKYPTIYHLRKKLVDSTDKADLRLIYLALAHMIKFRGHFLIEGDLNPDNSDVDKLFIQLVQTYNQLFEENPINASGVDAKAILSARLSKSRRLENLIAQLPGEKKNGLFGNLIALSLGLTPNFKSNFDLAEDAKLQLSKDTYDDDLDNLLAQIGDQYADLFLAAKNLSDAILLSDILRVNTEITKAPLSASMIKRYDEHHQDLTLLKALVRQQLPEKYKEIFFDQSKNGYAGYIDGGASQEEFYKFIKPILEKMDGTEELLVKLNREDLLRKQRTFDNGSIPHQIHLGELHAILRRQEDFYPFLKDNREKIEKILTFRIPYYVGPLARGNSRFAWMTRKSEETITPWNFEEVVDKGASAQSFIERMTNFDKNLPNEKVLPKHSLLYEYFTVYNELTKVKYVTEGMRKPAFLSGEQKKAIVDLLFKTNRKVTVKQLKEDYFKKIECFDSVEISGVEDRFNASLGTYHDLLKIIKDKDFLDNEENEDILEDIVLTLTLFEDREMIEERLKTYAHLFDDKVMKQLKRRRYTGWGRLSRKLINGIRDKQSGKTILDFLKSDGFANRNFMQLIHDDSLTFKEDIQKAQVSGQGDSLHEHIANLAGSPAIKKGILQTVKVVDELVKVMGRHKPENIVIEMARENQTTQKGQKNSRERMKRIEEGIKELGSQILKEHPVENTQLQNEKLYLYYLQNGRDMYVDQELDINRLSDYDVDHIVPQSFLKDDSIDNKVLTRSDKNRGKSDNVPSEEVVKKMKNYWRQLLNAKLITQRKFDNLTKAERGGLSELDKAGFIKRQLVETRQITKHVAQILDSRMNTKYDENDKLIREVKVITLKSKLVSDFRKDFQFYKVREINNYHHAHDAYLNAVVGTALIKKYPKLESEFVYGDYKVYDVRKMIAKSEQEIGKATAKYFFYSNIMNFFKTEITLANGEIRKRPLIETNGETGEIVWDKGRDFATVRKVLSMPQVNIVKKTEVQTGGFSKESILPKRNSDKLIARKKDWDPKKYGGFDSPTVAYSVLVVAKVEKGKSKKLKSVKELLGITIMERSSFEKNPIDFLEAKGYKEVKKDLIIKLPKYSLFELENGRKRMLASAGELQKGNELALPSKYVNFLYLASHYEKLKGSPEDNEQKQLFVEQHKHYLDEIIEQISEFSKRVILADANLDKVLSAYNKHRDKPIREQAENIIHLFTLTNLGAPAAFKYFDTTIDRKRYTSTKEVLDATLIHQSITGLYETRIDLSQLGGDHHHHHH

SEQ ID NO: 31 - protein, 1653 aa, synthetic construct
  REGION 1..1653: note = Synthetic Polypeptide
MGASKGEELFDGVVPILVELDGDVNGHEFSVRGEGEGDATEGELTLKFICTTGELPVPWPTLVTTLTSGVQCFSDYPDHMDQHDFFKSAMPEGYVQERTISFKDDGTYKTRAEVKFEGDTLVNRIELKGIDFKEDGNILGHKLEYNFNSHDVYITADKQENGIKAEFEIRHNVEDGSVQLADHYQQNTPIGDGPVLLPDDHYLSTESALSKDPNEDRDHMVLLEFVTAAGIDHGMDELYKTGGSGGSGGSGGSGGSGGSGGSGGSGGTALALPKKKRKVMDKKYSIGLDIGTNSVGWAVITDEYKVPSKKFKVLGNTDRHSIKKNLIGALLFDSGETAEATRLKRTARRRYTRRKNRICYLQEIFSNEMAKVDDSFFHRLEESFLVEEDKKHERHPIFGNIVDEVAYHEKYPTIYHLRKKLVDSTDKADLRLIYLALAHMIKFRGHFLIEGDLNPDNSDVDKLFIQLVQTYNQLFEENPINASGVDAKAILSARLSKSRRLENLIAQLPGEKKNGLFGNLIALSLGLTPNFKSNFDLAEDAKLQLSKDTYDDDLDNLLAQIGDQYADLFLAAKNLSDAILLSDILRVNTEITKAPLSASMIKRYDEHHQDLTLLKALVRQQLPEKYKEIFFDQSKNGYAGYIDGGASQEEFYKFIKPILEKMDGTEELLVKLNREDLLRKQRTFDNGSIPHQIHLGELHAILRRQEDFYPFLKDNREKIEKILTFRIPYYVGPLARGNSRFAWMTRKSEETITPWNFEEVVDKGASAQSFIERMTNFDKNLPNEKVLPKHSLLYEYFTVYNELTKVKYVTEGMRKPAFLSGEQKKAIVDLLFKTNRKVTVKQLKEDYFKKIECFDSVEISGVEDRFNASLGTYHDLLKIIKDKDFLDNEENEDILEDIVLTLTLFEDREMIEERLKTYAHLFDDKVMKQLKRRRYTGWGRLSRKLINGIRDKQSGKTILDFLKSDGFANRNFMQLIHDDSLTFKEDIQKAQVSGQGDSLHEHIANLAGSPAIKKGILQTVKVVDELVKVMGRHKPENIVIEMARENQTTQKGQKNSRERMKRIEEGIKELGSQILKEHPVENTQLQNEKLYLYYLQNGRDMYVDQELDINRLSDYDVDHIVPQSFLKDDSIDNKVLTRSDKNRGKSDNVPSEEVVKKMKNYWRQLLNAKLITQRKFDNLTKAERGGLSELDKAGFIKRQLVETRQITKHVAQILDSRMNTKYDENDKLIREVKVITLKSKLVSDFRKDFQFYKVREINNYHHAHDAYLNAVVGTALIKKYPKLESEFVYGDYKVYDVRKMIAKSEQEIGKATAKYFFYSNIMNFFKTEITLANGEIRKRPLIETNGETGEIVWDKGRDFATVRKVLSMPQVNIVKKTEVQTGGFSKESILPKRNSDKLIARKKDWDPKKYGGFDSPTVAYSVLVVAKVEKGKSKKLKSVKELLGITIMERSSFEKNPIDFLEAKGYKEVKKDLIIKLPKYSLFELENGRKRMLASAGELQKGNELALPSKYVNFLYLASHYEKLKGSPEDNEQKQLFVEQHKHYLDEIIEQISEFSKRVILADANLDKVLSAYNKHRDKPIREQAENIIHLFTLTNLGAPAAFKYFDTTIDRKRYTSTKEVLDATLIHQSITGLYETRIDLSQLGGDHHHHHH

SEQ ID NO: 32 - protein, 353 aa, synthetic construct
  REGION 1..353: note = Synthetic Polypeptide
MASNLLTVHQNLPALPVDATSDEVRKNLMDMFRDRQAFSEHTWKMLLSVCRSWAAWCKLNNRKWFPAEPEDVRDYLLYLQARGLAVKTIQQHLGQLNMLHRRSGLPRPSDSNAVSLVMRRIRKENVDAGERAKQALAFERTDFDQVRSLMENSDRCQDIRNLAFLGIAYNTLLRIAEIARIRVKDISRTDGGRMLIHIGRTKTLVSTAGVEKALSLGVTKLVERWISVSGVADDPNNYLFCRVRKNGVAAPSATSQLSTRALEGIFEATHRLIYGAKDDSGQRYLAWSGHSARVGAARDMARAGVSIPEIMQAGGWTNVNIVMNYIRNLDSETGAMVRLLEDGDGGSHHHHHH

SEQ ID NO: 33 - protein, 620 aa, synthetic construct
  REGION 1..620: note = Synthetic Polypeptide
MGASKGERLFRGKVPILVELKGDVNGHKFSVRGKGKGDATRGKLTLKFICTTGKLPVPWPTLVTTLTYGVQCFSRYPKHMKRHDFFKSAMPKGYVQERTISFKKDGKYKTRAEVKFEGRTLVNRIKLKGRDFKEKGNILGHKLRYNFNSHKVYITADKRKNGIKAKFKIRHNVKDGSVQLADHYQQNTPIGRGPVLLPRNHYLSTRSKLSKDPKEKRDHMVLLEFVTAAGIKHGRDERYKTGGSGGSGGSGGSGGSGGSGGSGGSGGTASNLLTVHQNLPALPVDATSDEVRKNLMDMFRDRQAFSEHTWKMLLSVCRSWAAWCKLNNRKWFPAEPEDVRDYLLYLQARGLAVKTIQQHLGQLNMLHRRSGLPRPSDSNAVSLVMRRIRKENVDAGERAKQALAFERTDFDQVRSLMENSDRCQDIRNLAFLGIAYNTLLRIAEIARIRVKDISRTDGGRMLIHIGRTKTLVSTAGVEKALSLGVTKLVERWISVSGVADDPNNYLFCRVRKNGVAAPSATSQLSTRALEGIFEATHRLIYGAKDDSGQRYLAWSGHSARVGAARDMARAGVSIPEIMQAGGWTNVNIVMNYIRNLDSETGAMVRLLEDGDGGSHHHHHH

SEQ ID NO: 34 - protein, 620 aa, synthetic construct
  REGION 1..620: note = Synthetic Polypeptide
MGASKGEELFDGVVPILVELDGDVNGHEFSVRGEGEGDATEGELTLKFICTTGELPVPWPTLVTTLTYGVQCFSDYPDHMDQHDFFKSAMPEGYVQERTISFKDDGTYKTRAEVKFEGDTLVNRIELKGIDFKEDGNILGHKLEYNFNSHDVYITADKQENGIKAEFEIRHNVEDGSVQLADHYQQNTPIGDGPVLLPDDHYLSTESALSKDPNEDRDHMVLLEFVTAAGIDHGMDELYKTGGSGGSGGSGGSGGSGGSGGSGGSGGTASNLLTVHQNLPALPVDATSDEVRKNLMDMFRDRQAFSEHTWKMLLSVCRSWAAWCKLNNRKWFPAEPEDVRDYLLYLQARGLAVKTIQQHLGQLNMLHRRSGLPRPSDSNAVSLVMRRIRKENVDAGERAKQALAFERTDFDQVRSLMENSDRCQDIRNLAFLGIAYNTLLRIAEIARIRVKDISRTDGGRMLIHIGRTKTLVSTAGVEKALSLGVTKLVERWISVSGVADDPNNYLFCRVRKNGVAAPSATSQLSTRALEGIFEATHRLIYGAKDDSGQRYLAWSGHSARVGAARDMARAGVSIPEIMQAGGWTNVNIVMNYIRNLDSETGAMVRLLEDGDGGSHHHHHH

SEQ ID NO: 35 - protein, 53 aa, synthetic construct
  REGION 1..53: note = Synthetic Polypeptide
GRADALDDFDLDMLGSDALDDFDLDMLGSDALDDFDLDMLGSDALDDFDLDML

SEQ ID NO: 36 - protein, 1210 aa, synthetic construct
  REGION 1..1210: note = Synthetic Polypeptide
MGASKGERLFRGKVPILVELKGDVNGHKFSVRGKGKGDATRGKLTLKFICTTGKLPVPWPTLVTTLTYGVQCFSRYPKHMKRHDFFKSAMPKGYVQERTISFKKDGKYKTRAEVKFEGRTLVNRIKLKGRDFKEKGNILGHKLRYNFNSHKVYITADKRKNGIKAKFKIRHNVKDGSVQLADHYQQNTPIGRGPVLLPRNHYLSTRSKLSKDPKEKRDHMVLLEFVTAAGIKHGRDERYKTGGSGGSGGSGGSGGSGGSGGSGGSGGTAPKKKRKVGIHRGVPMVDLRTLGYSQQQQEKIKPKVRSTVAQHHEALVGHGFTHAHIVALSQHPAALGTVAVKYQDMIAALPEATHEAIVGVGKQWSGARALEALLTVAGELRGPPLQLDTGQLLKIAKRGGVTAVEAVHAWRNALTGAPLNLTPDQVVAIASNIGGKQALETVQRLLPVLCQDHGLTPEQVVAIASNIGGKQALETVQRLLPVLCQAHGLTPDQVVAIASNGGGKQALETVQRLLPVLCQAHGLTPAQVVAIANNNGGKQALETVQRLLPVLCQDHGLTPDQVVAIASNGGGKQALETVQRLLPVLCQDHGLTPEQVVAIASNIGGKQALETVQRLLPVLCQAHGLTPDQVVAIASHDGGKQALETVQRLLPVLCQAHGLTPAQVVAIASHDGGKQALETVQRLLPVLCQDHGLTPDQVVAIASNIGGKQALETVQRLLPVLCQDHGLTPEQVVAIASNIGGKQALETVQRLLPVLCQAHGLTPDQVVAIANNNGGKQALETVQRLLPVLCQAHGLTPAQVVAIASNGGGKQALETVQRLLPVLCQDHGLTPDQVVAIASHDGGKQALETVQRLLPVLCQDHGLTPEQVVAIASNGGGKQALETVQRLLPVLCQAHGLTPDQVVAIASNGGGKQALETVQRLLPVLCQAHGLTPAQVVAIANNNGGKQALETVQRLLPVLCQDHGLTPDQVVAIASHDGGKQALETVQRLLPVLCQDHGLTPEQVVAIASHDGGKQALETVQRLLPVLCQAHGLTPEQVVAIASNIGGRPALESIVAQLSRPDPALAALTNDHLVALACLGGRPALDAVKKGLPHAPALIKRTNRRIPERTSHRVADHAQVVRVLGFFQCHSHPAQAFDDAMTQFGMSGGGSGRADALDDFDLDMLGSDALDDFDLDMLGSDALDDFDLDMLGSDALDDFDLDMLHHHHHH

SEQ ID NO: 37 - protein, 1210 aa, synthetic construct
  REGION 1..1210: note = Synthetic Polypeptide
MGASKGERLFRGKVPILVELKGDVNGHKFSVRGKGKGDATRGKLTLKFICTTGKLPVPWPTLVTTLTYGVQCFSRYPKHMKRHDFFKSAMPKGYVQERTISFKKDGKYKTRAEVKFEGRTLVNRIKLKGRDFKEKGNILGHKLRYNFNSHKVYITADKRKNGIKAKFKIRHNVKDGSVQLADHYQQNTPIGRGPVLLPRNHYLSTRSKLSKDPKEKRDHMVLLEFVTAAGIKHGRDERYKTGGSGGSGGSGGSGGSGGSGGSGGSGGTAPKKKRKVGIHRGVPMVDLRTLGYSQQQQEKIKPKVRSTVAQHHEALVGHGFTHAHIVALSQHPAALGTVAVKYQDMIAALPEATHEAIVGVGKQWSGARALEALLTVAGELRGPPLQLDTGQLLKIAKRGGVTAVEAVHAWRNALTGAPLNLTPDQVVAIASNGGGKQALETVQRLLPVLCQDHGLTPEQVVAIANNNGGKQALETVQRLLPVLCQAHGLTPDQVVAIANNNGGKQALETVQRLLPVLCQAHGLTPAQVVAIASHDGGKQALETVQRLLPVLCQDHGLTPDQVVAIASHDGGKQALETVQRLLPVLCQDHGLTPEQVVAIASHDGGKQALETVQRLLPVLCQAHGLTPDQVVAIASHDGGKQALETVQRLLPVLCQAHGLTPAQVVAIANNNGGKQALETVQRLLPVLCQDHGLTPDQVVAIANNNGGKQALETVQRLLPVLCQDHGLTPEQVVAIASHDGGKQALETVQRLLPVLCQAHGLTPDQVVAIANNNGGKQALETVQRLLPVLCQAHGLTPAQVVAIASNIGGKQALETVQRLLPVLCQDHGLTPDQVVAIANNNGGKQALETVQRLLPVLCQDHGLTPEQVVAIANNNGGKQALETVQRLLPVLCQAHGLTPDQVVAIANNNGGKQALETVQRLLPVLCQAHGLTPAQVVAIANNNGGKQALETVQRLLPVLCQDHGLTPDQVVAIASNGGGKQALETVQRLLPVLCQDHGLTPEQVVAIANNNGGKQALETVQRLLPVLCQAHGLTPEQVVAIASNGGGRPALESIVAQLSRPDPALAALTNDHLVALACLGGRPALDAVKKGLPHAPALIKRTNRRIPERTSHRVADHAQVVRVLGFFQCHSHPAQAFDDAMTQFGMSGGGSGRADALDDFDLDMLGSDALDDFDLDMLGSDALDDFDLDMLGSDALDDFDLDMLHHHHHH

SEQ ID NO: 38 - protein, 1182 aa, synthetic construct
  REGION 1..1182: note = Synthetic Polypeptide
MGASKGEELFDGVVPILVELDGDVNGHEFSVRGEGEGDATEGELTLKFICTTGELPVPWPTLVTTLTYGVQCFSDYPDHMDQHDFFKSAMPEGYVQERTISFKDDGTYKTRAEVKFEGDTLVNRIELKGIDFKEDGNILGHKLEYNFNSHDVYITADKQENGIKAEFEIRHNVEDGSVQLADHYQQNTPIGDGPVLLPDDHYLSTESALSKDPNEDRDHMVLLEFVTAAGIDHGMDELYKAPKKKRKVGIHRGVPMVDLRTLGYSQQQQEKIKPKVRSTVAQHHEALVGHGFTHAHIVALSQHPAALGTVAVKYQDMIAALPEATHEAIVGVGKQWSGARALEALLTVAGELRGPPLQLDTGQLLKIAKRGGVTAVEAVHAWRNALTGAPLNLTPDQVVAIASNIGGKQALETVQRLLPVLCQDHGLTPEQVVAIASNIGGKQALETVQRLLPVLCQAHGLTPDQVVAIASNGGGKQALETVQRLLPVLCQAHGLTPAQVVAIANNNGGKQALETVQRLLPVLCQDHGLTPDQVVAIASNGGGKQALETVQRLLPVLCQDHGLTPEQVVAIASNIGGKQALETVQRLLPVLCQAHGLTPDQVVAIASHDGGKQALETVQRLLPVLCQAHGLTPAQVVAIASHDGGKQALETVQRLLPVLCQDHGLTPDQVVAIASNIGGKQALETVQRLLPVLCQDHGLTPEQVVAIASNIGGKQALETVQRLLPVLCQAHGLTPDQVVAIANNNGGKQALETVQRLLPVLCQAHGLTPAQVVAIASNGGGKQALETVQRLLPVLCQDHGLTPDQVVAIASHDGGKQALETVQRLLPVLCQDHGLTPEQVVAIASNGGGKQALETVQRLLPVLCQAHGLTPDQVVAIASNGGGKQALETVQRLLPVLCQAHGLTPAQVVAIANNNGGKQALETVQRLLPVLCQDHGLTPDQVVAIASHDGGKQALETVQRLLPVLCQDHGLTPEQVVAIASHDGGKQALETVQRLLPVLCQAHGLTPEQVVAIASNIGGRPALESIVAQLSRPDPALAALTNDHLVALACLGGRPALDAVKKGLPHAPALIKRTNRRIPERTSHRVADHAQVVRVLGFFQCHSHPAQAFDDAMTQFGMSGGGSGRADALDDFDLDMLGSDALDDFDLDMLGSDALDDFDLDMLGSDALDDFDLDMLHHHHHH

SEQ ID NO: 39 - protein, 1182 aa, synthetic construct
  REGION 1..1182: note = Synthetic Polypeptide
MGASKGEELFDGVVPILVELDGDVNGHEFSVRGEGEGDATEGELTLKFICTTGELPVPWPTLVTTLTYGVQCFSDYPDHMDQHDFFKSAMPEGYVQERTISFKDDGTYKTRAEVKFEGDTLVNRIELKGIDFKEDGNILGHKLEYNFNSHDVYITADKQENGIKAEFEIRHNVEDGSVQLADHYQQNTPIGDGPVLLPDDHYLSTESALSKDPNEDRDHMVLLEFVTAAGIDHGMDELYKAPKKKRKVGIHRGVPMVDLRTLGYSQQQQEKIKPKVRSTVAQHHEALVGHGFTHAHIVALSQHPAALGTVAVKYQDMIAALPEATHEAIVGVGKQWSGARALEALLTVAGELRGPPLQLDTGQLLKIAKRGGVTAVEAVHAWRNALTGAPLNLTPDQVVAIASNGGGKQALETVQRLLPVLCQDHGLTPEQVVAIANNNGGKQALETVQRLLPVLCQAHGLTPDQVVAIANNNGGKQALETVQRLLPVLCQAHGLTPAQVVAIASHDGGKQALETVQRLLPVLCQDHGLTPDQVVAIASHDGGKQALETVQRLLPVLCQDHGLTPEQVVAIASHDGGKQALETVQRLLPVLCQAHGLTPDQVVAIASHDGGKQALETVQRLLPVLCQAHGLTPAQVVAIANNNGGKQALETVQRLLPVLCQDHGLTPDQVVAIANNNGGKQALETVQRLLPVLCQDHGLTPEQVVAIASHDGGKQALETVQRLLPVLCQAHGLTPDQVVAIANNNGGKQALETVQRLLPVLCQAHGLTPAQVVAIASNIGGKQALETVQRLLPVLCQDHGLTPDQVVAIANNNGGKQALETVQRLLPVLCQDHGLTPEQVVAIANNNGGKQALETVQRLLPVLCQAHGLTPDQVVAIANNNGGKQALETVQRLLPVLCQAHGLTPAQVVAIANNNGGKQALETVQRLLPVLCQDHGLTPDQVVAIASNGGGKQALETVQRLLPVLCQDHGLTPEQVVAIANNNGGKQALETVQRLLPVLCQAHGLTPEQVVAIASNGGGRPALESIVAQLSRPDPALAALTNDHLVALACLGGRPALDAVKKGLPHAPALIKRTNRRIPERTSHRVADHAQVVRVLGFFQCHSHPAQAFDDAMTQFGMSGGGSGRADALDDFDLDMLGSDALDDFDLDMLGSDALDDFDLDMLGSDALDDFDLDMLHHHHHH

SEQ ID NO: 40 - protein, 240 aa, synthetic construct
  REGION 1..240: note = Synthetic Polypeptide
MGASKGEELFDGVVPILVELDGDVNGHEFSVRGEGEGDATEGELTLKFICTTGELPVPWPTLVTTLTYGVQCFSDYPDHMDQHDFFKSAMPEGYVQERTISFKDDGTYKTRAEVKFEGDTLVNRIELKGIDFKEDGNILGHKLEYNFNSHDVYITADKQENGIKAEFEIRHNVEDGSVQLADHYQQNTPIGDGPVLLPDDHYLSTESALSKDPNEDRDHMVLLEFVTAAGIDHGMDELYK

SEQ ID NO: 41 - protein, 153 aa, synthetic construct
  REGION 1..153: note = Synthetic Polypeptide
APKKKRKVGIHRGVPMVDLRTLGYSQQQQEKIKPKVRSTVAQHHEALVGHGFTHAHIVALSQHPAALGTVAVKYQDMIAALPEATHEAIVGVGKQWSGARALEALLTVAGELRGPPLQLDTGQLLKIAKRGGVTAVEAVHAWRNALTGAPLNL

SEQ ID NO: 42 - protein, 101 aa, synthetic construct
  REGION 1..101: note = Synthetic Polypeptide
LESIVAQLSRPDPALAALTNDHLVALACLGGRPALDAVKKGLPHAPALIKRTNRRIPERTSHRVADHAQVVRVLGFFQCHSHPAQAFDDAMTQFGMSGGGS

SEQ ID NO: 43 - DNA, 4104 bp, Streptococcus pyogenes
  source 1..4104: mol_type = genomic DNA
atggataagaaatactcaataggcttagatatcggcacaaatagcgtcggatgggcggtgatcactgatgattataaggttccgtctaaaaagttcaaggttctgggaaatacagaccgccacagtatcaaaaaaaatcttataggggctcttttatttggcagtggagagacagcggaagcgactcgtctcaaacggacagctcgtagaaggtatacacgtcggaagaatcgtatttgttatctacaggagattttttcaaatgagatggcgaaagtagatgatagtttctttcatcgacttgaagagtcttttttggtggaagaagacaagaagcatgaacgtcatcctatttttggaaatatagtagatgaagttgcttatcatgagaaatatccaactatctatcatctgcgaaaaaaattggcagattctactgataaagcggatttgcgcttaatctatttggccttagcgcatatgattaagtttcgtggtcattttttgattgagggagatttaaatcctgataatagtgatgtggacaaactatttatccagttggtacaaatctacaatcaattatttgaagaaaaccctattaacgcaagtagagtagatgctaaagcgattctttctgcacgattgagtaaatcaagacgattagaaaatctcattgctcagctccccggtgagaagagaaatggcttgtttgggaatctcattgctttgtcattgggattgacccctaattttaaatcaaattttgatttggcagaagatgctaaattacagctttcaaaagatacttacgatgatgatttagataatttattggcgcaaattggagatcaatatgctgatttgtttttggcagctaagaatttatcagatgctattttactttcagatatcctaagagtaaatagtgaaataactaaggctcccctatcagcttcaatgattaagcgctacgatgaacatcatcaagacttgactcttttaaaagctttagttcgacaacaacttccagaaaagtataaagaaatcttttttgatcaatcaaaaaacggatatgcaggttatattgatgggggagctagccaagaagaattttataaatttatcaaaccaattttagaaaaaatggatggtactgaggaattattggtgaaactaaatcgtgaagatttgctgcgcaagcaacggacctttgacaacggctctattccccatcaaattcacttgggtgagctgcatgctattttgagaagacaagaagacttttatccatttttaaaagacaatcgtgagaagattgaaaaaatcttgacttttcgaattccttattatgttggtccattggcgcgtggcaatagtcgttttgcatggatgactcggaagtctgaagaaacaattaccccatggaattttgaagaagttgtcgataaaggtgcttcagctcaatcatttattgaacgcatgacaaactttgataaaaatcttccaaatgaaaaagtactaccaaaacatagtttgctttatgagtattttacggtttataacgaattgacaaaggtcaaatatgttactgagggaatgcgaaaaccagcatttctttcaggtgaacagaagaaagccattgttgatttactcttcaaaacaaatcgaaaagtaaccgttaagcaattaaaagaagattatttcaaaaaaatagaatgttttgatagtgttgaaatttcaggagttgaagatagatttaatgcttcattaggcgcctaccatgatttgctaaaaattattaaagataaagattttttggataatgaagaaaatgaagatatcttagaggatattgttttaacattgaccttatttgaagatagggggatgattgaggaaagacttaaaacatatgctcacctctttgatgataaggtgatgaaacagcttaaacgtcgccgttatactggttggggacgtttgtctcgaaaattgattaatggtattagggataagcaatctggcaaaacaatattagattttttgaaatcagatggttttgccaatcgcaattttatgcagctgatccatgatgatagtttgacatttaaagaagatattcaaaaagcacaggtgtctggacaaggccatagtttacatgaacagattgctaacttagctggcagtcctgctattaaaaaaggtattttacagactgtaaaaattgttgatgaactggtcaaagtaatggggcataagccagaaaatatcgttattgaaatggcacgtgaaaatcagacaactcaaaagggccagaaaaattcgcgagagcgtatgaaacgaatcgaagaaggtatcaaagaattaggaagtcagattcttaaagagcatcctgttgaaaatactcaattgcaaaatgaaaagctctatctctattatctacaaaatggaagagacatgtatgtggaccaagaattagatattaatcgtttaagtgattatgatgtcgatcacattgttccacaaagtttcattaaagacgattcaatagacaataaggtactaacgcgttctgataaaaatcgtggtaaatcggataacgttccaagtgaagaagtagtcaaaaagatgaaaaactattggagacaacttctaaacgccaagttaatcactcaacgtaagtttgataatttaacgaaagctgaacgtggaggtttgagtgaacttgataaagctggttttatcaaacgccaattggttgaaactcgccaaatcactaagcatgtggcacaaattttggatagtcgcatgaatactaaatacgatgaaaatgataaacttattcgagaggttaaagtgattaccttaaaatctaaattagtttctgacttccgaaaagatttccaattctataaagtacgtgagattaacaattaccatcatgcccatgatgcgtatctaaatgccgtcgttggaactgctttgattaagaaatatccaaaacttgaatcggagtttgtctatggtgattataaagtttatgatgttcgtaaaatgattgctaagtctgagcaagaaataggcaaagcaaccgcaaaatatttcttttactctaatatcatgaacttcttcaaaacagaaattacacttgcaaatggagagattcgcaaacgccctctaatcgaaactaatggggaaactggagaaattgtctgggataaagggcgagattttgccacagtgcgcaaagtattgtccatgccccaagtcaatattgtcaagaaaacagaagtacagacaggcggattctccaaggagtcaattttaccaaaaagaaattcggacaagcttattgctcgtaaaaaagactgggatccaaaaaaatatggtggttttgatagtccaacggtagcttattcagtcctagtggttgctaaggtggaaaaagggaaatcgaagaagttaaaatccgttaaagagttactagggatcacaattatggaaagaagttcctttgaaaaaaatccgattgactttttagaagctaaaggatataaggaagttaaaaaagacttaatcattaaactacctaaatatagtctttttgagttagaaaacggtcgtaaacggatgctggctagtgccggagaattacaaaaaggaaatgagctggctctgccaagcaaatatgtgaattttttatatttagctagtcattatgaaaagttgaagggtagtccagaagataacgaacaaaaacaattgtttgtggagcagcataagcattatttagatgagattattgagcaaatcagtgaattttctaagcgtgttattttagcagatgccaatttagataaagttcttagtgcatataacaaacatagagacaaaccaatacgtgaacaagcagaaaatattattcatttatttacgttgacgaatcttggagctcccgctgcttttaaatattttgatacaacaattgatcgtaaacgatatacgtctacaaaagaagttttagatgccactcttatccatcaatccatcactggtctttatgaaacacgcattgatttgagtcagctaggaggtgactga

SEQ ID NO: 44 - protein, 1368 aa, Streptococcus pyogenes
MDKKYSIGLAIGTNSVGWAVITDEYKVPSKKFKVLGNTDRHSIKKNLIGALLFDSGETAEATRLKRTARRRYTRRKNRICYLQEIFSNEMAKVDDSFFHRLEESFLVEEDKKHERHPIFGNIVDEVAYHEKYPTIYHLRKKLVDSTDKADLRLIYLALAHMIKFRGHFLIEGDLNPDNSDVDKLFIQLVQTYNQLFEENPINASGVDAKAILSARLSKSRRLENLIAQLPGEKKNGLFGNLIALSLGLTPNFKSNFDLAEDAKLQLSKDTYDDDLDNLLAQIGDQYADLFLAAKNLSDAILLSDILRVNTEITKAPLSASMIKRYDEHHQDLTLLKALVRQQLPEKYKEIFFDQSKNGYAGYIDGGASQEEFYKFIKPILEKMDGTEELLVKLNREDLLRKQRTFDNGSIPHQIHLGELHAILRRQEDFYPFLKDNREKIEKILTFRIPYYVGPLARGNSRFAWMTRKSEETITPWNFEEVVDKGASAQSFIERMTNFDKNLPNEKVLPKHSLLYEYFTVYNELTKVKYVTEGMRKPAFLSGEQKKAIVDLLFKTNRKVTVKQLKEDYFKKIECFDSVEISGVEDRFNASLGTYHDLLKIIKDKDFLDNEENEDILEDIVLTLTLFEDREMIEERLKTYAHLFDDKVMKQLKRRRYTGWGRLSRKLINGIRDKQSGKTILDFLKSDGFANRNFMQLIHDDSLTFKEDIQKAQVSGQGDSLHEHIANLAGSPAIKKGILQTVKVVDELVKVMGRHKPENIVIEMARENQTTQKGQKNSRERMKRIEEGIKELGSQILKEHPVENTQLQNEKLYLYYLQNGRDMYVDQELDINRLSDYDVDHIVPQSFLKDDSIDNKVLTRSDKNRGKSDNVPSEEVVKKMKNYWRQLLNAKLITQRKFDNLTKAERGGLSELDKAGFIKRQLVETRQITKHVAQILDSRMNTKYDENDKLIREVKVITLKSKLVSDFRKDFQFYKVREINNYHHAHDAYLNAVVGTALIKKYPKLESEFVYGDYKVYDVRKMIAKSEQEIGKATAKYFFYSNIMNFFKTEITLANGEIRKRPLIETNGETGEIVWDKGRDFATVRKVLSMPQVNIVKKTEVQTGGFSKESILPKRNSDKLIARKKDWDPKKYGGFDSPTVAYSVLVVAKVEKGKSKKLKSVKELLGITIMERSSFEKNPIDFLEAKGYKEVKKDLIIKLPKYSLFELENGRKRMLASAGELQKGNELALPSKYVNFLYLASHYEKLKGSPEDNEQKQLFVEQHKHYLDEIIEQISEFSKRVILADANLDKVLSAYNKHRDKPIREQAENIIHLFTLTNLGAPAAFKYFDTTIDRKRYTSTKEVLDATLIHQSITGLYETRIDLSQLGGD

SEQ ID NO: 45 - protein, 1368 aa, synthetic construct
  REGION 1..1368: note = Synthetic Polypeptide
MDKKYSIGLAIGTNSVGWAVITDEYKVPSKKFKVLGNTDRHSIKKNLIGALLFDSGETAEATRLKRTARRRYTRRKNRICYLQEIFSNEMAKVDDSFFHRLEESFLVEEDKKHERHPIFGNIVDEVAYHEKYPTIYHLRKKLVDSTDKADLRLIYLALAHMIKFRGHFLIEGDLNPDNSDVDKLFIQLVQTYNQLFEENPINASGVDAKAILSARLSKSRRLENLIAQLPGEKKNGLFGNLIALSLGLTPNFKSNFDLAEDAKLQLSKDTYDDDLDNLLAQIGDQYADLFLAAKNLSDAILLSDILRVNTEITKAPLSASMIKRYDEHHQDLTLLKALVRQQLPEKYKEIFFDQSKNGYAGYIDGGASQEEFYKFIKPILEKMDGTEELLVKLNREDLLRKQRTFDNGSIPHQIHLGELHAILRRQEDFYPFLKDNREKIEKILTFRIPYYVGPLARGNSRFAWMTRKSEETITPWNFEEVVDKGASAQSFIERMTNFDKNLPNEKVLPKHSLLYEYFTVYNELTKVKYVTEGMRKPAFLSGEQKKAIVDLLFKTNRKVTVKQLKEDYFKKIECFDSVEISGVEDRFNASLGTYHDLLKIIKDKDFLDNEENEDILEDIVLTLTLFEDREMIEERLKTYAHLFDDKVMKQLKRRRYTGWGRLSRKLINGIRDKQSGKTILDFLKSDGFANRNFMQLIHDDSLTFKEDIQKAQVSGQGDSLHEHIANLAGSPAIKKGILQTVKVVDELVKVMGRHKPENIVIEMARENQTTQKGQKNSRERMKRIEEGIKELGSQILKEHPVENTQLQNEKLYLYYLQNGRDMYVDQELDINRLSDYDVDAIVPQSFLKDDSIDNKVLTRSDKNRGKSDNVPSEEVVKKMKNYWRQLLNAKLITQRKFDNLTKAERGGLSELDKAGFIKRQLVETRQITKHVAQILDSRMNTKYDENDKLIREVKVITLKSKLVSDFRKDFQFYKVREINNYHHAHDAYLNAVVGTALIKKYPKLESEFVYGDYKVYDVRKMIAKSEQEIGKATAKYFFYSNIMNFFKTEITLANGEIRKRPLIETNGETGEIVWDKGRDFATVRKVLSMPQVNIVKKTEVQTGGFSKESILPKRNSDKLIARKKDWDPKKYGGFDSPTVAYSVLVVAKVEKGKSKKLKSVKELLGITIMERSSFEKNPIDFLEAKGYKEVKKDLIIKLPKYSLFELENGRKRMLASAGELQKGNELALPSKYVNFLYLASHYEKLKGSPEDNEQKQLFVEQHKHYLDEIIEQISEFSKRVILADANLDKVLSAYNKHRDKPIREQAENIIHLFTLTNLGAPAAFKYFDTTIDRKRYTSTKEVLDATLIHQSITGLYETRIDLSQLGGD

SEQ ID NO: 46 - protein, 1368 aa, synthetic construct; identical to SEQ ID NO: 44
  REGION 1..1368: note = Synthetic Polypeptide

SEQ ID NO: 47 - protein, 16 aa, synthetic construct
  REGION 1..16: note = Synthetic Polypeptide
MAPKKKRKVGIHRGVP

SEQ ID NO: 48 - protein, 23 aa, synthetic construct
  REGION 1..23: note = Synthetic Polypeptide
MDYKDHDGDYKDHDIDYKDDDDK

SEQ ID NO: 49 - protein, 198 aa, synthetic construct
  REGION 1..198: note = Synthetic Polypeptide
GSQLVKSELEEKKSELRHKLKYVPHEYIELIEIARNSTQDRILEMKVMEFFMKVYGYRGKHLGGSRKPDGAIYTVGSPIDYGVIVDTKAYSGGYNLPIGQADEMQRYVEENQTRNKHINPNEWWKVYPSSVTEFKFLFVSGHFKGNYKAQLTRLNHITNCNGAVLSVEELLIGGEMIKAGTLTLEEVRRKFNNGEINF

SEQ ID NO: 50 - DNA, 4836 bp, synthetic construct
  misc_feature 1..4836: note = Synthetic Polynucleotide
  source 1..4836: mol_type = other DNA
atggataaaaagtattctattggtttagctatcggcactaattccgttggatgggctgtcataaccgatgaatacaaagtaccttcaaagaaatttaaggtgttggggaacacagaccgtcattcgattaaaaagaatcttatcggtgccctcctattcgatagtggcgaaacggcagaggcgactcgcctgaaacgaaccgctcggagaaggtatacacgtcgcaagaaccgaatatgttacttacaagaaatttttagcaatgagatggccaaagttgacgattctttctttcaccgtttggaagagtccttccttgtcgaagaggacaagaaacatgaacggcaccccatctttggaaacatagtagatgaggtggcatatcatgaaaagtacccaacgatttatcacctcagaaaaaagctagttgactcaactgataaagcggacctgaggttaatctacttggctcttgcccatatgataaagttccgtgggcactttctcattgagggtgatctaaatccggacaactcggatgtcgacaaactgttcatccagttagtacaaacctataatcagttgtttgaagagaaccctataaatgcaagtggcgtggatgcgaaggctattcttagcgcccgcctctctaaatcccgacggctagaaaacctgatcgcacaattacccggagagaagaaaaatgggttgttcggtaaccttatagcgctctcactaggcctgacaccaaattttaagtcgaacttcgacttagctgaagatgccaaattgcagcttagtaaggacacgtacgatgacgatctcgacaatctactggcacaaattggagatcagtatgcggacttatttttggctgccaaaaaccttagcgatgcaatcctcctatctgacatactgagagttaatactgagattaccaaggcgccgttatccgcttcaatgatcaaaaggtacgatgaacatcaccaagacttgacacttctcaaggccctagtccgtcagcaactgcctgagaaatataaggaaatattctttgatcagtcgaaaaacgggtacgcaggttatattgacggcggagcgagtcaagaggaattctacaagtttatcaaacccatattagagaagatggatgggacggaagagttgcttgtaaaactcaatcgcgaagatctactgcgaaagcagcggactttcgacaacggtagcattccacatcaaatccacttaggcgaattgcatgctatacttagaaggcaggaggatttttatccgttcctcaaagacaatcgtgaaaagattgagaaaatcctaacctttcgcataccttactatgtgggacccctggcccgagggaactctcggttcgcatggatgacaagaaagtccgaagaaacgattactccatggaattttgaggaagttgtcgataaaggtgcgtcagctcaatcgttcatcgagaggatgaccaactttgacaagaatttaccgaacgaaaaagtattgcctaagcacagtttactttacgagtatttcacagtgtacaatgaactcacgaaagttaagtatgtcactgagggcatgcgtaaacccgcctttctaagcggagaacagaagaaagcaatagtagatctgttattcaagaccaaccgcaaagtgacagttaagcaattgaaagaggactactttaagaaaattgaatgcttcgattctgtcgagatctccggggtagaagatcgatttaatgcgtcacttggtacgtatcatgacctcctaaagataattaaagataaggacttcctggataacgaagagaatgaagatatcttagaagatatagtgttgactcttaccctctttgaagatcgggaaatgattgaggaaagactaaaaacatacgctcacctgttcgacgataaggttatgaaacagttaaagaggcgtcgctatacgggctggggacgattgtcgcggaaacttatcaacgggataagagacaagcaaagtggtaaaactattctcgattttctaaagagcgacggcttcgccaataggaactttatgcagctgatccatgatgactctttaaccttcaaagaggatatacaaaaggcacaggtttccggacaaggggactcattgcacgaacatattgcgaatcttgctggttcgccagccatcaaaaagggcatactccagacagtcaaagtagtggatgagctagttaaggtcatgggacgtcacaaaccggaaaacattgtaatcgagatggcacgcgaaaatcaaacgactcagaaggggcaaaaaaacagtcgagagcggatgaagagaatagaagagggtattaaagaactgggcagccagatcttaaaggagcatcctgtggaaaatacccaattgcagaacgagaaactttacctctattacctacaaaatggaagggacatgtatgttgatcaggaactggacataaaccgtttatctgattacgacgtcgatgccattgtaccccaatcctttttgaaggacgattcaatcgacaataaagtgcttacacgctcggataagaaccgagggaaaagtgacaatgttccaagcgaggaagtcgtaaagaaaatgaagaactattggcggcagctcctaaatgcgaaactgataacgcaaagaaagttcgataacttaactaaagctgagaggggtggcttgtctgaacttgacaaggccggatttattaaacgtcagctcgtggaaacccgccaaatcacaaagcatgttgcacagatactagattcccgaatgaatacgaaatacgacgagaacgataagctgattcgggaagtcaaagtaatcactttaaagtcaaaattggtgtcggacttcagaaaggattttcaattctataaagttagggagataaataactaccaccatgcgcacgacgcttatcttaatgccgtcgtagggaccgcactcattaagaaatacccgaagctagaaagtgagtttgtgtatggtgattacaaagtttatgacgtccgtaagatgatcgcgaaaagcgaacaggagataggcaaggctacagccaaatacttcttttattctaacattatgaatttctttaagacggaaatcactctggcaaacggagagatacgcaaacgacctttaattgaaaccaatggggagacaggtgaaatcgtatgggataagggccgggacttcgcgacggtgagaaaagttttgtccatgccccaagtcaacatagtaaagaaaactgaggtgcagaccggagggttttcaaaggaatcgattcttccaaaaaggaatagtgataagctcatcgctcgtaaaaaggactgggacccgaaaaagtacggtggcttcgatagccctacagttgcctattctgtcctagtagtggcaaaagttgagaagggaaaatccaagaaactgaagtcagtcaaagaattattggggataacgattatggagcgctcgtcttttgaaaagaaccccatcgacttccttgaggcgaaaggttacaaggaagtaaaaaaggatctcataattaaactaccaaagtatagtctgtttgagttagaaaatggccgaaaacggatgttggctagcgccggagagcttcaaaaggggaacgaactcgcactaccgtctaaatacgtgaatttcctgtatttagcgtcccattacgagaagttgaaaggttcacctgaagataacgaacagaagcaactttttgttgagcagcacaaacattatctcgacgaaatcatagagcaaatttcggaattcagtaagagagtcatcctagctgatgccaatctggacaaagtattaagcgcatacaacaagcacagggataaacccatacgtgagcaggcggaaaatattatccatttgtttactcttaccaacctcggcgctccagccgcattcaagtattttgacacaacgatagatcgcaaacgatacacttctaccaaggaggtgctagacgcgacactgattcaccaatccatcacgggattatatgaaactcggatagatttgtcacagcttgggggtgacggatcccccaagaagaagaggaaagtctcgagcgactacaaagaccatgacggtgattataaagatcatgacatcgattacaaggatgacgatgacaaggctgcaggatcaggtggaagtggcggcagcggaggttctggatcccaactagtcaaaagtgaactggaggagaagaaatctgaacttcgtcataaattgaaatatgtgcctcatgaatatattgaattaattgaaattgccagaaattccactcaggatagaattcttgaaatgaaggtaatggaattttttatgaaagtttatggatatagaggtaaacatttgggtggatcaaggaaaccggacggagcaatttatactgtcggatctcctattgattacggtgtgatcgtggatactaaagcttatagcggaggttataatctgccaattggccaagcagatgaaatgcaacgatatgtcgaagaaaatcaaacacgaaacaaacatatcaaccctaatgaatggtggaaagtctatccatcttctgtaacggaatttaagtttttatttgtgagtggtcactttaaaggaaactacaaagctcagcttacacgattaaatcatatcactaattgtaatggagctgttcttagtgtagaagagcttttaattggtggagaaatgattaaagccggcacattaaccttagaggaagtcagacggaaatttaataacggcgagataaacttt

SEQ ID NO: 51 - DNA, 4845 bp, synthetic construct
  misc_feature 1..4845: note = Synthetic Polynucleotide
  source 1..4845: mol_type = other DNA
atggactacaaagaccatgacggtgattataaagatcatgacatcgattacaaggatgacgatgacaagatggcccccaagaagaagaggaaggtgggcattcaccgcggggtacctatggataaaaagtattctattggtttagctatcggcactaattccgttggatgggctgtcataaccgatgaatacaaagtaccttcaaagaaatttaaggtgttggggaacacagaccgtcattcgattaaaaagaatcttatcggtgccctcctattcgatagtggcgaaacggcagaggcgactcgcctgaaacgaaccgctcggagaaggtatacacgtcgcaagaaccgaatatgttacttacaagaaatttttagcaatgagatggccaaagttgacgattctttctttcaccgtttggaagagtccttccttgtcgaagaggacaagaaacatgaacggcaccccatctttggaaacatagtagatgaggtggcatatcatgaaaagtacccaacgatttatcacctcagaaaaaagctagttgactcaactgataaagcggacctgaggttaatctacttggctcttgcccatatgataaagttccgtgggcactttctcattgagggtgatctaaatccggacaactcggatgtcgacaaactgttcatccagttagtacaaacctataatcagttgtttgaagagaaccctataaatgcaagtggcgtggatgcgaaggctattcttagcgcccgcctctctaaatcccgacggctagaaaacctgatcgcacaattacccggagagaagaaaaatgggttgttcggtaaccttatagcgctctcactaggcctgacaccaaattttaagtcgaacttcgacttagctgaagatgccaaattgcagcttagtaaggacacgtacgatgacgatctcgacaatctactggcacaaattggagatcagtatgcggacttatttttggctgccaaaaaccttagcgatgcaatcctcctatctgacatactgagagttaatactgagattaccaaggcgccgttatccgcttcaatgatcaaaaggtacgatgaacatcaccaagacttgacacttctcaaggccctagtccgtcagcaactgcctgagaaatataaggaaatattctttgatcagtcgaaaaacgggtacgcaggttatattgacggcggagcgagtcaagaggaattctacaagtttatcaaacccatattagagaagatggatgggacggaagagttgcttgtaaaactcaatcgcgaagatctactgcgaaagcagcggactttcgacaacggtagcattccacatcaaatccacttaggcgaattgcatgctatacttagaaggcaggaggatttttatccgttcctcaaagacaatcgtgaaaagattgagaaaatcctaacctttcgcataccttactatgtgggacccctggcccgagggaactctcggttcgcatggatgacaagaaagtccgaagaaacgattactccatggaattttgaggaagttgtcgataaaggtgcgtcagctcaatcgttcatcgagaggatgaccaactttgacaagaatttaccgaacgaaaaagtattgcctaagcacagtttactttacgagtatttcacagtgtacaatgaactcacgaaagttaagtatgtcactgagggcatgcgtaaacccgcctttctaagcggagaacagaagaaagcaatagtagatctgttattcaagaccaaccgcaaagtgacagttaagcaattgaaagaggactactttaagaaaattgaatgcttcgattctgtcgagatctccggggtagaagatcgatttaatgcgtcacttggtacgtatcatgacctcctaaagataattaaagataaggacttcctggataacgaagagaatgaagatatcttagaagatatagtgttgactcttaccctctttgaagatcgggaaatgattgaggaaagactaaaaacatacgctcacctgttcgacgataaggttatgaaacagttaaagaggcgtcgctatacgggctggggacgattgtcgcggaaacttatcaacgggataagagacaagcaaagtggtaaaactattctcgattttctaaagagcgacggcttcgccaataggaactttatgcagctgatccatgatgactctttaaccttcaaagaggatatacaaaaggcacaggtttccggacaaggggactcattgcacgaacatattgcgaatcttgctggttcgccagccatcaaaaagggcatactccagacagtcaaagtagtggatgagctagttaaggtcatgggacgtcacaaaccggaaaacattgtaatcgagatggcacgcgaaaatcaaacgactcagaaggggcaaaaaaacagtcgagagcggatgaagagaatagaagagggtattaaagaactgggcagccagatcttaaaggagcatcctgtggaaaatacccaattgcagaacgagaaactttacctctattacctacaaaatggaagggacatgtatgttgatcaggaactggacataaaccgtttatctgattacgacgtcgatgccattgtaccccaatcctttttgaaggacgattcaatcgacaataaagtgcttacacgctcggataagaaccgagggaaaagtgacaatgttccaagcgaggaagtcgtaaagaaaatgaagaactattggcggcagctcctaaatgcgaaactgataacgcaaagaaagttcgataacttaactaaagctgagaggggtggcttgtctgaacttgacaaggccggatttattaaacgtcagctcgtggaaacccgccaaatcacaaagcatgttgcacagatactagattcccgaatgaatacgaaatacgacgagaacgataagctgattcgggaagtcaaagtaatcactttaaagtcaaaattggtgtcggacttcagaaaggattttcaattctataaagttagggagataaataactaccaccatgcgcacgacgcttatcttaatgccgtcgtagggaccgcactcattaagaaatacccgaagctagaaagtgagtttgtgtatggtgattacaaagtttatgacgtccgtaagatgatcgcgaaaagcgaacaggagataggcaaggctacagccaaatacttcttttattctaacattatgaatttctttaagacggaaatcactctggcaaacggagagatacgcaaacgacctttaattgaaaccaatggggagacaggtgaaatcgtatgggataagggccgggacttcgcgacggtgagaaaagttttgtccatgccccaagtcaacatagtaaagaaaactgaggtgcagaccggagggttttcaaaggaatcgattcttccaaaaaggaatagtgataagctcatcgctcgtaaaaaggactgggacccgaaaaagtacggtggcttcgatagccctacagttgcctattctgtcctagtagtggcaaaagttgagaagggaaaatccaagaaactgaagtcagtcaaagaattattggggataacgattatggagcgctcgtcttttgaaaagaaccccatcgacttccttgaggcgaaaggttacaaggaagtaaaaaaggatctcataattaaactaccaaagtatagtctgtttgagttagaaaatggccgaaaacggatgttggctagcgccggagagcttcaaaaggggaacgaactcgcactaccgtctaaatacgtgaatttcctgtatttagcgtcccattacgagaagttgaaaggttcacctgaagataacgaacagaagcaactttttgttgagcagcacaaacattatctcgacgaaatcatagagcaaatttcggaattcagtaagagagtcatcctagctgatgccaatctggacaaagtattaagcgcatacaacaagcacagggataaacccatacgtgagcaggcggaaaatattatccatttgtttactcttaccaacctcggcgctccagccgcattcaagtattttgacacaacgatagatcgcaaacgatacacttctaccaaggaggtgctagacgcgacactgattcaccaatccatcacgggattatatgaaactcggatagatttgtcacagcttgggggtgactcaggtggaagtggcggcagcggaggttctggatcccaactagtcaaaagtgaactggaggagaagaaatctgaacttcgtcataaattgaaatatgtgcctcatgaatatattgaattaattgaaattgccagaaattccactcaggatagaattcttgaaatgaaggtaatggaattttttatgaaagtttatggatatagaggtaaacatttgggtggatcaaggaaaccggacggagcaatttatactgtcggatctcctattgattacggtgtgatcgtggatactaaagcttatagcggaggttataatctgccaattggccaagcagatgaaatgcaacgatatgtcgaagaaaatcaaacacgaaacaaacatatcaaccctaatgaatggtggaaagtctatccatcttctgtaacggaatttaagtttttatttgtgagtggtcactttaaaggaaactacaaagctcagcttacacgattaaatcatatcactaattgtaatggagctgttcttagtgtagaagagcttttaattggtggagaaatgattaaagccggcacattaaccttagaggaagtcagacggaaatttaataacggcgagataaacttt

SEQ ID NO: 52 - DNA, 4836 bp, synthetic construct
  misc_feature 1..4836: note = Synthetic Polynucleotide
  source 1..4836: mol_type = other DNA
atgggatcccaactagtcaaaagtgaactggaggagaagaaatctgaacttcgtcataaattgaaatatgtgcctcatgaatatattgaattaattgaaattgccagaaattccactcaggatagaattcttgaaatgaaggtaatggaattttttatgaaagtttatggatatagaggtaaacatttgggtggatcaaggaaaccggacggagcaatttatactgtcggatctcctattgattacggtgtgatcgtggatactaaagcttatagcggaggttataatctgccaattggccaagcagatgaaatgcaacgatatgtcgaagaaaatcaaacacgaaacaaacatatcaaccctaatgaatggtggaaagtctatccatcttctgtaacggaatttaagtttttatttgtgagtggtcactttaaaggaaactacaaagctcagcttacacgattaaatcatatcactaattgtaatggagctgttcttagtgtagaagagcttttaattggtggagaaatgattaaagccggcacattaaccttagaggaagtcagacggaaatttaataacggcgagataaactttggcggtagtgggggatctgggggaagtatggataaaaagtattctattggtttagctatcggcactaattccgttggatgggctgtcataaccgatgaatacaaagtaccttcaaagaaatttaaggtgttggggaacacagaccgtcattcgattaaaaagaatcttatcggtgccctcctattcgatagtggcgaaacggcagaggcgactcgcctgaaacgaaccgctcggagaaggtatacacgtcgcaagaaccgaatatgttacttacaagaaatttttagcaatgagatggccaaagttgacgattctttctttcaccgtttggaagagtccttccttgtcgaagaggacaagaaacatgaacggcaccccatctttggaaacatagtagatgaggtggcatatcatgaaaagtacccaacgatttatcacctcagaaaaaagctagttgactcaactgataaagcggacctgaggttaatctacttggctcttgcccatatgataaagttccgtgggcactttctcattgagggtgatctaaatccggacaactcggatgtcgacaaactgttcatccagttagtacaaacctataatcagttgtttgaagagaaccctataaatgcaagtggcgtggatgcgaaggctattcttagcgcccgcctctctaaatcccgacggctagaaaacctgatcgcacaattacccggagagaagaaaaatgggttgttcggtaaccttatagcgctctcactaggcctgacaccaaattttaagtcgaacttcgacttagctgaagatgccaaattgcagcttagtaaggacacgtacgatgacgatctcgacaatctactggcacaaattggagatcagtatgcggacttatttttggctgccaaaaaccttagcgatgcaatcctcctatctgacatactgagagttaatactgagattaccaaggcgccgttatccgcttcaatgatcaaaaggtacgatgaacatcaccaagacttgacacttctcaaggccctagtccgtcagcaactgcctgagaaatataaggaaatattctttgatcagtcgaaaaacgggtacgcaggttatattgacggcggagcgagtcaagaggaattctacaagtttatcaaacccatattagagaagatggatgggacggaagagttgcttgtaaaactcaatcgcgaagatctactgcgaaagcagcggactttcgacaacggtagcattccacatcaaatccacttaggcgaattgcatgctatacttagaaggcaggaggatttttatccgttcctcaaagacaatcgtgaaaagattgagaaaatcctaacctttcgcataccttactatgtgggacccctggcccgagggaactctcggttcgcatggatgacaagaaagtccgaagaaacgattactccatggaattttgaggaagttgtcgataaaggtgcgtcagctcaatcgttcatcgagaggatgaccaactttgacaagaatttaccgaacgaaaaagtattgcctaagcacagtttactttacgagtatttcacagtgtacaatgaactcacgaaagttaagtatgtcactgagggcatgcgtaaacccgcctttctaagcggagaacagaagaaagcaatagtagatctgttattcaagaccaaccgcaaagtgacagttaagcaattgaaagaggactactttaagaaaattgaatgcttcgattctgtcgagatctccggggtagaagatcgatttaatgcgtcacttggtacgtatcatgacctcctaaagataattaaagataaggacttcctggataacgaagagaatgaagatatcttagaagatatagtgttgactcttaccctctttgaagatcgggaaatgattgaggaaagactaaaaacatacgctcacctgttcgacgataaggttatgaaacagttaaagaggcgtcgctatacgggctggggacgattgtcgcggaaacttatcaacgggataagagacaagcaaagtggtaaaactattctcgattttctaaagagcgacggcttcgccaataggaactttatgcagctgatccatgatgactctttaaccttcaaagaggatatacaaaaggcacaggtttccggacaaggggactcattgcacgaacatattgcgaatcttgctggttcgccagccatcaaaaagggcatactccagacagtcaaagtagtggatgagctagttaaggtcatgggacgtcacaaaccggaaaacattgtaatcgagatggcacgcgaaaatcaaacgactcagaaggggcaaaaaaacagtcgagagcggatgaagagaatagaagagggtattaaagaactgggcagccagatcttaaaggagcatcctgtggaaaatacccaattgcagaacgagaaactttacctctattacctacaaaatggaagggacatgtatgttgatcaggaactggacataaaccgtttatctgattacgacgtcgatgccattgtaccccaatcctttttgaaggacgattcaatcgacaataaagtgcttacacgctcggataagaaccgagggaaaagtgacaatgttccaagcgaggaagtcgtaaagaaaatgaagaactattggcggcagctcctaaatgcgaaactgataacgcaaagaaagttcgataacttaactaaagctgagaggggtggcttgtctgaacttgacaaggccggatttattaaacgtcagctcgtggaaacccgccaaatcacaaagcatgttgcacagatactagattcccgaatgaatacgaaatacgacgagaacgataagctgattcgggaagtcaaagtaatcactttaaagtcaaaattggtgtcggacttcagaaaggattttcaattctataaagttagggagataaataactaccaccatgcgcacgacgcttatcttaatgccgtcgtagggaccgcactcattaagaaatacccgaagctagaaagtgagtttgtgtatggtgattacaaagtttatgacgtccgtaagatgatcgcgaaaagcgaacaggagataggcaaggctacagccaaatacttcttttattctaacattatgaatttctttaagacggaaatcactctggcaaacggagagatacgcaaacgacctttaattgaaaccaatggggagacaggtgaaatcgtatgggataagggccgggacttcgcgacggtgagaaaagttttgtccatgccccaagtcaacatagtaaagaaaactgaggtgcagaccggagggttttcaaaggaatcgattcttccaaaaaggaatagtgataagctcatcgctcgtaaaaaggactgggacccgaaaaagtacggtggcttcgatagccctacagttgcctattctgtcctagtagtggcaaaagttgagaagggaaaatccaagaaactgaagtcagtcaaagaattattggggataacgattatggagcgctcgtcttttgaaaagaaccccatcgacttccttgaggcgaaaggttacaaggaagtaaaaaaggatctcataattaaactaccaaagtatagtctgtttgagttagaaaatggccgaaaacggatgttggctagcgccggagagcttcaaaaggggaacgaactcgcactaccgtctaaatacgtgaatttcctgtatttagcgtcccattacgagaagttgaaaggttcacctgaagataacgaacagaagcaactttttgttgagcagcacaaacattatctcgacgaaatcatagagcaaatttcggaattcagtaagagagtcatcctagctgatgccaatctggacaaagtattaagcgcatacaacaagcacagggataaacccatacgtgagcaggcggaaaatattatccatttgtttactcttaccaacctcggcgctccagccgcattcaagtattttgacacaacgatagatcgcaaacgatacacttctaccaaggaggtgctagacgcgacactgattcaccaatccatcacgggattatatgaaactcggatagatttgtcacagcttgggggtgacggatcccccaagaagaagaggaaagtctcgagcgactacaaagaccatgacggtgattataaagatcatgacatcgattacaaggatgacgatgacaaggctgcagga

SEQ ID NO: 53 - DNA, 4854 bp, synthetic construct
  misc_feature 1..4854: note = Synthetic Polynucleotide
  source 1..4854: mol_type = other DNA
atggactacaaagaccatgacggtgattataaagatcatgacatcgattacaaggatgacgatgacaagatggcccccaagaagaagaggaaggtgggcattcaccgcggggtacctggaggttctatgggatcccaactagtcaaaagtgaactggaggagaagaaatctgaacttcgtcataaattgaaatatgtgcctcatgaatatattgaattaattgaaattgccagaaattccactcaggatagaattcttgaaatgaaggtaatggaattttttatgaaagtttatggatatagaggtaaacatttgggtggatcaaggaaaccggacggagcaatttatactgtcggatctcctattgattacggtgtgatcgtggatactaaagcttatagcggaggttataatctgccaattggccaagcagatgaaatgcaacgatatgtcgaagaaaatcaaacacgaaacaaacatatcaaccctaatgaatggtggaaagtctatccatcttctgtaacggaatttaagtttttatttgtgagtggtcactttaaaggaaactacaaagctcagcttacacgattaaatcatatcactaattgtaatggagctgttcttagtgtagaagagcttttaattggtggagaaatgattaaagccggcacattaaccttagaggaagtcagacggaaatttaataacggcgagataaactttggcggtagtgggggatctgggggaagtatggataaaaagtattctattggtttagctatcggcactaattccgttggatgggctgtcataaccgatgaatacaaagtaccttcaaagaaatttaaggtgttggggaacacagaccgtcattcgattaaaaagaatcttatcggtgccctcctattcgatagtggcgaaacggcagaggcgactcgcctgaaacgaaccgctcggagaaggtatacacgtcgcaagaaccgaatatgttacttacaagaaatttttagcaatgagatggccaaagttgacgattctttctttcaccgtttggaagagtccttccttgtcgaagaggacaagaaacatgaacggcaccccatctttggaaacatagtagatgaggtggcatatcatgaaaagtacccaacgatttatcacctcagaaaaaagctagttgactcaactgataaagcggacctgaggttaatctacttggctcttgcccatatgataaagttccgtgggcactttctcattgagggtgatctaaatccggacaactcggatgtcgacaaactgttcatccagttagtacaaacctataatcagttgtttgaagagaaccctataaatgcaagtggcgtggatgcgaaggctattcttagcgcccgcctctctaaatcccgacggctagaaaacctgatcgcacaattacccggagagaagaaaaatgggttgttcggtaaccttatagcgctctcactaggcctgacaccaaattttaagtcgaacttcgacttagctgaagatgccaaattgcagcttagtaaggacacgtacgatgacgatctcgacaatctactggcacaaattggagatcagtatgcggacttatttttggctgccaaaaaccttagcgatgcaatcctcctatctgacatactgagagttaatactgagattaccaaggcgccgttatccgcttcaatgatcaaaaggtacgatgaacatcaccaagacttgacacttctcaaggccctagtccgtcagcaactgcctgagaaatataaggaaatattctttgatcagtcgaaaaacgggtacgcaggttatattgacggcggagcgagtcaagaggaattctacaagtttatcaaacccatattagagaagatggatgggacggaagagttgcttgtaaaactcaatcgcgaagatctactgcgaaagcagcggactttcgacaacggtagcattccacatcaaatccacttaggcgaattgcatgctatacttagaaggcaggaggatttttatccgttcctcaaagacaatcgtgaaaagattgagaaaatcctaacctttcgcataccttactatgtgggacccctggcccgagggaactctcggttcgcatggatgacaagaaagtccgaagaaacgattactccatggaattttgaggaagttgtcgataaaggtgcgtcagctcaatcgttcatcgagaggatgaccaactttgacaagaatttaccgaacgaaaaagtattgcctaagcacagtttactttacgagtatttcacagtgtacaatgaactcacgaaagttaagtatgtcactgagggcatgcgtaaacccgcctttctaagcggagaacagaagaaagcaatagtagatctgttattcaagaccaaccgcaaagtgacagttaagcaattgaaagaggactactttaagaaaattgaatgcttcgattctgtcgagatctccggggtagaagatcgatttaatgcgtcacttggtacgtatcatgacctcctaaagataattaaagataaggacttcctggataacgaagagaatgaagatatcttagaagatatagtgttgactcttaccctctttgaagatcgggaaatgattgaggaaagactaaaaacatacgctcacctgttcgacgataaggttatgaaacagttaaagaggcgtcgctatacgggctggggacgattgtcgcggaaacttatcaacgggataagagacaagcaaagtggtaaaactattctcgattttctaaagagcgacggcttcgccaataggaactttatgcagctgatccatgatgactctttaaccttcaaagaggatatacaaaaggcacaggtttccggacaaggggactcattgcacgaacatattgcgaatcttgctggttcgccagccatcaaaaagggcatactccagacagtcaaagtagtggatgagctagttaaggtcatgggacgtcacaaaccggaaaacattgtaatcgagatggcacgcgaaaatcaaacgactcagaaggggcaaaaaaacagtcgagagcggatgaagagaatagaagagggtattaaagaactgggcagccagatcttaaaggagcatcctgtggaaaatacccaattgcagaacgagaaactttacctctattacctacaaaatggaagggacatgtatgttgatcaggaactggacataaaccgtttatctgattacgacgtcgatgccattgtaccccaatcctttttgaaggacgattcaatcgacaataaagtgcttacacgctcggataagaaccgagggaaaagtgacaatgttccaagcgaggaagtcgtaaagaaaatgaagaactattggcggcagctcctaaatgcgaaactgataacgcaaagaaagttcgataacttaactaaagctgagaggggtggcttgtctgaacttgacaaggccggatttattaaacgtcagctcgtggaaacccgccaaatcacaaagcatgttgcacagatactagattcccgaatgaatacgaaatacgacgagaacgataagctgattcgggaagtcaaagtaatcactttaaagtcaaaattggtgtcggacttcagaaaggattttcaattctataaagttagggagataaataactaccaccatgcgcacgacgcttatcttaatgccgtcgtagggaccgcactcattaagaaatacccgaagctagaaagtgagtttgtgtatggtgattacaaagtttatgacgtccgtaagatgatcgcgaaaagcgaacaggagataggcaaggctacagccaaatacttcttttattctaacattatgaatttctttaagacggaaatcactctggcaaacggagagatacgcaaacgacctttaattgaaaccaatggggagacaggtgaaatcgtatgggataagggccgggacttcgcgacggtgagaaaagttttgtccatgccccaagtcaacatagtaaagaaaactgaggtgcagaccggagggttttcaaaggaatcgattcttccaaaaaggaatagtgataagctcatcgctcgtaaaaaggactgggacccgaaaaagtacggtggcttcgatagccctacagttgcctattctgtcctagtagtggcaaaagttgagaagggaaaatccaagaaactgaagtcagtcaaagaattattggggataacgattatggagcgctcgtcttttgaaaagaaccccatcgacttccttgaggcgaaaggttacaaggaagtaaaaaaggatctcataattaaactaccaaagtatagtctgtttgagttagaaaatggccgaaaacggatgttggctagcgccggagagcttcaaaaggggaacgaactcgcactaccgtctaaatacgtgaatttcctgtatttagcgtcccattacgagaagttgaaaggttcacctgaagataacgaacagaagcaactttttgttgagcagcacaaacattatctcgacgaaatcatagagcaaatttcggaattcagtaagagagtcatcctagctgatgccaatctggacaaagtattaagcgcatacaacaagcacagggataaacccatacgtgagcaggcggaaaatattatccatttgtttactcttaccaacctcggcgctccagccgcattcaagtattttgacacaacgatagatcgcaaacgatacacttctaccaaggaggtgctagacgcgacactgattcaccaatccatcacgggattatatgaaactcggatagatttgtcacagcttgggggtgac

SEQ ID NO: 54 - DNA, 4869 bp, synthetic construct
  misc_feature 1..4869: note = Synthetic Polynucleotide
  source 1..4869: mol_type = other DNA
atggactacaaagaccatgacggtgattataaagatcatgacatcgattacaaggatgacgatgacaagatggcccccaagaagaagaggaaggtgggcattcaccgcggggtacctggaggttctggatcccaactagtcaaaagtgaactggaggagaagaaatctgaacttcgtcataaattgaaatatgtgcctcatgaatatattgaattaattgaaattgccagaaattccactcaggatagaattcttgaaatgaaggtaatggaattttttatgaaagtttatggatatagaggtaaacatttgggtggatcaaggaaaccggacggagcaatttatactgtcggatctcctattgattacggtgtgatcgtggatactaaagcttatagcggaggttataatctgccaattggccaagcagatgaaatgcaacgatatgtcgaagaaaatcaaacacgaaacaaacatatcaaccctaatgaatggtggaaagtctatccatcttctgtaacggaatttaagtttttatttgtgagtggtcactttaaaggaaactacaaagctcagcttacacgattaaatcatatcactaattgtaatggagctgttcttagtgtagaagagcttttaattggtggagaaatgattaaagccggcacattaaccttagaggaagtcagacggaaatttaataacggcgagataaactttagcggcagcgagactcccgggacctcagagtccgccacacccgaaagtgataaaaagtattctattggtttagctatcggcactaattccgttggatgggctgtcataaccgatgaatacaaagtaccttcaaagaaatttaaggtgttggggaacacagaccgtcattcgattaaaaagaatcttatcggtgccctcctattcgatagtggcgaaacggcagaggcgactcgcctgaaacgaaccgctcggagaaggtatacacgtcgcaagaaccgaatatgttacttacaagaaatttttagcaatgagatggccaaagttgacgattctttctttcaccgtttggaagagtccttccttgtcgaagaggacaagaaacatgaacggcaccccatctttggaaacatagtagatgaggtggcatatcatgaaaagtacccaacgatttatcacctcagaaaaaagctagttgactcaactgataaagcggacctgaggttaatctacttggctcttgcccatatgataaagttccgtgggcactttctcattgagggtgatctaaatccggacaactcggatgtcgacaaactgttcatccagttagtacaaacctataatcagttgtttgaagagaaccctataaatgcaagtggcgtggatgcgaaggctattcttagcgcccgcctctctaaatcccgacggctagaaaacctgatcgcacaattacccggagagaagaaaaatgggttgttcggtaaccttatagcgctctcactaggcctgacaccaaattttaagtcgaacttcgacttagctgaagatgccaaattgcagcttagtaaggacacgtacgatgacgatctcgacaatctactggcacaaattggagatcagtatgcggacttatttttggctgccaaaaaccttagcgatgcaatcctcctatctgacatactgagagttaatactgagattaccaaggcgccgttatccgcttcaatgatcaaaaggtacgatgaacatcaccaagacttgacacttctcaaggccctagtccgtcagcaactgcctgagaaatataaggaaatattctttgatcagtcgaaaaacgggtacgcaggttatattgacggcggagcgagtcaagaggaattctacaagtttatcaaacccatattagagaagatggatgggacggaagagttgcttgtaaaactcaatcgcgaagatctactgcgaaagcagcggactttcgacaacggtagcattccacatcaaatccacttaggcgaattgcatgctatacttagaaggcaggaggatttttatccgttcctcaaagacaatcgtgaaaagattgagaaaatcctaacctttcgcataccttactatgtgggacccctggcccgagggaactctcggttcgcatggatgacaagaaagtccgaagaaacgattactccatggaattttgaggaagttgtcgataaaggtgcgtcagctcaatcgttcatcgagaggatgaccaactttgacaagaatttaccgaacgaaaaagtattgcctaagcacagtttactttacgagtatttcacagtgtacaatgaactcacgaaagttaagtatgtcactgagggcatgcgtaaacccgcctttctaagcggagaacagaagaaagcaatagtagatctgttattcaagaccaaccgcaaagtgacagttaagcaattgaaagaggactactttaagaaaattgaatgcttcgattctgtcgagatctccggggtagaagatcgatttaatgcgtcacttggtacgtatcatgacctcctaaagataattaaagataaggacttcctggataacgaagagaatgaagatatcttagaagatatagtgttgactcttaccctctttgaagatcgggaaatgattgaggaaagactaaaaacatacgctcacctgttcgacgataaggttatgaaacagttaaagaggcgtcgctatacgggctggggacgattgtcgcggaaacttatcaacgggataagagacaagcaaagtggtaaaactattctcgattttctaaagagcgacggcttcgccaataggaactttatgcagctgatccatgatgactctttaaccttcaaagaggatatacaaaaggcacaggtttccggacaaggggactcattgcacgaacatattgcgaatcttgctggttcgccagccatcaaaaagggcatactccagacagtcaaagtagtggatgagctagttaaggtcatgggacgtcacaaaccggaaaacattgtaatcgagatggcacgcgaaaatcaaacgactcagaaggggcaaaaaaacagtcgagagcggatgaagagaatagaagagggtattaaagaactgggcagccagatcttaaaggagcatcctgtggaaaatacccaattgcagaacgagaaactttacctctattacctacaaaatggaagggacatgtatgttgatcaggaactggacataaaccgtttatctgattacgacgtcgatgccattgtaccccaatcctttttgaaggacgattcaatcgacaataaagtgcttacacgctcggataagaaccgagggaaaagtgacaatgttccaagcgaggaagtcgtaaagaaaatgaagaactattggcggcagctcctaaatgcgaaactgataacgcaaagaaagttcgataacttaactaaagctgagaggggtggcttgtctgaacttgacaaggccggatttattaaacgtcagctcgtggaaacccgccaaatcacaaagcatgttgcacagatactagattcccgaatgaatacgaaatacgacgagaacgataagctgattcgggaagtcaaagtaatcactttaaagtcaaaattggtgtcggacttcagaaaggattttcaattctataaagttagggagataaataactaccaccatgcgcacgacgcttatcttaatgccgtcgtagggaccgcactcattaagaaatacccgaagctagaaagtgagtttgtgtatggtgattacaaagtttatgacgtccgtaagatgatcgcgaaaagcgaacaggagataggcaaggctacagccaaatacttcttttattctaacattatgaatttctttaagacggaaatcactctggcaaacggagagatacgcaaacgacctttaattgaaaccaatggggagacaggtgaaatcgtatgggataagggccgggacttcgcgacggtgagaaaagttttgtccatgccccaagtcaacatagtaaagaaaactgaggtgcagaccggagggttttcaaaggaatcgattcttccaaaaaggaatagtgataagctcatcgctcgtaaaaaggactgggacccgaaaaagtacggtggcttcgatagccctacagttgcctattctgtcctagtagtggcaaaagttgagaagggaaaatccaagaaactgaagtcagtcaaagaattattggggataacgattatggagcgctcgtcttttgaaaagaaccccatcgacttccttgaggcgaaaggttacaaggaagtaaaaaaggatctcataattaaactaccaaagtatagtctgtttgagttagaaaatggccgaaaacggatgttggctagcgccggagagcttcaaaaggggaacgaactcgcactaccgtctaaatacgtgaatttcctgtatttagcgtcccattacgagaagttgaaaggttcacctgaagataacgaacagaagcaactttttgttgagcagcacaaacattatctcgacgaaatcatagagcaaatttcggaattcagtaagagagtcatcctagctgatgccaatctggacaaagtattaagcgcatacaacaagcacagggataaacccatacgtgagcaggcggaaaatattatccatttgtttactcttaccaacctcggcgctccagccgcattcaagtattttgacacaacgatagatcgcaaacgatacacttctaccaaggaggtgctagacgcgacactgattcaccaatccatcacgggattatatgaaactcggatagatttgtcacagcttgggggtgac

SEQ ID NO: 55 - DNA, 432 bp, synthetic construct
  misc_feature 1..432: note = Synthetic Polynucleotide
  source 1..432: mol_type = other DNA
atggccctgtttggctacgcacgcgtgtctaccagtcaacagtcactcgatttgcaagtgagggctcttaaagatgccggagtgaaggcaaacagaatttttactgataaggccagcggaagcagcacagacagagaggggctggatctcctgagaatgaaggtaaaggagggtgatgtgatcttggtcaaaaaattggatcgactggggagagacacagctgatatgcttcagcttattaaagagtttgacgctcagggtgttgccgtgaggtttatcgatgacggcatctcaaccgactcctacattggtcttatgtttgtgacaattttgtccgctgtggctcaggctgagcggagaaggattctcgaaaggacgaatgagggacggcaagcagctaagttgaaaggtatcaaatttggcagacgaagg

SEQ ID NO: 56 - protein, 144 aa, synthetic construct
  REGION 1..144: note = Synthetic Polypeptide
MALFGYARVSTSQQSLDLQVRALKDAGVKANRIFTDKASGSSTDREGLDLLRMKVKEGDVILVKKLDRLGRDTADMLQLIKEFDAQGVAVRFIDDGISTDSYIGLMFVTILSAVAQAERRRILERTNEGRQAAKLKGIKFGRRR

SEQ ID NO: 57 - DNA, 414 bp, synthetic construct
  misc_feature 1..414: note = Synthetic Polynucleotide
  source 1..414: mol_type = other DNA
atggcaaccattggctacataagggtgtctaccatcgaccaaaatatcgacctgcagcgcaacgctctgacatccgccaactgcgatcggatcttcgaggataggatcagtggcaagatcgccaaccggcccggtctgaagcgggctctgaagtacgtgaataagggcgatactctggttgtgtggaagttggatcgcttgggtagatcagtgaagaatctcgtagccctgataagcgagctgcacgagaggggtgcacatttccattctctgaccgattccatcgatacgtctagcgccatgggccgattcttcttttacgtcatgtccgccctcgctgaaatggagcgcgaacttattgttgaacggactttggctggactggcagcggctagagcacagggccgacttgga

SEQ ID NO: 58 - protein, 138 aa, synthetic construct
  REGION 1..138: note = Synthetic Polypeptide
MATIGYIRVSTIDQNIDLQRNALTSANCDRIFEDRISGKIANRPGLKRALKYVNKGDTLVVWKLDRLGRSVKNLVALISELHERGAHFHSLTDSIDTSSAMGRFFFYVMSALAEMERELIVERTLAGLAAARAQGRLG

SEQ ID NO: 59 - DNA, 432 bp, synthetic construct
  misc_feature 1..432: note = Synthetic Polynucleotide
  source 1..432: mol_type = other DNA
atgctcattggctatgtaagggtcagcaccaatgaccaaaacacagacttgcaacgcaatgctttggtttgcgccggatgtgaacagatatttgaagataaactgagcggcactcggacagacagacctgggcttaagagagcactgaaaagactgcagaagggggacaccctggtcgtctggaaactggatcgcctcggacgcagcatgaaacatctgattagcctggttggtgagcttagggagagaggaatcaacttcagaagcctgaccgactccatcgacaccagtagccccatgggacgattcttcttctatgtgatgggagcacttgctgagatggaaagagagcttattatcgaaagaactatggctggtatcgctgctgcccggaacaaaggcagacggttcggcagaccgccgaagagcggc

SEQ ID NO: 60 - protein, 144 aa, synthetic construct
  REGION 1..144: note = Synthetic Polypeptide
MLIGYVRVSTNDQNTDLQRNALVCAGCEQIFEDKLSGTRTDRPGLKRALKRLQKGDTLVVWKLDRLGRSMKHLISLVGELRERGINFRSLTDSIDTSSPMGRFFFYVMGALAEMERELIIERTMAGIAAARNKGRRFGRPPKSG

SEQ ID NO: 61 - protein, 198 aa, Homo sapiens [sequence omitted]

SEQ ID NO: 62 - protein, 198 aa, Mus musculus
MDSLLMKQKKFLYHFKNVRWAKGRHETYLCYVVKRRDSATSCSLDFGHLRNKSGCHVELLFLRYISDWDLDPGRCYRVTWFTSWSPCYDCARHVAEFLRWNPNLSLRIFTARLYFCEDRKAEPEGLRRLHRAGVQIGIMTFKDYFYCWNTFVENRERTFKAWEGLHENSVRLTRQLRRILLPLYEVDDLRDAFRMLGF

SEQ ID NO: 63 - protein, 198 aa, Canis lupus
MDSLLMKQRKFLYHFKNVRWAKGRHETYLCYVVKRRDSATSFSLDFGHLRNKSGCHVELLFLRYISDWDLDPGRCYRVTWFTSWSPCYDCARHVADFLRGYPNLSLRIFAARLYFCEDRKAEPEGLRRLHRAGVQIAIMTFKDYFYCWNTFVENREKTFKAWEGLHENSVRLSRQLRRILLPLYEVDDLRDAFRTLGL

SEQ ID NO: 64 - protein, 199 aa, Bos taurus
MDSLLKKQRQFLYQFKNVRWAKGRHETYLCYVVKRRDSPTSFSLDFGHLRNKAGCHVELLFLRYISDWDLDPGRCYRVTWFTSWSPCYDCARHVADFLRGYPNLSLRIFTARLYFCDKERKAEPEGLRRLHRAGVQIAIMTFKDYFYCWNTFVENHERTFKAWEGLHENSVRLSRQLRRILLPLYEVDDLRDAFRTLGL

SEQ ID NO: 65 - protein, 429 aa, Mus musculus
MGPFCLGCSHRKCYSPIRNLISQETFKFHFKNLGYAKGRKDTFLCYEVTRKDCDSPVSLHHGVFKNKDNIHAEICFLYWFHDKVLKVLSPREEFKITWYMSWSPCFECAEQIVRFLATHHNLSLDIFSSRLYNVQDPETQQNLCRLVQEGAQVAAMDLYEFKKCWKKFVDNGGRRFRPWKRLLTNFRYQDSKLQEILRPCYIPVPSSSSSTLSNICLTKGLPETRFCVEGRRMDPLSEEEFYSQFYNQRVKHLCYYHRMKPYLCYQLEQFNGQAPLKGCLLSEKGKQHAEILFLDKIRSMELSQVTITCYLTWSPCPNCAWQLAAFKRDRPDLILHIYTSRLYFHWKRPFQKGLCSLWQSGILVDVMDLPQFTDCWTNFVNPKRPFWPWKGLEIISRRTQRRLRRIKESWGLQDLVNDFGNLQLGPPMS

SEQ ID NO: 66 - protein, 429 aa, Rattus norvegicus
MGPFCLGCSHRKCYSPIRNLISQETFKFHFKNLRYAIDRKDTFLCYEVTRKDCDSPVSLHHGVFKNKDNIHAEICFLYWFHDKVLKVLSPREEFKITWYMSWSPCFECAEQVLRFLATHHNLSLDIFSSRLYNIRDPENQQNLCRLVQEGAQVAAMDLYEFKKCWKKFVDNGGRRFRPWKKLLTNFRYQDSKLQEILRPCYIPVPSSSSSTLSNICLTKGLPETRFCVERRRVHLLSEEEFYSQFYNQRVKHLCYYHGVKPYLCYQLEQFNGQAPLKGCLLSEKGKQHAEILFLDKIRSMELSQVIITCYLTWSPCPNCAWQLAAFKRDRPDLILHIYTSRLYFHWKRPFQKGLCSLWQSGILVDVMDLPQFTDCWTNFVNPKRPFWPWKGLEIISRRTQRRLHRIKESWGLQDLVNDFGNLQLGPPMS

SEQ ID NO: 67 - protein, 370 aa, Macaca mulatta
MVEPMDPRTFVSNFNNRPILSGLNTVWLCCEVKTKDPSGPPLDAKIFQGKVYSKAKYHPEMRFLRWFHKWRQLHHDQEYKVTWYVSWSPCTRCANSVATFLAKDPKVTLTIFVARLYYFWKPDYQQALRILCQKRGGPHATMKIMNYNEFQDCWNKFVDGRGKPFKPRNNLPKHYTLLQATLGELLRHLMDPGTFTSNFNNKPWVSGQHETYLCYKVERLHNDTWVPLNQHRGFLRNQAPNIHGFPKGRHAELCFLDLIPFWKLDGQQYRVTCFTSWSPCFSCAQEMAKFISNNEHVSLCIFAARIYDDQGRYQEGLRALHRDGAKIAMMNYSEFEYCWDTFVDRQGRPFQPWDGLDEHSQALSGRLRAI

SEQ ID NO: 68 - protein, 384 aa, Pan troglodytes
MKPHFRNPVERMYQDTFSDNFYNRPILSHRNTVWLCYEVKTKGPSRPPLDAKIFRGQVYSKLKYHPEMRFFHWFSKWRKLHRDQEYEVTWYISWSPCTKCTRDVATFLAEDPKVTLTIFVARLYYFWDPDYQEALRSLCQKRDGPRATMKIMNYDEFQHCWSKFVYSQRELFEPWNNLPKYYILLHIMLGEILRHSMDPPTFTSNFNNELWVRGRHETYLCYEVERLHNDTWVLLNQRRGFLCNQAPHKHGFLEGRHAELCFLDVIPFWKLDLHQDYRVTCFTSWSPCFSCAQEMAKFISNNKHVSLCIFAARIYDDQGRCQEGLRTLAKAGAKISIMTYSEFKHCWDTFVDHQGCPFQPWDGLEEHSQALSGRLRAILQNQGN

SEQ ID NO: 69 - protein, 377 aa, Chlorocebus sabaeus
MNPQIRNMVEQMEPDIFVYYFNNRPILSGRNTVWLCYEVKTKDPSGPPLDANIFQGKLYPEAKDHPEMKFLHWFRKWRQLHRDQEYEVTWYVSWSPCTRCANSVATFLAEDPKVTLTIFVARLYYFWKPDYQQALRILCQERGGPHATMKIMNYNEFQHCWNEFVDGQGKPFKPRKNLPKHYTLLHATLGELLRHVMDPGTFTSNFNNKPWVSGQRETYLCYKVERSHNDTWVLLNQHRGFLRNQAPDRHGFPKGRHAELCFLDLIPFWKLDDQQYRVTCFTSWSPCFSCAQKMAKFISNNKHVSLCIFAARIYDDQGRCQEGLRTLHRDGAKIAVMNYSEFEYCWDTFVDRQGRPFQPWDGLDEHSQALSGRLRAI

SEQ ID NO: 70 - protein, 384 aa, Homo sapiens
MKPHFRNTVERMYRDTFSYNFYNRPILSRRNTVWLCYEVKTKGPSRPPLDAKIFRGQVYSELKYHPEMRFFHWFSKWRKLHRDQEYEVTWYISWSPCTKCTRDMATFLAEDPKVTLTIFVARLYYFWDPDYQEALRSLCQKRDGPRATMKIMNYDEFQHCWSKFVYSQRELFEPWNNLPKYYILLHIMLGEILRHSMDPPTFTFNFNNEPWVRGRHETYLCYEVERMHNDTWVLLNQRRGFLCNQAPHKHGFLEGRHAELCFLDVIPFWKLDLDQDYRVTCFTSWSPCFSCAQEMAKFISKNKHVSLCIFTARIYDDQGRCQEGLRTLAEAGAKISIMTYSEFKHCWDTFVDHQGCPFQPWDGLDEHSQDLSGRLRAILQNQEN

SEQ ID NO: 71 - protein, 373 aa, Homo sapiens
MKPHFRNTVERMYRDTFSYNFYNRPILSRRNTVWLCYEVKTKGPSRPRLDAKIFRGQVYSQPEHHAEMCFLSWFCGNQLPAYKCFQITWFVSWTPCPDCVAKLAEFLAEHPNVTLTISAARLYYYWERDYRRALCRLSQAGARVKIMDDEEFAYCWENFVYSEGQPFMPWYKFDDNYAFLHRTLKEILRNPMEAMYPHIFYFHFKNLRKAYGRNESWLCFTMEVVKHHSPVSWKRGVFRNQVDPETHCHAERCFLSWFCDDILSPNTNYEVTWYTSWSPCPECAGEVAEFLARHSNVNLTIFTARLYYFWDTDYQEGLRSLSQEGASVEIMGYKDFKYCWENFVYNDDEPFKPWKGLKYNFLFLDSKLQEILE

SEQ ID NO: 72 - protein, 382 aa, Homo sapiens
MNPQIRNPMERMYRDTFYDNFENEPILYGRSYTWLCYEVKIKRGRSNLLWDTGVFRGQVYFKPQYHAEMCFLSWFCGNQLPAYKCFQITWFVSWTPCPDCVAKLAEFLSEHPNVTLTISAARLYYYWERDYRRALCRLSQAGARVTIMDYEEFAYCWENFVYNEGQQFMPWYKFDENYAFLHRTLKEILRYLMDPDTFTFNFNNDPLVLRRRQTYLCYEVERLDNGTWVLMDQHMGFLCNEAKNLLCGFYGRHAELRFLDLVPSLQLDPAQIYRVTWFISWSPCFSWGCAGEVRAFLQENTHVRLRIFAARIYDYDPLYKEALQMLRDAGAQVSIMTYDEFEYCWDTFVYRQGCPFQPWDGLEEHSQALSGRLRAILQNQGN

SEQ ID NO: 73 - protein, 190 aa, Homo sapiens
MNPQIRNPMKAMYPGTFYFQFKNLWEANDRNETWLCFTVEGIKRRSVVSWKTGVFRNQVDSETHCHAERCFLSWFCDDILSPNTKYQVTWYTSWSPCPDCAGEVAEFLARHSNVNLTIFTARLYYFQYPCYQEGLRSLSQEGVAVEIMDYEDFKYCWENFVYNDNEPFKPWKGLKTNFRLLKRRLRESLQ

SEQ ID NO: 74 - protein, 199 aa, Homo sapiens
MEASPASGPRHLMDPHIFTSNFNNGIGRHKTYLCYEVERLDNGTSVKMDQHRGFLHNQAKNLLCGFYGRHAELRFLDLVPSLQLDPAQIYRVTWFISWSPCFSWGCAGEVRAFLQENTHVRLRIFAARIYDYDPLYKEALQMLRDAGAQVSIMTYDEFKHCWDTFVDHQGCPFQPWDGLDEHSQALSGRLRAILQNQGN

SEQ ID NO: 75 - protein, 200 aa, Homo sapiens
MALLTAETFRLQFNNKRRLRRPYYPRKALLCYQLTPQNGSTPTRGYFENKKKCHAEICFINEIKSMGLDETQCYQVTCYLTWSPCSSCAWELVDFIKAHDHLNLGIFASRLYYHWCKPQQKGLRLLCGSQVPVEVMGFPKFADCWENFVDHEKPLSFNPYKMLEELDKNSRAIKRRLERIKIPGVRAQGRYMDILCDAEV

SEQ ID NO: 76 - protein, 386 aa, Homo sapiens
MNPQIRNPMERMYRDTFYDNFENEPILYGRSYTWLCYEVKIKRGRSNLLWDTGVFRGPVLPKRQSNHRQEVYFRFENHAEMCFLSWFCGNRLPANRRFQITWFVSWNPCLPCVVKVTKFLAEHPNVTLTISAARLYYYRDRDWRWVLLRLHKAGARVKIMDYEDFAYCWENFVCNEGQPFMPWYKFDDNYASLHRTLKEILRNPMEAMYPHIFYFHFKNLLKACGRNESWLCFTMEVTKHHSAVFRKRGVFRNQVDPETHCHAERCFLSWFCDDILSPNTNYEVTWYTSWSPCPECAGEVAEFLARHSNVNLTIFTARLCYFWDTDYQEGLCSLSQEGASVKIMGYKDFVSCWKNFVYSDDEPFKPWKGLQTNFRLLKRRLREILQ

SEQ ID NO: 77 - protein, 236 aa, Homo sapiens
MTSEKGPSTGDPTLRRRIEPWEFDVFYDPRELRKEACLLYEIKWGMSRKIWRSSGKNTTNHVEVNFIKKFTSERDFHPSMSCSITWFLSWSPCWECSQAIREFLSRHPGVTLVIYVARLFWHMDQQNRQGLRDLVNSGVTIQIMRASEYYHCWRNFVNYPPGDEAHWPQYPPLWMMLYALELHCIILSLPPCLKISRRWQNHLTFFRLHLQNCHYQTIPPHILLATGLIHPSVAWR

SEQ ID NO: 78 - protein, 229 aa, Mus musculus
MSSETGPVAVDPTLRRRIEPHEFEVFFDPRELRKETCLLYEINWGGRHSVWRHTSQNTSNHVEVNFLEKFTTERYFRPNTRCSITWFLSWSPCGECSRAITEFLSRHPYVTLFIYIARLYHHTDQRNRQGLRDLISSGVTIQIMTEQEYCYCWRNFVNYPPSNEAYWPRYPHLWVKLYVLELYCIILGLPPCLKILRRKQPQLTFFTITLQTCHYQRIPPHLLWATGLK

SEQ ID NO: 79 - protein, 229 aa, Rattus norvegicus [sequence omitted]

SEQ ID NO: 80 - protein, 191 aa, Homo sapiens
MEAKAAPKPAASGACSVSAEETEKWMEEAMHMAKEALENTEVPVGCLMVYNNEVVGKGRNEVNQTKNATRHAEMVAIDQVLDWCRQSGKSPSEVFEHTVLYVTVEPCIMCAAALRLMKIPLVVYGCQNERFGGCGSVLNIASADLPNTGRPFQCIPGYRAEEAVEMLKTFYKQENPNAPKSKVRKKECQKS

SEQ ID NO: 81 - protein, 191 aa, Mus musculus
MEEKVESTTTPDGPCVVSVQETEKWMEEAMRMAKEALENIEVPVGCLMVYNNEVVGKGRNEVNQTKNATRHAEMVAIDQVLDWCHQHGQSPSTVFEHTVLYVTVEPCIMCAAALRLMKIPLVVYGCQNERFGGCGSVLNIASADLPNTGRPFQCIPGYRAEEAVELLKTFYKQENPNAPKSKVRKKDCQKS

SEQ ID NO: 82 - protein, 499 aa, Mus musculus
MWTADEIAQLCYAHYNVRLPKQGKPEPNREWTLLAAVVKIQASANQACDIPEKEVQVTKEVVSMGTGTKCIGQSKMRESGDILNDSHAEIIARRSFQRYLLHQLHLAAVLKEDSIFVPGTQRGLWRLRPDLSFVFFSSHTPCGDASIIPMLEFEEQPCCPVIRSWANNSPVQETENLEDSKDKRNCEDPASPVAKKMRLGTPARSLSNCVAHHGTQESGPVKPDVSSSDLTKEEPDAANGIASGSFRVVDVYRTGAKCVPGETGDLREPGAAYHQVGLLRVKPGRGDRTCSMSCSDKMARWNVLGCQGALLMHFLEKPIYLSAVVIGKCPYSQEAMRRALTGRCEETLVLPRGFGVQELEIQQSGLLFEQSRCAVHRKRGDSPGRLVPCGAAISWSAVPQQPLDVTANGFPQGTTKKEIGSPRARSRISKVELFRSFQKLLSSIADDEQPDSIRVTKKLDTYQEYKDAASAYQEAWGALRRIQPFASWIRNPPDYHQFK

SEQ ID NO: 83 - protein, 502 aa, Homo sapiens
MWTADEIAQLCYEHYGIRLPKKGKPEPNHEWTLLAAVVKIQSPADKACDTPDKPVQVTKEVVSMGTGTKCIGQSKMRKNGDILNDSHAEVIARRSFQRYLLHQLQLAATLKEDSIFVPGTQKGVWKLRRDLIFVFFSSHTPCGDASIIPMLEFEDQPCCPVFRNWAHNSSVEASSNLEAPGNERKCEDPDSPVTKKMRLEPGTAAREVTNGAAHHQSFGKQKSGPISPGIHSCDLTVEGLATVTRIAPGSAKVIDVYRTGAKCVPGEAGDSGKPGAAFHQVGLLRVKPGRGDRTRSMSCSDKMARWNVLGCQGALLMHLLEEPIYLSAVVIGKCPYSQEAMQRALIGRCQNVSALPKGFGVQELKILQSDLLFEQSRSAVQAKRADSPGRLVPCGAAISWSAVPEQPLDVTANGFPQGTTKKTIGSLQARSQISKVELFRSFQKLLSRIARDKWPHSLRVQKLDTYQEYKEAASSYQEAWSTLRKQVFGSWIRNPPDYHQFK

SEQ ID NO: 84 - protein, 57 aa, synthetic construct
  REGION 1..57: note = Synthetic Polypeptide
GSGRADALDDFDLDMLGSDALDDFDLDMLGSDALDDFDLDMLGSDALDDFDLDMLIN

SEQ ID NO: 85 - protein, 85 aa, synthetic construct
  REGION 1..85: note = Synthetic Polypeptide
APPTDVSLGDELHLDGEDVAMAHADALDDFDLDMLGDGDSPGPGFTPHDSAPYGALDMADFEFEQMFTDALGIDEYGGEFPGIRR

SEQ ID NO: 86 - protein, 184 aa, synthetic construct
  REGION 1..184: note = Synthetic Polypeptide
PSGQISNQALALAPSSAPVLAQTMVPSSAMVPLAQPPAPAPVLTPGPPQSLSAPVPKSTQAGEGTLSEALLHLQFDADEDLGALLGNSTDPGVFTDLASVDNSEFQQLLNQGVSMSHSTAEPMLMEYPEAITRLVTGSQRPPDPAPTPLGTSGLPNGLSGDEDFSSIADMDFSALLSQISSSGQ

SEQ ID NO: 87 - protein, 1467 aa, synthetic construct
  REGION 1..1467: note = Synthetic Polypeptide
MDKKYSIGLAIGTNSVGWAVITDEYKVPSKKFKVLGNTDRHSIKKNLIGALLFDSGETAEATRLKRTARRRYTRRKNRICYLQEIFSNEMAKVDDSFFHRLEESFLVEEDKKHERHPIFGNIVDEVAYHEKYPTIYHLRKKLVDSTDKADLRLIYLALAHMIKFRGHFLIEGDLNPDNSDVDKLFIQLVQTYNQLFEENPINASGVDAKAILSARLSKSRRLENLIAQLPGEKKNGLFGNLIALSLGLTPNFKSNFDLAEDAKLQLSKDTYDDDLDNLLAQIGDQYADLFLAAKNLSDAILLSDILRVNTEITKAPLSASMIKRYDEHHQDLTLLKALVRQQLPEKYKEIFFDQSKNGYAGYIDGGASQEEFYKFIKPILEKMDGTEELLVKLNREDLLRKQRTFDNGSIPHQIHLGELHAILRRQEDFYPFLKDNREKIEKILTFRIPYYVGPLARGNSRFAWMTRKSEETITPWNFEEVVDKGASAQSFIERMTNFDKNLPNEKVLPKHSLLYEYFTVYNELTKVKYVTEGMRKPAFLSGEQKKAIVDLLFKTNRKVTVKQLKEDYFKKIECFDSVEISGVEDRFNASLGTYHDLLKIIKDKDFLDNEENEDILEDIVLTLTLFEDREMIEERLKTYAHLFDDKVMKQLKRRRYTGWGRLSRKLINGIRDKQSGKTILDFLKSDGFANRNFMQLIHDDSLTFKEDIQKAQVSGQGDSLHEHIANLAGSPAIKKGILQTVKVVDELVKVMGRHKPENIVIEMARENQTTQKGQKNSRERMKRIEEGIKELGSQILKEHPVENTQLQNEKLYLYYLQNGRDMYVDQELDINRLSDYDVDAIVPQSFLKDDSIDNKVLTRSDKNRGKSDNVPSEEVVKKMKNYWRQLLNAKLITQRKFDNLTKAERGGLSELDKAGFIKRQLVETRQITKHVAQILDSRMNTKYDENDKLIREVKVITLKSKLVSDFRKDFQFYKVREINNYHHAHDAYLNAVVGTALIKKYPKLESEFVYGDYKVYDVRKMIAKSEQEIGKATAKYFFYSNIMNFFKTEITLANGEIRKRPLIETNGETGEIVWDKGRDFATVRKVLSMPQVNIVKKTEVQTGGFSKESILPKRNSDKLIARKKDWDPKKYGGFDSPTVAYSVLVVAKVEKGKSKKLKSVKELLGITIMERSSFEKNPIDFLEAKGYKEVKKDLIIKLPKYSLFELENGRKRMLASAGELQKGNELALPSKYVNFLYLASHYEKLKGSPEDNEQKQLFVEQHKHYLDEIIEQISEFSKRVILADANLDKVLSAYNKHRDKPIREQAENIIHLFTLTNLGAPAAFKYFDTTIDRKRYTSTKEVLDATLIHQSITGLYETRIDLSQLGGDGSPKKKRKVSSDYKDHDGDYKDHDIDYKDDDDKAAGGGGSGRADALDDFDLDMLGSDALDDFDLDMLGSDALDDFDLDMLGSDALDDFDLDMLHHHHHH

SEQ ID NO: 88 - protein, 94 aa, Homo sapiens
MNMFKEAVTFKDVAVAFTEEELGLLGPAQRKLYRDVMVENFRNLLSVGHPPFKQDVSPIERNEQLWIMTTATRRQGNLDTLPVKALLLYDLAQT

SEQ ID NO: 89 - protein, 74 aa, Homo sapiens
EQVSFKDVCVDFTQEEWYLLDPAQKILYRDVILENYSNLVSVGYCITKPEVIFKIEQGEEPWILEKGFPSQCHP

SEQ ID NO: 90 - protein, 42 aa, Homo sapiens
EAVTFKDVAVVFTEEELGLLDPAQRKLYRDVMLENFRNLLSV

SEQ ID NO: 91 - protein, 69 aa, Mus musculus
MDLVTYDDVHVNFTQDEWALLDPSQKSLYKGVMLETYKNLTAIGYIWEEHTIEDHFQTSRSHGSNKKTH

SEQ ID NO: 92 - protein, 32 aa, synthetic construct
  REGION 1..32: note = Synthetic Polypeptide
GSGMNIQMLLEAADYLERREREAEHGYASMLP

SEQ ID NO: 93 - protein, 130 aa, synthetic construct
  REGION 1..130: note = Synthetic Polypeptide
GSGMNIQMLLEAADYLERREREAEHGYASMLPGSGMNIQMLLEAADYLERREREAEHGYASMLPGSGMNIQMLLEAADYLERREREAEHGYASMLPGSGMNIQMLLEAADYLERREREAEHGYASMLPSR

SEQ ID NO: 94 - protein, 876 aa, Homo sapiens
MLSGKKAAAAAAAAAAAATGTEAGPGTAGGSENGSEVAAQPAGLSGPAEVGPGAVGERTPRKKEPPRASPPGGLAEPPGSAGPQAGPTVVPGSATPMETGIAETPEGRRTSRRKRAKVEYREMDESLANLSEDEYYSEEERNAKAEKEKKLPPPPPQAPPEEENESEPEEPSGQAGGLQDDSSGGYGDGQASGVEGAAFQSRLPHDRMTSQEAACFPDIISGPQQTQKVFLFIRNRTLQLWLDNPKIQLTFEATLQQLEAPYNSDTVLVHRVHSYLERHGLINFGIYKRIKPLPTKKTGKVIIIGSGVSGLAAARQLQSFGMDVTLLEARDRVGGRVATFRKGNYVADLGAMVVTGLGGNPMAVVSKQVNMELAKIKQKCPLYEANGQADTVKVPKEKDEMVEQEFNRLLEATSYLSHQLDFNVLNNKPVSLGQALEVVIQLQEKHVKDEQIEHWKKIVKTQEELKELLNKMVNLKEKIKELHQQYKEASEVKPPRDITAEFLVKSKHRDLTALCKEYDELAETQGKLEEKLQELEANPPSDVYLSSRDRQILDWHFANLEFANATPLSTLSLKHWDQDDDFEFTGSHLTVRNGYSCVPVALAEGLDIKLNTAVRQVRYTASGCEVIAVNTRSTSQTFIYKCDAVLCTLPLGVLKQQPPAVQFVPPLPEWKTSAVQRMGFGNLNKVVLCFDRVFWDPSVNLFGHVGSTTASRGELFLFWNLYKAPILLALVAGEAAGIMENISDDVIVGRCLAILKGIFGSSAVPQPKETVVSRWRADPWARGSYSYVAAGSSGNDYDLMAQPITPGPSIPGAPQPIPRLFFAGEHTIRNYPATVHGALLSGLREAGRIADQFLGAMYTLPRQATPGVPAQQSPSM

SEQ ID NO: 95 - protein, 852 aa, Homo sapiens
MLSGKKAAAAAAAAAAAATGTEAGPGTAGGSENGSEVAAQPAGLSGPAEVGPGAVGERTPRKKEPPRASPPGGLAEPPGSAGPQAGPTVVPGSATPMETGIAETPEGRRTSRRKRAKVEYREMDESLANLSEDEYYSEEERNAKAEKEKKLPPPPPQAPPEEENESEPEEPSGVEGAAFQSRLPHDRMTSQEAACFPDIISGPQQTQKVFLFIRNRTLQLWLDNPKIQLTFEATLQQLEAPYNSDTVLVHRVHSYLERHGLINFGIYKRIKPLPTKKTGKVIIIGSGVSGLAAARQLQSFGMDVTLLEARDRVGGRVATFRKGNYVADLGAMVVTGLGGNPMAVVSKQVNMELAKIKQKCPLYEANGQAVPKEKDEMVEQEFNRLLEATSYLSHQLDFNVLNNKPVSLGQALEVVIQLQEKHVKDEQIEHWKKIVKTQEELKELLNKMVNLKEKIKELHQQYKEASEVKPPRDITAEFLVKSKHRDLTALCKEYDELAETQGKLEEKLQELEANPPSDVYLSSRDRQILDWHFANLEFANATPLSTLSLKHWDQDDDFEFTGSHLTVRNGYSCVPVALAEGLDIKLNTAVRQVRYTASGCEVIAVNTRSTSQTFIYKCDAVLCTLPLGVLKQQPPAVQFVPPLPEWKTSAVQRMGFGNLNKVVLCFDRVFWDPSVNLFGHVGSTTASRGELFLFWNLYKAPILLALVAGEAAGIMENISDDVIVGRCLAILKGIFGSSAVPQPKETVVSRWRADPWARGSYSYVAAGSSGNDYDLMAQPITPGPSIPGAPQPIPRLFFAGEHTIRNYPATVHGALLSGLREAGRIADQFLGAMYTLPRQATPGVPAQQSPSM

SEQ ID NO: 96 - protein, 817 aa, synthetic construct
  REGION 1..817: note = Synthetic Polypeptide
SIVAQLSRPDPALAALTNDHLVALACLGGRPALDAVKKGLPHAPALIKRTNRRIPERTSHRVADHAQVVRVLGFFQCHSHPAQAFDDAMTQFGMSGGGSLPTCSCLDRVIQKDKGPYYTHLGAGPSVAAVREIMENRYGQKGNAIRIEIVVYTGKEGKSSHGCPIAKWVLRRSSDEEKVLCLVRQRTGHHCPTAVMVVLIMVWDGIPLPMADRLYTELTENLKSYNGHPTDRRCTLNENRTCTCQGIDPETCGASFSFGCSWSMYFNGCKFGRSPSPRRFRIDPSSPLHEKNLEDNLQSLATRLAPIYKQYAPVAYQNQVEYENVARECRLGSKEGRPFSGVTACLDFCAHPHRDIHNMNNGSTVVCTLTREDNRSLGVIPQDEQLHVLPLYKLSDTDEFGSKEGMEAKIKSGAIEVLAPRRKKRTCFTQPVPRSGKKRAAMMTEVLAHKIRAVEKKPIPRIKRKNNSTTTNNSKPSSLPTLGSNTETVQPEVKSETEPHFILKSSDNTKTYSLMPSAPHPVKEASPGFSWSPKTASATPAPLKNDATASCGFSERSSTPHCTMPSGRLSGANAAAADGPGISQLGEVAPLPTLSAPVMEPLINSEPSTGVTEPLTPHQPNHQPSFLTSPQDLASSPMEEDEQHSEADEPPSDEPLSDDPLSPAEEKLPHIDEYWSDSEHIFLDANIGGVAIAPAHGSVLIECARRELHATTPVEHPNRNHPTRLSLVFYQHKNLNKPQHGFELNKIKFEAKEAKNKKMKASEQKDQAANEGPEQSSEVNELNQIPSHKALTLTHDNVVTVSPYALTHVAGPYNHWV

SEQ ID NO: 97 - protein, 340 aa, X. laevis
ASSPKKKRKVEASMSRVVKPKVASMEEMAAFHTDAYLQHLHKVSEEGDNDDPETLEYGLGYDCPITEGIYDYAAAVGGATLTAAEQLIEGKTRIAVNWPGGWHHAKKDEASGFCYLNDAVLGILKLREKFDRVLYVDMDLHHGDGVEDAFSFTSKVMTVSLHKFSPGFFPGTGDVSDIGLGKGRYYSINVPLQDGIQDDKYYQICEGVLKEVFTTFNPEAVVLQLGADTIAGDPMCSFNMTPEGIGKCLKYVLQWQLPTLILGGGGYHLPNTARCWTYLTALIVGRTLSSEIPDHEFFTEYGPDYVLEITPSCRPDRNDTQKVQEILQSIKGNLKRVVEF

SEQ ID NO: 98 - protein, 331 aa, S. cerevisiae
ASSPKKKRKVEASRRVAYFYDADVGNYAYGAGHPMKPHRIRMAHSLIMNYGLYKKMEIYRAKPATKQEMCQFHTDEYIDFLSRVTPDNLEMFKRESVKFNVGDDCPVFDGLYEYCSISGGGSMEGAARLNRGKCDVAVNYAGGLHHAKKSEASGFCYLNDIVLGIIELLRYHPRVLYIDIDVHHGDGVEEAFYTTDRVMTCSFHKYGEFFPGTGELRDIGVGAGKNYAVNVPLRDGIDDATYRSVFEPVIKKIMEWYQPSAVVLQCGGDSLSGDRLGCFNLSMEGHANCVNYVKSFGIPMMVVGGGGYTMRNVARTWCFETGLLNNVVLDK

SEQ ID NO: 99 - protein, 315 aa, M. loti
ASSPKKKRKVEASMPLQIVHHPDYDAGFATNHRFPMSKYPLLMEALRARGLASPDALNTTEPAPASWLKLAHAADYVDQVISCSVPEKIEREIGFPVGPRVSLRAQLATGGTILAARLALRHGIACNTAGGSHHARRAQGAGFCTFNDVAVASLVLLDEGAAQNILVVDLDVHQGDGTADILSDEPGVFTFSMHGERNYPVRKIASDLDIALPDGTGDAAYLRRLATILPELSARARWDIVFYNAGVDVHAEDRLGRLALSNGGLRARDEMVIGHFRALGIPVCGVIGGGYSTDVPALASRHAILFEVASTYAEF

SEQ ID NO: 100 - protein, 362 aa, Homo sapiens
ASSPKKKRKVEASMLHTTQLYQHVPETRWPIVYSPRYNITFMGLEKLHPFDAGKWGKVINFLKEEKLLSDSMLVEAREASEEDLLVVHTRRYLNELKWSFAVATITEIPPVIFLPNFLVQRKVLRPLRTQTGGTIMAGKLAVERGWAINVGGGFHHCSSDRGGGFCAYADITLAIKFLFERVEGISRATIIDLDAHQGNGHERDFMDDKRVYIMDVYNRHIYPGDRFAKQAIRRKVELEWGTEDDEYLDKVERNIKKSLQEHLPDVVVYNAGTDILEGDRLGGLSISPAGIVKRDELVFRMVRGRRVPILMVTSGGYQKRTARIIADSILNLFGLGLIGPESPSVSAQNSDTPLLPPAVPEF

SEQ ID NO: 101 - protein, 226 aa, A. thaliana
ASSPKKKRKVEASMEFWGIEVKSGKPVTVTPEEGILIHVSQASLGECKNKKGEFVPLHVKVGNQNLVLGTLSTENIPQLFCDLVFDKEFELSHTWGKGSVYFVGYKTPNIEPQGYSEEEEEEEEEVPAGNAAKAVAKPKAKPAEVKPAVDDEEDESDSDGMDEDDSDGEDSEEEEPTPKKPASSKKRANETTPKAPVSAKKAKVAVTPQKTDEKKKGGKAANQSEF

SEQ ID NO: 102 - protein, 272 aa, Homo sapiens
ASSPKKKRKVEASMVGAGISTPSGIPDFRSPGSGLYSNLQQYDLPYPEAIFELPFFFHNPKPFFTLAKELYPGNYKPNVTHYFLRLLHDKGLLLRLYTQNIDGLERVSGIPASKLVEAHGTFASATCTVCQRPFPGEDIRADVMADRVPRCPVCTGVVKPDIVFFGEPLPQRFLLHVVDFPMADLLLILGTSLEVEPFASLTEAVRSSVPRLLINRDLVGPLAWHPRSRDVAQLGDVVHGVESLVELLGWTEEMRDLVQRETGKLDGPDKEF

SEQ ID NO: 103 - protein, 306 aa, S. cerevisiae
ASSPKKKRKVEASTEMSVRKIAAHMKSNPNAKVIFMVGAGISTSCGIPDFRSPGTGLYHNLARLKLPYPEAVFDVDFFQSDPLPFYTLAKELYPGNFRPSKFHYLLKLFQDKDVLKRVYTQNIDTLERQAGVKDDLIIEAHGSFAHCHCIGCGKVYPPQVFKSKLAEHPIKDFVKCDVCGELVKPAIVFFGEDLPDSFSETWLNDSEWLREKITTSGKHPQQPLVIVVGTSLAVYPFASLPEEIPRKVKRVLCNLETVGDFKANKRPTDLIVHQYSDEFAEQLVEELGWQEDFEKILTAQGGMGEF

SEQ ID NO: 104 - protein, 257 aa, E. coli
ASSPKKKRKVEASMEKPRVLVLTGAGISAESGIRTFRAADGLWEEHRVEDVATPEGFDRDPELVQAFYNARRRQLQQPEIQPNAAHLALAKLQDALGDRFLLVTQNIDNLHERAGNTNVIHMHGELLKVRCSQSGQVLDWTGDVTPEDKCHCCQFPAPLRPHVVWFGEMPLGMDEIYMALSMADIFIAIGTSGHVYPAAGFVHEAKLHGAHTVELNLEPSQVGNEFAEKYYGPASQVVPEFVEKLLKGLKAGSIAEF

SEQ ID NO: 105 - protein, 346 aa, C. albicans
ASSPKKKRKVEASMPSLDDILKPVAEAVKNGKKVTFFNGAGISTGAGIPDFRSPDTGLYANLAKLNLPFAEAVFDIDFFKEDPKPFYTLAEELYPGNFAPTKFHHFIKLLQDQGSLKRVYTQNIDTLERLAGVEDKYIVEAHGSFASNHCVDCHKEMTTETLKTYMKDKKIPSCQHCEGYVKPDIVFFGEGLPVKFFDLWEDDCEDVEVAIVAGTSLTVFPFASLPGEVNKKCLRVLVNKEKVGTFKHEPRKSDIIALHDCDIVAERLCTLLGLDDKLNEVYEKEKIKYSKAETKEIKMHEIEDKLKEEAHLKEDKHTTKVDKKEKQNDANDKELEQLIDKAKAEF

SEQ ID NO: 106 - protein, 289 aa, Homo sapiens
ASSPKKKRKVEASSSSMADFRKFFAKAKHIVIISGAGVSAESGVPTFRGAGGYWRKWQAQDLATPLAFAHNPSRVWEFYHYRREVMGSKEPNAGHRAIAECETRLGKQGRRVVVITQNIDELHRKAGTKNLLEIHGSLFKTRCTSCGVVAENYKSPICPALSGKGAPEPGTQDASIPVEKLPRCEEAGCGGLLRPHVVWFGENLDPAILEEVDRELAHCDLCLVVGTSSVVYPAAMFAPQVAARGVPVAEFNTETTPATNRFRFHFQGPCGTTLPEALACHENETVSEF

SEQ ID NO: 107 - protein, 288 aa, P. falciparum
ASSPKKKRKVEASMGNLMISFLKKDTQSITLEELAKIIKKCKHVVALTGSGTSAESNIPSFRGSSNSIWSKYDPRIYGTIWGFWKYPEKIWEVIRDISSDYEIEINNGHVALSTLESLGYLKSVVTQNVDGLHEASGNTKVISLHGNVFEAVCCTCNKIVKLNKIMLQKTSHFMHQLPPECPCGGIFKPNIILFGEVVSSDLLKEAEEEIAKCDLLLVIGTSSTVSTATNLCHFACKKKKKIVEINISKTYITNKMSDYHVCAKFSELTKVANILKGSSEKNKKIMEF

SEQ ID NO: 108 - protein, 304 aa, Homo sapiens
ASSPKKKRKVEASMSVNYAAGLSPYADKGKCGLPEIFDPPEELERKVWELARLVWQSSSVVFHTGAGISTASGIPDFRGPHGVWTMEERGLAPKFDTTFESARPTQTHMALVQLERVGLLRFLVSQNVDGLHVRSGFPRDKLAELHGNMFVEECAKCKTQYVRDTVVGTMGLKATGRLCTVAKARGLRACRGELRDTILDWEDSLPDRDLALADEASRNADLSITLGTSLQIRPSGNLPLATKRRGGRLVIVNLQPTKHDRHADLRIHGYVDEVMTRLMKHLGLEIPAWDGPRVLERALPPLEF

SEQ ID NO: 109 - protein, 234 aa, C. trachomatis
ASSPKKKRKVEASMTTNSTQDTLYLSLHGGIDSAIPYPVRRVEQLLQFSFLPELQFQNAAVKQRIQRLCYREEKRLAVSSLAKWLGQLHKQRLRAPKNPPVAICWINSYVGYGVFARESIPAWSYIGEYTGILRRRQALWLDENDYCFRYPVPRYSFRYFTIDSGMQGNVTRFINHSDNPNLEAIGAFENGIFHIIIRAIKDILPGEELCYHYGPLYWKHRKKREEFVPQEEEF

SEQ ID NO: 110 - protein, 134 aa, P. bursaria chlorella virus
ASSPKKKRKVEASMFNDRVIVKKSPLGGYGVFARKSFEKGELVEECLCIVRHNDDWGTALEDYLFSRKNMSAMALGFGAIFNHSKDPNARHELTAGLKRMRIFTIKPIAIGEEITISYGDDYWLSRPRLTQNEF

SEQ ID NO: 111 - protein, 349 aa, Homo sapiens
ASSPKKKRKVEASNLKCVRILKQFHKDLERELLRRHHRSKTPRHLDPSLANYLVQKAKQRRALRRWEQELNAKRSHLGRITVENEVDLDGPPRAFVYINEYRVGEGITLNQVAVGCECQDCLWAPTGGCCPGASLHKFAYNDQGQVRLRAGLPIYECNSRCRCGYDCPNRVVQKGIRYDLCIFRTDDGRGWGVRTLEKIRKNSFVMEYVGEIITSEEAERRGQIYDRQGATYLFDLDYVEDVYTVDAAYYGNISHFVNHSCDPNLQVYNVFIDNLDERLPRIAFFATRTIRAGEELTFDYNMQVDPVDMESTRMDSNFGLAGLPGSPKKRVRIECKCGTESCRKYLFEF

SEQ ID NO: 112 - protein, 346 aa, N. crassa
ASSPKKKRKVEASMEKAFRPHFFNHGKPDANPKEKKNCHWCQIRSFATHAQLPISIVNREDDAFLNPNFRFIDHSIIGKNVPVADQSFRVGCSCASDEECMYSTCQCLDEMAPDSDEEADPYTRKKRFAYYSQGAKKGLLRDRVLQSQEPIYECHQGCACSKDCPNRVVERGRTVPLQIFRTKDRGWGVKCPVNIKRGQFVDRYLGEIITSEEADRRRAESTIARRKDVYLFALDKFSDPDSLDPLLAGQPLEVDGEYMSGPTRFINHSCDPNMAIFARVGDHADKHIHDLALFAIKDIPKGTELTFDYVNGLTGLESDAHDPSKISEMTKCLCGTAKCRGYLWEF

SEQ ID NO: 113 - protein, 282 aa, A. thaliana
ASSPKKKRKVEASDISGGLEFKGIPATNRVDDSPVSPTSGFTYIKSLIIEPNVIIPKSSTGCNCRGSCTDSKKCACAKLNGGNFPYVDLNDGRLIESRDVVFECGPHCGCGPKCVNRTSQKRLRFNLEVFRSAKKGWAVRSWEYIPAGSPVCEYIGVVRRTADVDTISDNEYIFEIDCQQTMQGLGGRQRRLRDVAVPMNNGVSQSSEDENAPEFCIDAGSTGNFARFINHSCEPNLFVQCVLSSHQDIRLARVVLFAADNISPMQELTYDYGYALDSVHEF

SEQ ID NO: 114 - protein, 328 aa, A. thaliana
ASSPKKKRKVEASQSAYLHVSLARISDEDCCANCKGNCLSADFPCTCARETSGEYAYTKEGLLKEKFLDTCLKMKKEPDSFPKVYCKDCPLERDHDKGTYGKCDGHLIRKFIKECWRKCGCDMQCGNRVVQRGIRCQLQVYFTQEGKGWGLRTLQDLPKGTFICEYIGEILTNTELYDRNVRSSSERHTYPVTLDADWGSEKDLKDEEALCLDATICGNVARFINHRCEDANMIDIPIEIETPDRHYYHIAFFTLRDVKAMDELTWDYMIDFNDKSHPVKAFRCCCGSESCRDRKIKGSQGKSIERRKIVSAKKQQGSKEVSKKRKEF

SEQ ID NO: 115 - protein, 303 aa, C. elegans
ASSPKKKRKVEASMQLHEQIANISVTFNDIPRSDHSMTPTELCYFDDFATTLVVDSVLNFTTHKMSKKRRYLYQDEYRTARTVMKTFREQRDWTNAIYGLLTLRSVSHFLSKLPPNKLFEFRDHIVRFLNMFILDSGYTIQECKRYSQEGHQGAKLVSTGVWSRGDKIERLSGVVCLLSSEDEDSILAQEGSDFSVMYSTRKRCSTLWLGPGAYINHDCRPTCEFVSHGSTAHIRVLRDMVPGDEITCFYGSEFFGPNNIDCECCTCEKNMNGAFSYLRGNENAEPIISEKKTKYELRSRSEF

SEQ ID NO: 116 - protein, 257 aa, C. elegans
ASSPKKKRKVEASMKVAAKKLATSRMRKDRAAAASPSSDIENSENPSSLASHSSSSGRMTPSKNTRSRKGVSVKDVSNHKITEFFQVRRSNRKTSKQISDEAKHALRDTVLKGTNERLLEVYKDVVKGRGIRTKVNFEKGDFVVEYRGVMMEYSEAKVIEEQYSNDEEIGSYMYFFEHNNKKWCIDATKESPWKGRLINHSVLRPNLKTKVVEIDGSHHLILVARRQIAQGEELLYDYGDRSAETIAKNPWLVNTEF

SEQ ID NO: 117 - protein, 224 aa, Homo sapiens
ASSPKKKRKVEASSCDSTNAAIAKQALKKPIKGKQAPRKKAQGKTQQNRKLTDFYPVRRSSRKSKAELQSEERKRIDELIESGKEEGMKIDLIDGKGRGVIATKQFSRGDFVVEYHGDLIEITDAKKREALYAQDPSTGCYMYYFQYLSKTYCVDATRETNRLGRLINHSKCGNCQTKLHDIDGVPHLILIASRDIAAGEELLYDYGDRSKASIEAFPWLKHEF

SEQ ID NO: 118 - protein, 319 aa, T. gondii
ASSPKKKRKVEASASRRTGEFLRDAQAPSRWLKRSKTGQDDGAFCLETWLAGAGDDAAGGERGRDREGAADKAKQREERRQKELEERFEEMKVEFEEKAQRMIARRAALTGEIYSDGKGSKKPRVPSLPENDDDALIEIIIDPEQGILKWPLSVMSIRQRTVIYQECLRRDLTACIHLTKVPGKGRAVFAADTILKDDFVVEYKGELCSEREAREREQRYNRSKVPMGSFMFYFKNGSRMMAIDATDEKQDFGPARLINHSRRNPNMTPRAITLGDFNSEPRLIFVARRNIEKGEELLVDYGERDPDVIKEHPWLNSEF

SEQ ID NO: 119 - DNA, 20 bp, synthetic construct
  misc_feature 1..20: note = Synthetic Polynucleotide
  source 1..20: mol_type = other DNA
ggcctgcttcgtggcaatgc

SEQ ID NO: 120 - DNA, 20 bp, synthetic construct
  misc_feature 1..20: note = Synthetic Polynucleotide
  source 1..20: mol_type = other DNA
acctgggccagggagggagg

SEQ ID NO: 121 - DNA, 20 bp, synthetic construct
  misc_feature 1..20: note = Synthetic Polynucleotide
  source 1..20: mol_type = other DNA
ctcacttagactttctctcc

SEQ ID NO: 122 - DNA, 20 bp, synthetic construct
  misc_feature 1..20: note = Synthetic Polynucleotide
  source 1..20: mol_type = other DNA
ctcggagtctagctcctgca

SEQ ID NO: 123 - DNA, 20 bp, synthetic construct
  misc_feature 1..20: note = Synthetic Polynucleotide
  source 1..20: mol_type = other DNA
tggccccagtctctcttcta

SEQ ID NO: 124 - DNA, 20 bp, synthetic construct
  misc_feature 1..20: note = Synthetic Polynucleotide
  source 1..20: mol_type = other DNA
cagcctctgaacagctcccg

SEQ ID NO: 125 - DNA, 20 bp, synthetic construct
  misc_feature 1..20: note = Synthetic Polynucleotide
  source 1..20: mol_type = other DNA
tgacttggcctttgtaggaa

SEQ ID NO: 126 - DNA, 20 bp, synthetic construct
  misc_feature 1..20: note = Synthetic Polynucleotide
  source 1..20: mol_type = other DNA
gaggctactgaaacataagt

SEQ ID NO: 127 - DNA, 20 bp, synthetic construct
  misc_feature 1..20: note = Synthetic Polynucleotide
  source 1..20: mol_type = other DNA
tgctacctgtacatctgcac

SEQ ID NO: 128 - DNA, 20 bp, synthetic construct
  misc_feature 1..20: note = Synthetic Polynucleotide
  source 1..20: mol_type = other DNA
catcaatgattgggcatttc

SEQ ID NO: 129 - DNA, 20 bp, synthetic construct
  misc_feature 1..20: note = Synthetic Polynucleotide
  source 1..20: mol_type = other DNA
actccagtcccaaatatgta

SEQ ID NO: 130 - DNA, 20 bp, synthetic construct
  misc_feature 1..20: note = Synthetic Polynucleotide
  source 1..20: mol_type = other DNA
actagggggcgctcggccac

SEQ ID NO: 131 - DNA, 20 bp, synthetic construct
  misc_feature 1..20: note = Synthetic Polynucleotide
  source 1..20: mol_type = other DNA
ctgagtcaactgtaagcatt

SEQ ID NO: 132 - DNA, 20 bp, synthetic construct
  misc_feature 1..20: note = Synthetic Polynucleotide
  source 1..20: mol_type = other DNA
ggccaggtgcagtgattcat

SEQ ID NO: 133 - DNA, 20 bp, synthetic construct
  misc_feature 1..20: note = Synthetic Polynucleotide
  source 1..20: mol_type = other DNA
tcgtgtcatcttgtttgtgc

SEQ ID NO: 134 - DNA, 20 bp, synthetic construct
  misc_feature 1..20: note = Synthetic Polynucleotide
  source 1..20: mol_type = other DNA
ggcagagcccagcggacact

SEQ ID NO: 135 - DNA, 20 bp, synthetic construct
  misc_feature 1..20: note = Synthetic Polynucleotide
  source 1..20: mol_type = other DNA
caaggtgagcctgggtctgt

SEQ ID NO: 136 - DNA, 20 bp, synthetic construct
  misc_feature 1..20: note = Synthetic Polynucleotide
  source 1..20: mol_type = other DNA
atcactgcccaagaagtgca

SEQ ID NO: 137 - DNA, 20 bp, synthetic construct
  misc_feature 1..20: note = Synthetic Polynucleotide
  source 1..20: mol_type = other DNA
ttgtaggatgtttagcagca

SEQ ID NO: 138 - DNA, 20 bp, synthetic construct
  misc_feature 1..20: note = Synthetic Polynucleotide
  source 1..20: mol_type = other DNA
acttgctctctttagagaac

SEQ ID NO: 139 - DNA, 20 bp, synthetic construct
  misc_feature 1..20: note = Synthetic Polynucleotide
  source 1..20: mol_type = other DNA
ctcaagcaggccccgctggt

SEQ ID NO: 140 - DNA, 20 bp, synthetic construct
  misc_feature 1..20: note = Synthetic Polynucleotide
  source 1..20: mol_type = other DNA
ttttggaccaaacctttttg

SEQ ID NO: 141 - DNA, 20 bp, synthetic construct
  misc_feature 1..20: note = Synthetic Polynucleotide
  source 1..20: mol_type = other DNA
tgaggttatttgtccattgt

SEQ ID NO: 142 - DNA, 20 bp, synthetic construct
  misc_feature 1..20: note = Synthetic Polynucleotide
  source 1..20: mol_type = other DNA
taaggggagtatttacacca

SEQ ID NO: 143 - DNA, 20 bp, synthetic construct
  misc_feature 1..20: note = Synthetic Polynucleotide
  source 1..20: mol_type = other DNA
tcaagagcagaaaatgtgac

SEQ ID NO: 144 - DNA, 20 bp, synthetic construct
  misc_feature 1..20: note = Synthetic Polynucleotide
  source 1..20: mol_type = other DNA
cttgcagggaccttctgatt

SEQ ID NO: 145 - DNA, 20 bp, synthetic construct
  misc_feature 1..20: note = Synthetic Polynucleotide
  source 1..20: mol_type = other DNA
tgtgtgtaggactaaactct

SEQ ID NO: 146 - DNA, 20 bp, synthetic construct
  misc_feature 1..20: note = Synthetic Polynucleotide
  source 1..20: mol_type = other DNA
gatagcagtatgaccttggg

SEQ ID NO: 147 - DNA, 20 bp, synthetic construct
  misc_feature 1..20: note = Synthetic Polynucleotide
  source 1..20: mol_type = other DNA
agcgtgtccggcgagggcga

SEQ ID NO: 148 - DNA, 20 bp, synthetic construct
  misc_feature 1..20: note = Synthetic Polynucleotide
  source 1..20: mol_type = other DNA
agcgtgtccggcgagggcga

SEQ ID NO: 149 - DNA, 25 bp, synthetic construct
  misc_feature 1..25: note = Synthetic Polynucleotide
  source 1..25: mol_type = other DNA
cagaatcggaggacaaaatacaaac

SEQ ID NO: 150 - DNA, 25 bp, synthetic construct
  misc_feature 1..25: note = Synthetic Polynucleotide
  source 1..25: mol_type = other DNA
acgaagcaggccaacggggaggaca

SEQ ID NO: 151 - DNA, 37 bp, synthetic construct
  misc_feature 1..37: note = Synthetic Polynucleotide
  source 1..37: mol_type = other DNA
taatacgactcactatagggcacgggcagcttgccgg

SEQ ID NO: 152 - DNA, 55 bp, synthetic construct
  misc_feature 1..55: note = Synthetic Polynucleotide
  source 1..55: mol_type = other DNA
taatacgactcactataggcctcgaacttcacctcggcggaaaggacgaaacacc

SEQ ID NO: 153 - DNA, 54 bp, synthetic construct
  misc_feature 1..54: note = Synthetic Polynucleotide
  source 1..54: mol_type = other DNA
taatacgactcactataggctgaagggcatcgacttcagaaaggacgaaacacc

SEQ ID NO: 154 - DNA, 55 bp, synthetic construct
  misc_feature 1..55: note = Synthetic Polynucleotide
  source 1..55: mol_type = other DNA
taatacgactcactataggcagctcgatgcggttcaccagaaaggacgaaacacc

SEQ ID NO: 155 - DNA, 55 bp, synthetic construct
  misc_feature 1..55: note = Synthetic Polynucleotide
  source 1..55: mol_type = other DNA
taatacgactcactataggcaaggaggacggcaacatccgaaaggacgaaacacc

SEQ ID NO: 156 - DNA, 54 bp, synthetic construct
  misc_feature 1..54: note = Synthetic Polynucleotide
  source 1..54: mol_type = other DNA
taatacgactcactataggagtccgagcagaagaagaagaaaggacgaaacacc

SEQ ID NO: 157 - DNA, 54 bp, synthetic construct
  misc_feature 1..54: note = Synthetic Polynucleotide
  source 1..54: mol_type = other DNA
taatacgactcactataggggtggggggagtttgctccgaaaggacgaaacacc

SEQ ID NO: 158 - DNA, 54 bp, synthetic construct
  misc_feature 1..54: note = Synthetic Polynucleotide
  source 1..54: mol_type = other DNA
taatacgactcactataggcagatgtagtgtttccacagaaaggacgaaacacc

SEQ ID NO: 159 - DNA, 21 bp, synthetic construct
  misc_feature 1..21: note = Synthetic Polynucleotide
  source 1..21: mol_type = other DNA
aaaaaaagcaccgactcggtg

SEQ ID NO: 160 - DNA, 22 bp, synthetic construct
  misc_feature 1..22: note = Synthetic Polynucleotide
  source 1..22: mol_type = other DNA
ctgtacaaaaaagcaggcttta

SEQ ID NO: 161 - DNA, 83 bp, synthetic construct
  misc_feature 1..83: note = Synthetic Polynucleotide
  source 1..83: mol_type = other DNA
aaaaaaagcaccgactcggtgccactttttcaagttgataacggactagccttattttaacttgctatttctagctctaaaac

SEQ ID NO: 162 - DNA, 60 bp, synthetic construct
  misc_feature 1..60: note = Synthetic Polynucleotide
  source 1..60: mol_type = other DNA
gaaaggacgaaacaccggcctcgaacttcacctcggcggttttagagctagaaatagcaa

SEQ ID NO: 163 - DNA, 60 bp, synthetic construct
  misc_feature 1..60: note = Synthetic Polynucleotide
  source 1..60: mol_type = other DNA
gaaaggacgaaacaccggcagctcgatgcggttcaccagttttagagctagaaatagcaa

SEQ ID NO: 164 - DNA, 59 bp, synthetic construct
  misc_feature 1..59: note = Synthetic Polynucleotide
  source 1..59: mol_type = other DNA
gaaaggacgaaacaccggctgaagggcatcgacttcagttttagagctagaaatagcaa

SEQ ID NO: 165 - DNA, 60 bp, synthetic construct
  misc_feature 1..60: note = Synthetic Polynucleotide
  source 1..60: mol_type = other DNA
gaaaggacgaaacaccggcaaggaggacggcaacatccgttttagagctagaaatagcaa

SEQ ID NO: 166 - DNA, 59 bp, synthetic construct
  misc_feature 1..59: note = Synthetic Polynucleotide
  source 1..59: mol_type = other DNA
gaaaggacgaaacaccggcagatgtagtgtttccacagttttagagctagaaatagcaa

SEQ ID NO: 167 - DNA, 59 bp, synthetic construct
  misc_feature 1..59: note = Synthetic Polynucleotide
  source 1..59: mol_type = other DNA
gaaaggacgaaacaccggagtccgagcagaagaagaagttttagagctagaaatagcaa

SEQ ID NO: 168 - DNA, 59 bp, synthetic construct
  misc_feature 1..59: note = Synthetic Polynucleotide
  source 1..59: mol_type = other DNA
gaaaggacgaaacaccggggtggggggagtttgctccgttttagagctagaaatagcaa

SEQ ID NO: 169 - DNA, 20 bp, synthetic construct
  misc_feature 1..20: note = Synthetic Polynucleotide
  source 1..20: mol_type = other DNA
tacggcaagctgaccctgaa

SEQ ID NO: 170 - DNA, 20 bp, synthetic construct
  misc_feature 1..20: note = Synthetic Polynucleotide
  source 1..20: mol_type = other DNA
gtccatgccgagagtgatcc

SEQ ID NO: 171 - DNA, 20 bp, synthetic construct
  misc_feature 1..20: note = Synthetic Polynucleotide
  source 1..20: mol_type = other DNA
gccaggggctgttatcttgg

SEQ ID NO: 172 - DNA, 21 bp, synthetic construct
  misc_feature 1..21: note = Synthetic Polynucleotide
  source 1..21: mol_type = other DNA
atgcacagaagcacaggttga

SEQ ID NO: 173 - DNA, 20 bp, synthetic construct
  misc_feature 1..20: note = Synthetic Polynucleotide
  source 1..20: mol_type = other DNA
ctgtgtcctcttcctgccct

SEQ ID NO: 174 - DNA, 20 bp, synthetic construct
  misc_feature 1..20: note = Synthetic Polynucleotide
  source 1..20: mol_type = other DNA
ctctccgaggagaaggccaa

SEQ ID NO: 175 - DNA, 20 bp, synthetic construct
  misc_feature 1..20: note = Synthetic Polynucleotide
  source 1..20: mol_type = other DNA
ccacacagcttcccgttctc

SEQ ID NO: 176 - DNA, 20 bp, synthetic construct
  misc_feature 1..20: note = Synthetic Polynucleotide
  source 1..20: mol_type = other DNA
gagagccgttccctctttgc

SEQ ID NO: 177 - DNA, 52 bp, synthetic construct
  misc_feature 1..52: note = Synthetic Polynucleotide
  source 1..52: mol_type = other DNA
cactctttccctacacgacgctcttccgatctcctccccattggcctgcttc

SEQ ID NO: 178 - DNA, 53 bp, synthetic construct
  misc_feature 1..53: note = Synthetic Polynucleotide
  source 1..53: mol_type = other DNA
cactctttccctacacgacgctcttccgatcttcgtcctgctctcacttagac

SEQ ID NO: 179 - DNA, 52 bp, synthetic construct
  misc_feature 1..52: note = Synthetic Polynucleotide
  source 1..52: mol_type = other DNA
cactctttccctacacgacgctcttccgatctttttgtggcttggccccagt

SEQ ID NO: 180 - DNA, 53 bp, synthetic construct
  misc_feature 1..53: note = Synthetic Polynucleotide
  source 1..53: mol_type = other DNA
cactctttccctacacgacgctcttccgatcttgcagtctcatgacttggcct

SEQ ID NO: 181 - DNA, 52 bp, synthetic construct
  misc_feature 1..52: note = Synthetic Polynucleotide
  source 1..52: mol_type = other DNA
cactctttccctacacgacgctcttccgatctttctgagggctgctacctgt

SEQ ID NO: 182 - DNA, 54 bp, synthetic construct
  misc_feature 1..54: note = Synthetic Polynucleotide
  source 1..54: mol_type = other DNA
cactctttccctacacgacgctcttccgatctacatgaagcaactccagtccca

SEQ ID NO: 183 - DNA, 54 bp, synthetic construct
  misc_feature 1..54: note = Synthetic Polynucleotide
  source 1..54: mol_type = other DNA
cactctttccctacacgacgctcttccgatctagcagacccactgagtcaactg

SEQ ID NO: 184 - DNA, 51 bp, synthetic construct
  misc_feature 1..51: note = Synthetic Polynucleotide
  source 1..51: mol_type = other DNA
cactctttccctacacgacgctcttccgatctcccgccacagtcgtgtcat

SEQ ID NO: 185 - DNA, 50 bp, synthetic construct
  misc_feature 1..50: note = Synthetic Polynucleotide
  source 1..50: mol_type = other DNA
cactctttccctacacgacgctcttccgatctcgccccggtacaaggtga

SEQ ID NO: 186 - DNA, 55 bp, synthetic construct
  misc_feature 1..55: note = Synthetic Polynucleotide
  source 1..55: mol_type = other DNA
cactctttccctacacgacgctcttccgatctgtaccgtacattgtaggatgttt

SEQ ID NO: 187 - DNA, 53 bp, synthetic construct
  misc_feature 1..53: note = Synthetic Polynucleotide
  source 1..53: mol_type = other DNA
cactctttccctacacgacgctcttccgatctcctcatctccctcaagcaggc

SEQ ID NO: 188 - DNA, 55 bp, synthetic construct
  misc_feature 1..55: note = Synthetic Polynucleotide
  source 1..55: mol_type = other DNA
cactctttccctacacgacgctcttccgatctattctgctcttgaggttatttgt

SEQ ID NO: 189 - DNA, 56 bp, synthetic construct
  misc_feature 1..56: note = Synthetic Polynucleotide
  source 1..56: mol_type = other DNA
cactctttccctacacgacgctcttccgatctcacctctgcctcaagagcagaaaa

SEQ ID NO: 190 - DNA, 55 bp, synthetic construct
  misc_feature 1..55: note = Synthetic Polynucleotide
  source 1..55: mol_type = other DNA
cactctttccctacacgacgctcttccgatcttgtgtgtgtgtgtgtgtaggact

SEQ ID NO: 191 - DNA, 48 bp, synthetic construct
  misc_feature 1..48: note = Synthetic Polynucleotide
  source 1..48: mol_type = other DNA
ggagttcagacgtgtgctcttccgatcttcatctgtgcccctccctcc

SEQ ID NO: 192 - DNA, 47 bp, synthetic construct
  misc_feature 1..47: note = Synthetic Polynucleotide
  source 1..47: mol_type = other DNA
ggagttcagacgtgtgctcttccgatctcgagaaggaggtgcaggag

SEQ ID NO: 193 - DNA, 48 bp, synthetic construct
  misc_feature 1..48: note = Synthetic Polynucleotide
  source 1..48: mol_type = other DNA
ggagttcagacgtgtgctcttccgatctcgggagctgttcagaggctg

SEQ ID NO: 194 - DNA, 48 bp, synthetic construct
  misc_feature 1..48: note = Synthetic Polynucleotide
  source 1..48: mol_type = other DNA
ggagttcagacgtgtgctcttccgatctctcacctgggcgagaaaggt

SEQ ID NO: 195 - DNA, 52 bp, synthetic construct
  misc_feature 1..52: note = Synthetic Polynucleotide
  source 1..52: mol_type = other DNA
ggagttcagacgtgtgctcttccgatctaaaactcaaagaaatgcccaatca

SEQ ID NO: 196 - DNA, 48 bp, synthetic construct
  misc_feature 1..48: note = Synthetic Polynucleotide
  source 1..48: mol_type = other DNA
ggagttcagacgtgtgctcttccgatctagacgctgctcgctccattc

SEQ ID NO: 197 - DNA, 50 bp, synthetic construct
  misc_feature 1..50: note = Synthetic Polynucleotide
  source 1..50: mol_type = other DNA
ggagttcagacgtgtgctcttccgatctacaggcatgaatcactgcacct

SEQ ID NO: 198 - DNA, 49 bp, synthetic construct
  misc_feature 1..49: note = Synthetic Polynucleotide
  source 1..49: mol_type = other DNA
ggagttcagacgtgtgctcttccgatctgcggcaacttcagacaaccga

SEQ ID NO: 199 - DNA, 46 bp, synthetic construct
  misc_feature 1..46: note = Synthetic Polynucleotide
  source 1..46: mol_type = other DNA
ggagttcagacgtgtgctcttccgatctgacccaggggcaccagtt

SEQ ID NO: 200 - DNA, 53 bp, synthetic construct
  misc_feature 1..53: note = Synthetic Polynucleotide
  source 1..53: mol_type = other DNA
ggagttcagacgtgtgctcttccgatctctgccttcattgcttaaaagtggat

SEQ ID NO: 201 - DNA, 51 bp, synthetic construct
  misc_feature 1..51: note = Synthetic Polynucleotide
  source 1..51: mol_type = other DNA
ggagttcagacgtgtgctcttccgatctacagttgaaggaaggaaacatgc

SEQ ID NO: 202 - DNA, 48 bp, synthetic construct
  misc_feature 1..48: note = Synthetic Polynucleotide
  source 1..48: mol_type = other DNA
ggagttcagacgtgtgctcttccgatctgctgcatttgcccatttcca

SEQ ID NO: 203 - DNA, 49 bp, synthetic construct
  misc_feature 1..49: note = Synthetic Polynucleotide
  source 1..49: mol_type = other DNA
ggagttcagacgtgtgctcttccgatctgttgggggaggaggagcttat

SEQ ID NO: 204 - DNA, 53 bp, synthetic construct
  misc_feature 1..53: note = Synthetic Polynucleotide
  source 1..53: mol_type = other DNA
ggagttcagacgtgtgctcttccgatctctaagagctataagggcaaatgact

SEQ ID NO: 205 - DNA, 56 bp, synthetic construct
  misc_feature 1..56: note = Synthetic Polynucleotide
  misc_feature 33..36: note = n is a, c, g, or t
  source 1..56: mol_type = other DNA
cactctttccctacacgacgctcttccgatctnnnnacgtaaacggccacaagttc

SEQ ID NO: 206 - DNA, 50 bp, synthetic construct
  misc_feature 1..50: note = Synthetic Polynucleotide
  source 1..50: mol_type = other DNA
ggagttcagacgtgtgctcttccgatctgtcgtccttgaagaagatggtg

SEQ ID NO: 207 - DNA, 54 bp, synthetic construct
  misc_feature 1..54: note = Synthetic Polynucleotide
  source 1..54: mol_type = other DNA
cactctttccctacacgacgctcttccgatctccaggtgaaggtgtggttccag

SEQ ID NO: 208 - DNA, 49 bp, synthetic construct
  misc_feature 1..49: note = Synthetic Polynucleotide
  source 1..49: mol_type = other DNA
ggagttcagacgtgtgctcttccgatctcccctagtcattggaggtgac

SEQ ID NO: 209 - DNA, 23 bp, synthetic construct
  misc_feature 1..23: note = Synthetic Polynucleotide
  source 1..23: mol_type = other DNA
gagtccgagcagaagaagaaggg

SEQ ID NO: 210 - DNA, 23 bp, synthetic construct
  misc_feature 1..23: note = Synthetic Polynucleotide
  source 1..23: mol_type = other DNA
gaggccgagcagaagaaagacgg

SEQ ID NO: 211 - DNA, 23 bp, synthetic construct
  misc_feature 1..23: note = Synthetic Polynucleotide
  source 1..23: mol_type = other DNA
gagtcctagcaggagaagaagag

SEQ ID NO: 212 - DNA, 23 bp, synthetic construct
  misc_feature 1..23: note = Synthetic Polynucleotide
  source 1..23: mol_type = other DNA
gagtctaagcagaagaagaagag

SEQ ID NO: 213 - DNA, 23 bp, synthetic construct
  misc_feature 1..23: note = Synthetic Polynucleotide
  source 1..23: mol_type = other DNA
gagttagagcagaagaagaaagg

SEQ ID NO: 214 - DNA, 23 bp, synthetic construct
  misc_feature 1..23: note = Synthetic Polynucleotide
  source 1..23: mol_type = other DNA
gggtggggggagtttgctcctgg

SEQ ID NO: 215 - DNA, 23 bp, synthetic construct
  misc_feature 1..23: note = Synthetic Polynucleotide
  source 1..23: mol_type = other DNA
ggatggagggagtttgctcctgg

SEQ ID NO: 216 - DNA, 23 bp, synthetic construct
  misc_feature 1..23: note = Synthetic Polynucleotide
  source 1..23: mol_type = other DNA
gggagggtggagtttgctcctgg

SEQ ID NO: 217 - DNA, 23 bp, synthetic construct
  misc_feature 1..23: note = Synthetic Polynucleotide
  source 1..23: mol_type = other DNA
cgggggagggagtttgctcctgg

SEQ ID NO: 218 - DNA, 23 bp, synthetic construct
  misc_feature 1..23: note = Synthetic Polynucleotide
  source 1..23: mol_type = other DNA
ggggaggggaagtttgctcctgg

SEQ ID NO: 219 - DNA, 23 bp, synthetic construct
  misc_feature 1..23: note = Synthetic Polynucleotide
  source 1..23: mol_type = other DNA
gcagatgtagtgtttccacaggg

SEQ ID NO: 220 - DNA, 23 bp, synthetic construct
  misc_feature 1..23: note = Synthetic Polynucleotide
  source 1..23: mol_type = other DNA
acaaatgtagtatttccacaggg

SEQ ID NO: 221 - DNA, 23 bp, synthetic construct
  misc_feature 1..23: note = Synthetic Polynucleotide
  source 1..23: mol_type = other DNA
ccagatgtagtattcccacaggg

SEQ ID NO: 222 - DNA, 23 bp, synthetic construct
  misc_feature 1..23: note = Synthetic Polynucleotide
  source 1..23: mol_type = other DNA
ctagatgaagtgcttccacatgg

SEQ ID NO: 223 - DNA, 133 bp, synthetic construct
  misc_feature 1..133: note = Synthetic Polynucleotide
  source 1..133: mol_type = other DNA
gggcgatgccacctacggcaagctgaccctgaagttcatctgcaccaccggcaagctgcccgtgccctggcccaccctcgtgaccaccctgacctacggcgtgcagtgcttcagccgctaccccgaccacatg

SEQ ID NO: 224 - DNA, 44 bp, synthetic construct
  misc_feature 1..44: note = Synthetic Polynucleotide
  source 1..44: mol_type = other DNA
gggcgatcggcgtgcagtgcttcagccgctaccccgaccacatg

SEQ ID NO: 225 - DNA, 60 bp, synthetic construct
  misc_feature 1..60: note = Synthetic Polynucleotide
  source 1..60: mol_type = other DNA
gggcgatgccacctacggcaagctgaccctgaagttcatctgcaccaccgcgaccacatg

SEQ ID NO: 226 - DNA, 131 bp, synthetic construct
  misc_feature 1..131: note = Synthetic Polynucleotide
  source 1..131: mol_type = other DNA
gggcgatgccacctacggcaagctgaccctgaagttcatctgcacccggcaagctgcccgtgccctggcccaccctcgtgaccaccctgacctacggcgtgcagtgcttcagccgctaccccgaccacatg

SEQ ID NO: 227 - DNA, 100 bp, synthetic construct
  misc_feature 1..100: note = Synthetic Polynucleotide
  source 1..100: mol_type = other DNA
gggcgatgccacctacggcaagctgcccgtgccctggcccaccctcgtgaccaccctgacctacggcgtgcagtgcttcagccgctaccccgaccacatg

SEQ ID NO: 228 - DNA, 131 bp, synthetic construct
  misc_feature 1..131: note = Synthetic Polynucleotide
  source 1..131: mol_type = other DNA
gggcgatgccacctacggcaagctgaccctgaagttcatctgcaccacgcaagctgcccgtgccctggcccaccctcgtgaccaccctgacctacggcgtgcagtgcttcagccgctaccccgaccacatg

SEQ ID NO: 229 - DNA, 131 bp, synthetic construct
  misc_feature 1..131: note = Synthetic Polynucleotide
  source 1..131: mol_type = other DNA
gggcgatgccacctacggcaagctgaccctgaagttcatctgcaccaccggcaagctgcgtgccctggcccaccctcgtgaccaccctgacctacggcgtgcagtgcttcagccgctaccccgaccacatg

SEQ ID NO: 230 - DNA, 131 bp, synthetic construct
  misc_feature 1..131: note = Synthetic Polynucleotide
  source 1..131: mol_type = other DNA
gggcgatgccacctacggcaagctgaccctgaagttcatctgcaccaccggcaagctgcccgccctggcccaccctcgtgaccaccctgacctacggcgtgcagtgcttcagccgctaccccgaccacatg

SEQ ID NO: 231 - DNA, 125 bp, synthetic construct
  misc_feature 1..125: note = Synthetic Polynucleotide
  source 1..125: mol_type = other DNA
gggcgatgccacctacggcaagctgaccctgaagttcatctggcaagctgcccgtgccctggcccaccctcgtgaccaccctgacctacggcgtgcagtgcttcagccgctaccccgaccacatg

SEQ ID NO: 232 - DNA, 82 bp, synthetic construct
  misc_feature 1..82: note = Synthetic Polynucleotide
  source 1..82: mol_type = other DNA
gggcgatgccacctacggcaagctgaccctgaagttcatctgcaccaccgcgcagtgcttcagccgctaccccgaccacatg

SEQ ID NO: 233 - DNA, 131 bp, synthetic construct
  misc_feature 1..131: note = Synthetic Polynucleotide
  source 1..131: mol_type = other DNA
gggcgatgccacctacggcaagctgaccctgaagttcatctgcaccacccaagctgcccgtgccctggcccaccctcgtgaccaccctgacctacggcgtgcagtgcttcagccgctaccccgaccacatg

SEQ ID NO: 234 - DNA, 135 bp, synthetic construct
  misc_feature 1..135: note = Synthetic Polynucleotide
  source 1..135: mol_type = other DNA
gggcgatgccacctacggcaagctgaccctgaagttcatctgcaccaccgatgcaagctgcccgtgccctggcccaccctcgtgaccaccctgacctacggcgtgcagtgcttcagccgctaccccgaccacatg

SEQ ID NO: 235 - DNA, 166 bp, synthetic construct
  misc_feature 1..166: note = Synthetic Polynucleotide
  source 1..166: mol_type = other DNA
gggcgatgccacctacggcaagctgaccctgaagttcatctgcaccaccggcaagctgaccctgaagttcatctgcaccaccggcaagctgcccgtgccctggcccaccctcgtgaccaccctgacctacggcgtgcagtgcttcagccgctaccccgaccacatg

SEQ ID NO: 236 - DNA, 130 bp, synthetic construct
  misc_feature 1..130: note = Synthetic Polynucleotide
  source 1..130: mol_type = other DNA
gggcgatgccacctacggcaagctgaccctgaagaaatgaagaaatgaagaaatgcccgtgccctggcccaccctcgtgaccaccctgacctacggcgtgcagtgcttcagccgctaccccgaccacatg

SEQ ID NO: 237 - DNA, 80 bp, synthetic construct
  misc_feature 1..80: note = Synthetic Polynucleotide
  source 1..80: mol_type = other DNA
ggcagaagctggaagaggaagggccggagtctgagcagaagaagaagggttcccaccatatcaaccggtggcgcatcgcc

SEQ ID NO: 238 - DNA, 77 bp, synthetic construct
  misc_feature 1..77: note = Synthetic Polynucleotide
  source 1..77: mol_type = other DNA
ggcagaagctggaagaggaagggccggagtctgagcagaagaagggttcccaccatatcaaccggtggcgcatcgcc

SEQ ID NO: 239 - DNA, 78 bp, synthetic construct
  misc_feature 1..78: note = Synthetic Polynucleotide
  source 1..78: mol_type = other DNA
ggcagaagctggaagaggaagggccggagtctgagcagaaagaagggttcccaccatatcaaccggtggcgcatcgcc

SEQ ID NO: 240 - DNA, 73 bp, synthetic construct
  misc_feature 1..73: note = Synthetic Polynucleotide
  source 1..73: mol_type = other DNA
ggcagaagctggaagaggaagggccggagtctgagagaagggttcccaccatatcaaccggtggcgcatcgcc

SEQ ID NO: 241 - DNA, 76 bp, synthetic construct
  misc_feature 1..76: note = Synthetic Polynucleotide
  source 1..76: mol_type = other DNA
ggcagaagctggaagaggaagggccggagtctgagcagagaagggttcccaccatatcaaccggtggcgcatcgcc

SEQ ID NO: 242 - DNA, 71 bp, synthetic construct
  misc_feature 1..71: note = Synthetic Polynucleotide
  source 1..71: mol_type = other DNA
ggcagaagctggaagaggaagggccggagtctgagaagggttcccaccatatcaaccggtggcgcatcgcc

SEQ ID NO: 243 - DNA, 71 bp, synthetic construct
  misc_feature 1..71: note = Synthetic Polynucleotide
  source 1..71: mol_type = other DNA
ggcagaagctggaagaggaagggccggagtctgagcagaagaaccaccatatcaaccggtggcgcatcgcc

SEQ ID NO: 244 - DNA, 70 bp, synthetic construct
  misc_feature 1..70: note = Synthetic Polynucleotide
  source 1..70: mol_type = other DNA
ggcagaagctggaagaggaagggccggagtctagaagggttcccaccatatcaaccggtggcgcatcgcc

SEQ ID NO: 245 - DNA, 78 bp, synthetic construct
  misc_feature 1..78: note = Synthetic Polynucleotide
  source 1..78: mol_type = other DNA
ggcagaagctggaagaggaagggccggagtctgagcagaagaagaagggttcaccatatcaaccggtggcgcatcgcc

SEQ ID NO: 246 - DNA, 74 bp, synthetic construct
  misc_feature 1..74: note = Synthetic Polynucleotide
  source 1..74: mol_type = other DNA
ggcagaagctggaagaggaagggccggagtctgagcagaagggttcccaccatatcaaccggtggcgcatcgcc

SEQ ID NO: 247 - DNA, 71 bp, synthetic construct
  misc_feature 1..71: note = Synthetic Polynucleotide
  source 1..71: mol_type = other DNA
ggcagaagctggaagaggaagggccggagtctgagcagggttcccaccatatcaaccggtggcgcatcgcc

SEQ ID NO: 248 - DNA, 77 bp, synthetic construct
  misc_feature 1..77: note = Synthetic Polynucleotide
  source 1..77: mol_type = other DNA
ggcagaagctggaagaggaagggccggagtctgagcagaagaccatatcccaccatatcaaccggtggcgcatcgcc

SEQ ID NO: 249 - DNA, 77 bp, synthetic construct
  misc_feature 1..77: note = Synthetic Polynucleotide
  source 1..77: mol_type = other DNA
ggcagaagctggaagaggaagggccggagtctgagcagaagaccatatccaaccatatcaaccggtggcgcatcgcc

SEQ ID NO: 250 - DNA, 83 bp, synthetic construct
  misc_feature 1..83: note = Synthetic Polynucleotide
  source 1..83: mol_type = other DNA
ggcagaagctggaagaggaagggccggagtctgagcagaagaagaagaagggttcccaccatatcaaccggtggcgcatcgcc

SEQ ID NO: 251 - protein, 39 aa, synthetic construct
  REGION 1..39: note = Synthetic Polypeptide
GGSGGSGGSGGSGGSGGSGGSGGSGGSTALALPKKKRKV

SEQ ID NO: 252 - protein, 27 aa, synthetic construct
  REGION 1..27: note = Synthetic Polypeptide
GGSGGSGGSGGSGGSGGSGGSGGSGGS

SEQ ID NO: 253 - protein, 6 aa, synthetic construct
  REGION 1..6: note = Synthetic Polypeptide
HHHHHH

SEQ ID NO: 254 - protein, 4 aa, synthetic construct
  REGION 1..4: note = Synthetic Polypeptide
ALAL

SEQ ID NO: 255 - protein, 28 aa, synthetic construct
  REGION 1..28: note = Synthetic Polypeptide
GGSGGSGGSGGSALALGGSGGSGGSGGS

SEQ ID NO: 256 - protein, 6 aa, synthetic construct
  REGION 1..6: note = Synthetic Polypeptide
  SITE 1: note = misc_feature - Xaa can be any naturally occurring amino acid
  SITE 6: note = misc_feature - Xaa can be any naturally occurring amino acid
XAGVFX

SEQ ID NO: 257 - protein, 6 aa, synthetic construct
  REGION 1..6: note = Synthetic Polypeptide
  SITE 1: note = misc_feature - Xaa can be any naturally occurring amino acid
  SITE 6: note = misc_feature - Xaa can be any naturally occurring amino acid
XGFLGX

SEQ ID NO: 258 - protein, 6 aa, synthetic construct
  REGION 1..6: note = Synthetic Polypeptide
  SITE 1: note = misc_feature - Xaa can be any naturally occurring amino acid
  SITE 6: note = misc_feature - Xaa can be any naturally occurring amino acid
XALALX

SEQ ID NO: 259 - protein, 7 aa, synthetic construct
  REGION 1..7: note = Synthetic Polypeptide
  SITE 1: note = misc_feature - Xaa can be any naturally occurring amino acid
  SITE 7: note = misc_feature - Xaa can be any naturally occurring amino acid
XALALAX

SEQ ID NO: 260 - protein, 1374 aa, synthetic construct
  REGION 1..1374: note = Synthetic Polypeptide
MDKKYSIGLAIGTNSVGWAVITDEYKVPSKKFKVLGNTDRHSIKKNLIGALLFDSGETAEATRLKRTARRRYTRRKNRICYLQEIFSNEMAKVDDSFFHRLEESFLVEEDKKHERHPIFGNIVDEVAYHEKYPTIYHLRKKLVDSTDKADLRLIYLALAHMIKFRGHFLIEGDLNPDNSDVDKLFIQLVQTYNQLFEENPINASGVDAKAILSARLSKSRRLENLIAQLPGEKKNGLFGNLIALSLGLTPNFKSNFDLAEDAKLQLSKDTYDDDLDNLLAQIGDQYADLFLAAKNLSDAILLSDILRVNTEITKAPLSASMIKRYDEHHQDLTLLKALVRQQLPEKYKEIFFDQSKNGYAGYIDGGASQEEFYKFIKPILEKMDGTEELLVKLNREDLLRKQRTFDNGSIPHQIHLGELHAILRRQEDFYPFLKDNREKIEKILTFRIPYYVGPLARGNSRFAWMTRKSEETITPWNFEEVVDKGASAQSFIERMTNFDKNLPNEKVLPKHSLLYEYFTVYNELTKVKYVTEGMRKPAFLSGEQKKAIVDLLFKTNRKVTVKQLKEDYFKKIECFDSVEISGVEDRFNASLGTYHDLLKIIKDKDFLDNEENEDILEDIVLTLTLFEDREMIEERLKTYAHLFDDKVMKQLKRRRYTGWGRLSRKLINGIRDKQSGKTILDFLKSDGFANRNFMQLIHDDSLTFKEDIQKAQVSGQGDSLHEHIANLAGSPAIKKGILQTVKVVDELVKVMGRHKPENIVIEMARENQTTQKGQKNSRERMKRIEEGIKELGSQILKEHPVENTQLQNEKLYLYYLQNGRDMYVDQELDINRLSDYDVDHIVPQSFLKDDSIDNKVLTRSDKNRGKSDNVPSEEVVKKMKNYWRQLLNAKLITQRKFDNLTKAERGGLSELDKAGFIKRQLVETRQITKHVAQILDSRMNTKYDENDKLIREVKVITLKSKLVSDFRKDFQFYKVREINNYHHAHDAYLNAVVGTALIKKYPKLESEFVYGDYKVYDVRKMIAKSEQEIGKATAKYFFYSNIMNFFKTEITLANGEIRKRPLIETNGETGEIVWDKGRDFATVRKVLSMPQVNIVKKTEVQTGGFSKESILPKRNSDKLIARKKDWDPKKYGGFDSPTVAYSVLVVAKVEKGKSKKLKSVKELLGITIMERSSFEKNPIDFLEAKGYKEVKKDLIIKLPKYSLFELENGRKRMLASAGELQKGNELALPSKYVNFLYLASHYEKLKGSPEDNEQKQLFVEQHKHYLDEIIEQISEFSKRVILADANLDKVLSAYNKHRDKPIREQAENIIHLFTLTNLGAPAAFKYFDTTIDRKRYTSTKEVLDATLIHQSITGLYETRIDLSQLGGDHHHHHH

SEQ ID NO: 261 - DNA, 4959 bp, synthetic construct
  misc_feature 1..4959: note = Synthetic Polynucleotide
  source 1..4959: mol_type = other DNA
atgggtgctagcaaaggtgaacgtctgtttcgtggtaaagtaccgatcttagtggaattaaagggcgacgtgaacggtcataaatttagcgtgcgcggcaaaggcaaaggtgacgctacccgtggtaaattgaccctgaagtttatttgcacaacaggcaaattacccgttccgtggcccaccttagtgaccaccctgacctccggcgttcagtgcttcagtcgttaccctaaacatatgaaacgtcacgattttttcaaatcagccatgcctaaaggatatgttcaagagcgtacaatcagcttcaagaaggatggcaaatataaaacgcgtgcggaagtgaaatttgaaggccgcacattagtaaatcgtatcaaactgaaaggtcgtgacttcaaagaaaaaggcaacattttaggccataaactgcgttataactttaattctcataaggtgtatattacggccgataaacgcaagaatggtatcaaggcaaaattcaaaattcgccataacgtgaaagacggcagcgttcaattagcggatcattatcaacaaaacacgccgattggtcgcgggcctgtactgttacctcgcaaccactacctgagcacccgttctaaactgagcaaagatccgaaagaaaaacgcgatcacatggttctgttagaattcgtgaccgctgcaggcattaagcacggacgcgacgaacgctacaagaccggtggtagcggtggttctggtggttctggtggtagcggcggtagcggtggtagcggtggtagcggtggcagcggcggtaccgcgctcgcgctgcccaagaagaagaggaaggtgatggataagaaatactcaataggcttagatatcggcacaaatagcgtcggatgggcggtgatcactgatgaatataaggttccgtctaaaaagttcaaggttctgggaaatacagaccgccacagtatcaaaaaaaatcttataggggctcttttatttgacagtggagagacagcggaagcgactcgtctcaaacggacagctcgtagaaggtatacacgtcggaagaatcgtatttgttatctacaggagattttttcaaatgagatggcgaaagtagatgatagtttctttcatcgacttgaagagtcttttttggtggaagaagacaagaagcatgaacgtcatcctatttttggaaatatagtagatgaagttgcttatcatgagaaatatccaactatctatcatctgcgaaaaaaattggtagattctactgataaagcggatttgcgcttaatctatttggccttagcgcatatgattaagtttcgtggtcattttttgattgagggagatttaaatcctgataatagtgatgtggacaaactatttatccagttggtacaaacctacaatcaattatttgaagaaaaccctattaacgcaagtggagtagatgctaaagcgattctttctgcacgattgagtaaatcaagacgattagaaaatctcattgctcagctccccggtgagaagaaaaatggcttatttgggaatctcattgctttgtcattgggtttgacccctaattttaaatcaaattttgatttggcagaagatgctaaattacagctttcaaaagatacttacgatgatgatttagataatttattggcgcaaattggagatcaatatgctgatttgtttttggcagctaagaatttatcagatgctattttactttcagatatcctaagagtaaatactgaaataactaaggctcccctatcagcttcaatgattaaacgctacgatgaacatcatcaagacttgactcttttaaaagctttagttcgacaacaacttccagaaaagtataaagaaatcttttttgatcaatcaaaaaacggatatgcaggttatattgatgggggagctagccaagaagaattttataaatttatcaaaccaattttagaaaaaatggatggtactgaggaattattggtgaaactaaatcgtgaagatttgctgcgcaagcaacggacctttgacaacggctctattccccatcaaattcacttgggtgagctgcatgctattttgagaagacaagaagacttttatccatttttaaaagacaatcgtgagaagattgaaaaaatcttgacttttcgaattccttattatgttggtccattggcgcgtggcaatagtcgttttgcatggatgactcggaagtctgaagaaacaattaccccatggaattttgaagaagttgtcgataaaggtgcttcagctcaatcatttattgaacgcatgacaaactttgataaaaatcttccaaatgaaaaagtactaccaaaacatagtttgctttatgagtattttacggtttataacgaattgacaaaggtcaaatatgttactgaaggaatgcgaaaaccagcatttctttcaggtgaacagaagaaagccattgttgatttactcttcaaaacaaatcgaaaagtaaccgttaagcaattaaaagaagattatttcaaaaaaatagaatgttttgatagtgttgaaatttcaggagttgaagatagatttaatgcttcattaggtacctaccatgatttgctaaaaattattaaagataaagattttttggataatgaagaaaatgaagatatcttagaggatattgttttaacattgaccttatttgaagatagggagatgattgaggaaagacttaaaacatatgctcacctctttgatgataaggtgatgaaacagcttaaacgtcgccgttatactggttggggacgtttgtctcgaaaattgattaatggtattagggataagcaatctggcaaaacaatattagattttttgaaatcagatggttttgccaatcgcaattttatgcagctgatccatgatgatagtttgacatttaaagaagacattcaaaaagcacaagtgtctggacaaggcgatagtttacatgaacatattgcaaatttagctggtagccctgctattaaaaaaggtattttacagactgtaaaagttgttgatgaattggtcaaagtaatggggcggcataagccagaaaatatcgttattgaaatggcacgtgaaaatcagacaactcaaaagggccagaaaaattcgcgagagcgtatgaaacgaatcgaagaaggtatcaaagaattaggaagtcagattcttaaagagcatcctgttgaaaatactcaattgcaaaatgaaaagctctatctctattatctccaaaatggaagagacatgtatgtggaccaagaattagatattaatcgtttaagtgattatgatgtcgatcacattgttccacaaagtttccttaaagacgattcaatagacaataaggtcttaacgcgttctgataaaaatcgtggtaaatcggataacgttccaagtgaagaagtagtcaaaaagatgaaaaactattggagacaacttctaaacgccaagttaatcactcaacgtaagtttgataatttaacgaaagctgaacgtggaggtttgagtgaacttgataaagctggttttatcaaacgccaattggttgaaactcgccaaatcactaagcatgtggcacaaattttggatagtcgcatgaatactaaatacgatgaaaatgataaacttattcgagaggttaaagtgattaccttaaaatctaaattagtttctgacttccgaaaagatttccaattctataaagtacgtgagattaacaattaccatcatgcccatgatgcgtatctaaatgccgtcgttggaactgctttgattaagaaatatccaaaacttgaatcggagtttgtctatggtgattataaagtttatgatgttcgtaaaatgattgctaagtctgagcaagaaataggcaaagcaaccgcaaaatatttcttttactctaatatcatgaacttcttcaaaacagaaattacacttgcaaatggagagattcgcaaacgccctctaatcgaaactaatggggaaactggagaaattgtctgggataaagggcgagattttgccacagtgcgcaaagtattgtccatgccccaagtcaatattgtcaagaaaacagaagtacagacaggcggattctccaaggagtcaattttaccaaaaagaaattcggacaagcttattgctcgtaaaaaagactgggatccaaaaaaatatggtggttttgatagtccaacggtagcttattcagtcctagtggttgctaaggtggaaaaagggaaatcgaagaagttaaaatccgttaaagagttactagggatcacaattatggaaagaagttcctttgaaaaaaatccgattgactttttagaagctaaaggatataaggaagttaaaaaagacttaatcattaaactacctaaatatagtctttttgagttagaaaacggtcgtaaacggatgctggctagtgccggagaattacaaaaaggaaatgagctggctctgccaagcaaatatgtgaattttttatatttagctagtcattatgaaaagttgaagggtagtccagaagataacgaacaaaaacaattgtttgtggagcagcataagcattatttagatgagattattgagcaaatcagtgaattttctaagcgtgttattttagcagatgccaatttagataaagttcttagtgcatataacaaacatagagacaaaccaatacgtgaacaagcagaaaatattattcatttatttacgttgacgaatcttggagctcccgctgcttttaaatattttgatacaacaattgatcgtaaacgatatacgtctacaaaagaagttttagatgccactcttatccatcaatccatcactggtctttatgaaacacgcattgatttgagtcagctaggaggtgaccatcaccaccaccatcac

SEQ ID NO: 262 - DNA, 4959 bp, synthetic construct
  misc_feature 1..4959: note = Synthetic Polynucleotide
  source 1..4959: mol_type = other DNA
atgggtgctagcaaaggtgaagagctgtttgacggtgtagtaccgatcttagtggaattagacggcgacgtgaacggtcacgaatttagcgtgcgcggcgagggcgaaggtgacgctaccgagggtgaattgaccctgaagtttatttgcacaacaggcgaattacccgttccgtggcccaccttagtgaccaccctgacctccggcgttcagtgcttcagtgattacccagatcatatggatcaacacgattttttcaaatcagccatgcctgaaggatatgttcaagagcgtacaatcagcttcaaggacgatggcacctataaaacgcgtgcggaagtgaaatttgaaggcgacacattagtaaaccgtatcgaactgaaaggtatcgacttcaaagaagacggcaacattttaggccataagctggaatataactttaattctcatgacgtgtatattacggccgataaacaggaaaacggtatcaaggcagaatttgaaattcgccataacgtggaggacggcagcgttcaattagcggatcattatcaacaaaacacgccgattggtgatgggcctgtactgttacctgacgatcactacctgagcacggagtcagccctgagcaaagatccgaacgaagaccgcgatcacatggttctgttagaattcgtgaccgctgcaggcattgatcatggaatggacgagctgtacaagaccggtggtagcggtggttctggtggttctggtggtagcggcggtagcggtggtagcggtggtagcggtggcagcggcggtaccgcgctcgcgctgcccaagaagaagaggaaggtgatggataagaaatactcaataggcttagatatcggcacaaatagcgtcggatgggcggtgatcactgatgaatataaggttccgtctaaaaagttcaaggttctgggaaatacagaccgccacagtatcaaaaaaaatcttataggggctcttttatttgacagtggagagacagcggaagcgactcgtctcaaacggacagctcgtagaaggtatacacgtcggaagaatcgtatttgttatctacaggagattttttcaaatgagatggcgaaagtagatgatagtttctttcatcgacttgaagagtcttttttggtggaagaagacaagaagcatgaacgtcatcctatttttggaaatatagtagatgaagttgcttatcatgagaaatatccaactatctatcatctgcgaaaaaaattggtagattctactgataaagcggatttgcgcttaatctatttggccttagcgcatatgattaagtttcgtggtcattttttgattgagggagatttaaatcctgataatagtgatgtggacaaactatttatccagttggtacaaacctacaatcaattatttgaagaaaaccctattaacgcaagtggagtagatgctaaagcgattctttctgcacgattgagtaaatcaagacgattagaaaatctcattgctcagctccccggtgagaagaaaaatggcttatttgggaatctcattgctttgtcattgggtttgacccctaattttaaatcaaattttgatttggcagaagatgctaaattacagctttcaaaagatacttacgatgatgatttagataatttattggcgcaaattggagatcaatatgctgatttgtttttggcagctaagaatttatcagatgctattttactttcagatatcctaagagtaaatactgaaataactaaggctcccctatcagcttcaatgattaaacgctacgatgaacatcatcaagacttgactcttttaaaagctttagttcgacaacaacttccagaaaagtataaagaaatcttttttgatcaatcaaaaaacggatatgcaggttatattgatgggggagctagccaagaagaattttataaatttatcaaaccaattttagaaaaaatggatggtactgaggaattattggtgaaactaaatcgtgaagatttgctgcgcaagcaacggacctttgacaacggctctattccccatcaaattcacttgggtgagctgcatgctattttgagaagacaagaagacttttatccatttttaaaagacaatcgtgagaagattgaaaaaatcttgacttttcgaattccttattatgttggtccattggcgcgtggcaatagtcgttttgcatggatgactcggaagtctgaagaaacaattaccccatggaattttgaagaagttgtcgataaaggtgcttcagctcaatcatttattgaacgcatgacaaactttgataaaaatcttccaaatgaaaaagtactaccaaaacatagtttgctttatgagtattttacggtttataacgaattgacaaaggtcaaatatgttactgaaggaatgcgaaaaccagcatttctttcaggtgaacagaagaaagccattgttgatttactcttcaaaacaaatcgaaaagtaaccgttaagcaattaaaagaagattatttcaaaaaaatagaatgttttgatagtgttgaaatttcaggagttgaagatagatttaatgcttcattaggtacctaccatgatttgctaaaaattattaaagataaagattttttggataatgaagaaaatgaagatatcttagaggatattgttttaacattgaccttatttgaagatagggagatgattgaggaaagacttaaaacatatgctcacctctttgatgataaggtgatgaaacagcttaaacgtcgccgttatactggttggggacgtttgtctcgaaaattgattaatggtattagggataagcaatctggcaaaacaatattagattttttgaaatcagatggttttgccaatcgcaattttatgcagctgatccatgatgatagtttgacatttaaagaagacattcaaaaagcacaagtgtctggacaaggcgatagtttacatgaacatattgcaaatttagctggtagccctgctattaaaaaaggtattttacagactgtaaaagttgttgatgaattggtcaaagtaatggggcggcataagccagaaaatatcgttattgaaatggcacgtgaaaatcagacaactcaaaagggccagaaaaattcgcgagagcgtatgaaacgaatcgaagaaggtatcaaagaattaggaagtcagattcttaaagagcatcctgttgaaaatactcaattgcaaaatgaaaagctctatctctattatctccaaaatggaagagacatgtatgtggaccaagaattagatattaatcgtttaagtgattatgatgtcgatcacattgttccacaaagtttccttaaagacgattcaatagacaataaggtcttaacgcgttctgataaaaatcgtggtaaatcggataacgttccaagtgaagaagtagtcaaaaagatgaaaaactattggagacaacttctaaacgccaagttaatcactcaacgtaagtttgataatttaacgaaagctgaacgtggaggtttgagtgaacttgataaagctggttttatcaaacgccaattggttgaaactcgccaaatcactaagcatgtggcacaaattttggatagtcgcatgaatactaaatacgatgaaaatgataaacttattcgagaggttaaagtgattaccttaaaatctaaattagtttctgacttccgaaaagatttccaattctataaagtacgtgagattaacaattaccatcatgcccatgatgcgtatctaaatgccgtcgttggaactgctttgattaagaaatatccaaaacttgaatcggagtttgtctatggtgattataaagtttatgatgttcgtaaaatgattgctaagtctgagcaagaaataggcaaagcaaccgcaaaatatttcttttactctaatatcatgaacttcttcaaaacagaaattacacttgcaaatggagagattcgcaaacgccctctaatcgaaactaatggggaaactggagaaattgtctgggataaagggcgagattttgccacagtgcgcaaagtattgtccatgccccaagtcaatattgtcaagaaaacagaagtacagacaggcggattctccaaggagtcaattttaccaaaaagaaattcggacaagcttattgctcgtaaaaaagactgggatccaaaaaaatatggtggttttgatagtccaacggtagcttattcagtcctagtggttgctaaggtggaaaaagggaaatcgaagaagttaaaatccgttaaagagttactagggatcacaattatggaaagaagttcctttgaaaaaaatccgattgactttttagaagctaaaggatataaggaagttaaaaaagacttaatcattaaactacctaaatatagtctttttgagttagaaaacggtcgtaaacggatgctggctagtgccggagaattacaaaaaggaaatgagctggctctgccaagcaaatatgtgaattttttatatttagctagtcattatgaaaagttgaagggtagtccagaagataacgaacaaaaacaattgtttgtggagcagcataagcattatttagatgagattattgagcaaatcagtgaattttctaagcgtgttattttagcagatgccaatttagataaagttcttagtgcatataacaaacatagagacaaaccaatacgtgaacaagcagaaaatattattcatttatttacgttgacgaatcttggagctcccgctgcttttaaatattttgatacaacaattgatcgtaaacgatatacgtctacaaaagaagttttagatgccactcttatccatcaatccatcactggtctttatgaaacacgcattgatttgagtcagctaggaggtgaccatcaccaccaccatcac

SEQ ID NO: 263 - DNA, 1059 bp, synthetic construct
  misc_feature 1..1059: note = Synthetic Polynucleotide
  source 1..1059: mol_type = other DNA
atggcgagcaatttactgaccgtacaccaaaatttgcctgcattgccggtcgatgcaacgagtgatgaggttcgcaagaacctgatggacatgttcagggatcgccaggcgttttctgagcatacctggaaaatgcttctgtccgtttgccggtcgtgggcggcatggtgcaagttgaataaccggaaatggtttcccgcagaacctgaagatgttcgcgattatcttctatatcttcaggcgcgcggtctggcagtaaaaactatccagcaacatttgggccagctaaacatgcttcatcgtcggtccgggctgccacgaccaagtgacagcaatgctgtttcactggttatgcggcgtatccgaaaagaaaacgttgatgccggtgaacgtgcaaaacaggctctagcgttcgaacgcactgatttcgaccaggttcgttcactcatggaaaatagcgatcgctgccaggatatacgtaatctggcatttctggggattgcttataacaccctgttacgtatagccgaaattgccaggatcagggttaaagatatctcacgtactgacggtgggagaatgttaatccatattggcagaacgaaaacgctggttagcaccgcaggtgtagagaaggcacttagcctgggggtaactaaactggtcgagcgatggatttccgtctctggtgtagctgatgatccgaataactacctgttttgccgggtcagaaaaaatggtgttgccgcgccatctgccaccagccagctatcaactcgcgccctggaagggatttttgaagcaactcatcgattgatttacggcgctaaggatgactctggtcagagatacctggcctggtctggacacagtgcccgtgtcggagccgcgcgagatatggcccgcgctggagtttcaataccggagatcatgcaagctggtggctggaccaatgtaaatattgtcatgaactatatccgtaacctggatagtgaaacaggggcaatggtgcgcctgctggaagatggcgacggcggatcccatcaccaccaccatcac

SEQ ID NO: 264 - DNA, 1860 bp, synthetic construct
  misc_feature 1..1860: note = Synthetic Polynucleotide
  source 1..1860: mol_type = other DNA
atgggtgctagcaaaggtgaagagctgtttgacggtgtagtaccgatcttagtggaattagacggcgacgtgaacggtcacgaatttagcgtgcgcggcgagggcgaaggtgacgctaccgagggtgaattgaccctgaagtttatttgcacaacaggcgaattacccgttccgtggcccaccttagtgaccaccctgacctatggcgttcagtgcttcagtgattacccagatcatatggatcaacacgattttttcaaatcagccatgcctgaaggatatgttcaagagcgtacaatcagcttcaaggacgatggcacctataaaacgcgtgcggaagtgaaatttgaaggcgacacattagtaaaccgtatcgaactgaaaggtatcgacttcaaagaagacggcaacattttaggccataagctggaatataactttaattctcatgacgtgtatattacggccgataaacaggaaaacggtatcaaggcagaatttgaaattcgccataacgtggaggacggcagcgttcaattagcggatcattatcaacaaaacacgccgattggtgatgggcctgtactgttacctgacgatcactacctgagcacggagtcagccctgagcaaagatccgaacgaagaccgcgatcacatggttctgttagaattcgtgaccgctgcaggcattgatcatggaatggacgagctgtacaagaccggtggtagcggtggttctggtggttctggtggtagcggcggtagcggtggtagcggtggtagcggtggcagcggcggtaccgcgagcaatttactgaccgtacaccaaaatttgcctgcattgccggtcgatgcaacgagtgatgaggttcgcaagaacctgatggacatgttcagggatcgccaggcgttttctgagcatacctggaaaatgcttctgtccgtttgccggtcgtgggcggcatggtgcaagttgaataaccggaaatggtttcccgcagaacctgaagatgttcgcgattatcttctatatcttcaggcgcgcggtctggcagtaaaaactatccagcaacatttgggccagctaaacatgcttcatcgtcggtccgggctgccacgaccaagtgacagcaatgctgtttcactggttatgcggcgtatccgaaaagaaaacgttgatgccggtgaacgtgcaaaacaggctctagcgttcgaacgcactgatttcgaccaggttcgttcactcatggaaaatagcgatcgctgccaggatatacgtaatctggcatttctggggattgcttataacaccctgttacgtatagccgaaattgccaggatcagggttaaagatatctcacgtactgacggtgggagaatgttaatccatattggcagaacgaaaacgctggttagcaccgcaggtgtagagaaggcacttagcctgggggtaactaaactggtcgagcgatggatttccgtctctggtgtagctgatgatccgaataactacctgttttgccgggtcagaaaaaatggtgttgccgcgccatctgccaccagccagctatcaactcgcgccctggaagggatttttgaagcaactcatcgattgatttacggcgctaaggatgactctggtcagagatacctggcctggtctggacacagtgcccgtgtcggagccgcgcgagatatggcccgcgctggagtttcaataccggagatcatgcaagctggtggctggaccaatgtaaatattgtcatgaactatatccgtaacctggatagtgaaacaggggcaatggtgcgcctgctggaagatggcgacggcggatcccatcaccaccaccatcac

SEQ ID NO: 265 - protein, 620 aa, synthetic construct
  REGION 1..620: note = Synthetic Polypeptide
MGASKGEELFTGVVPILVELDGDVNGHKFSVRGEGEGDATNGKLTLKFICTTGKLPVPWPTLVTTLTYGVQCFSRYPDHMKQHDFFKSAMPEGYVQERTISFKDDGTYKTRAEVKFEGDTLVNRIELKGIDFKEDGNILGHKLEYNFNSHNVYITADKQKNGIKANFKIRHNVEDGSVQLADHYQQNTPIGDGPVLLPDNHYLSTQSALSKDPNEKRDHMVLLEFVTAAGITHGMDELYKTGGSGGSGGSGGSGGSGGSGGSGGSGGTASNLLTVHQNLPALPVDATSDEVRKNLMDMFRDRQAFSEHTWKMLLSVCRSWAAWCKLNNRKWFPAEPEDVRDYLLYLQARGLAVKTIQQHLGQLNMLHRRSGLPRPSDSNAVSLVMRRIRKENVDAGERAKQALAFERTDFDQVRSLMENSDRCQDIRNLAFLGIAYNTLLRIAEIARIRVKDISRTDGGRMLIHIGRTKTLVSTAGVEKALSLGVTKLVERWISVSGVADDPNNYLFCRVRKNGVAAPSATSQLSTRALEGIFEATHRLIYGAKDDSGQRYLAWSGHSARVGAARDMARAGVSIPEIMQAGGWTNVNIVMNYIRNLDSETGAMVRLLEDGDGGSHHHHHH

SEQ ID NO: 266 - DNA, 1860 bp, synthetic construct
  misc_feature 1..1860: note = Synthetic Polynucleotide
  source 1..1860: mol_type = other DNA
atgggtgctagcaaaggtgaagagctgtttacgggtgtagtaccgatcttagtggaattagacggcgacgtgaacggtcacaaatttagcgtgcgcggcgaaggcgaaggtgacgctaccaatggtaaattgaccctgaagtttatttgcacaacaggcaaattacccgttccgtggcccaccttagtgaccaccctgacctatggcgttcagtgcttcagtcgttacccagatcatatgaaacaacacgattttttcaaatcagccatgcctgaaggatatgttcaagagcgtacaatcagcttcaaggacgatggcacctataaaacgcgtgcggaagtgaaatttgaaggcgacacattagtaaaccgtatcgaactgaaaggtatcgacttcaaagaagacggcaacattttaggccataagctggaatataactttaattctcataacgtgtatattacggccgataaacagaaaaacggtatcaaggcaaatttcaaaattcgccataacgtggaagacggcagcgttcaattagcggatcattatcaacaaaacacgccgattggtgacgggcctgtactgttacctgacaaccactacctgagcacccagtcagcactgagcaaagatccgaacgaaaaacgcgatcacatggttctgttagaattcgtgaccgctgcaggcattactcacggaatggacgaactctacaagaccggtggtagcggtggttctggtggttctggtggtagcggcggtagcggtggtagcggtggtagcggtggcagcggcggtaccgcgagcaatttactgaccgtacaccaaaatttgcctgcattgccggtcgatgcaacgagtgatgaggttcgcaagaacctgatggacatgttcagggatcgccaggcgttttctgagcatacctggaaaatgcttctgtccgtttgccggtcgtgggcggcatggtgcaagttgaataaccggaaatggtttcccgcagaacctgaagatgttcgcgattatcttctatatcttcaggcgcgcggtctggcagtaaaaactatccagcaacatttgggccagctaaacatgcttcatcgtcggtccgggctgccacgaccaagtgacagcaatgctgtttcactggttatgcggcgtatccgaaaagaaaacgttgatgccggtgaacgtgcaaaacaggctctagcgttcgaacgcactgatttcgaccaggttcgttcactcatggaaaatagcgatcgctgccaggatatacgtaatctggcatttctggggattgcttataacaccctgttacgtatagccgaaattgccaggatcagggttaaagatatctcacgtactgacggtgggagaatgttaatccatattggcagaacgaaaacgctggttagcaccgcaggtgtagagaaggcacttagcctgggggtaactaaactggtcgagcgatggatttccgtctctggtgtagctgatgatccgaataactacctgttttgccgggtcagaaaaaatggtgttgccgcgccatctgccaccagccagctatcaactcgcgccctggaagggatttttgaagcaactcatcgattgatttacggcgctaaggatgactctggtcagagatacctggcctggtctggacacagtgcccgtgtcggagccgcgcgagatatggcccgcgctggagtttcaataccggagatcatgcaagctggtggctggaccaatgtaaatattgtcatgaactatatccgtaacctggatagtgaaacaggggcaatggtgcgcctgctggaagatggcgacggcggatcccatcaccaccaccatcac

SEQ ID NO: 267 - protein, 620 aa, synthetic construct
  REGION 1..620: note = Synthetic Polypeptide
MGASKGEELFTGVVPILVELDGDVNGHKFSVRGEGEGDATNGKLTLKFICTTGKLPVPWPTLVTTLTYGVQCFSRYPDHMDQHDFFKSAMPEGYVQERTISFKDDGTYKTRAEVKFEGDTLVNRIELKGIDFKEDGNILGHKLEYNFNSHDVYITADKQENGIKAEFEIRHNVEDGSVQLADHYQQNTPIGDGPVLLPDDHYLSTESALSKDPNEDRDHMVLLEFVTAAGIDHGMDELYKTGGSGGSGGSGGSGGSGGSGGSGGSGGTASNLLTVHQNLPALPVDATSDEVRKNLMDMFRDRQAFSEHTWKMLLSVCRSWAAWCKLNNRKWFPAEPEDVRDYLLYLQARGLAVKTIQQHLGQLNMLHRRSGLPRPSDSNAVSLVMRRIRKENVDAGERAKQALAFERTDFDQVRSLMENSDRCQDIRNLAFLGIAYNTLLRIAEIARIRVKDISRTDGGRMLIHIGRTKTLVSTAGVEKALSLGVTKLVERWISVSGVADDPNNYLFCRVRKNGVAAPSATSQLSTRALEGIFEATHRLIYGAKDDSGQRYLAWSGHSARVGAARDMARAGVSIPEIMQAGGWTNVNIVMNYIRNLDSETGAMVRLLEDGDGGSHHHHHH

SEQ ID NO: 268 - DNA, 1860 bp, synthetic construct
  misc_feature 1..1860: note = Synthetic Polynucleotide
  source 1..1860: mol_type = other DNA
atgggtgctagcaaaggtgaagagctgtttacgggtgtagtaccgatcttagtggaattagacggcgacgtgaacggtcacaaatttagcgtgcgcggcgaaggcgaaggtgacgctaccaatggtaaattgaccctgaagtttatttgcacaacaggcaaattacccgttccgtggcccaccttagtgaccaccctgacctatggcgttcagtgcttcagtcgttacccagatcatatggatcaacacgattttttcaaatcagccatgcctgaaggatatgttcaagagcgtacaatcagcttcaaggacgatggcacctataaaacgcgtgcggaagtgaaatttgaaggcgacacattagtaaaccgtatcgaactgaaaggtatcgacttcaaagaagacggcaacattttaggccataagctggaatataactttaattctcatgacgtgtatattacggccgataaacaggaaaacggtatcaaggcagaatttgaaattcgccataacgtggaggacggcagcgttcaattagcggatcattatcaacaaaacacgccgattggtgatgggcctgtactgttacctgacgatcactacctgagcacggagtcagccctgagcaaagatccgaacgaagaccgcgatcacatggttctgttagaattcgtgaccgctgcaggcattgatcatggaatggacgagctgtacaagaccggtggtagcggtggttctggtggttctggtggtagcggcggtagcggtggtagcggtggtagcggtggcagcggcggtaccgcgagcaatttactgaccgtacaccaaaatttgcctgcattgccggtcgatgcaacgagtgatgaggttcgcaagaacctgatggacatgttcagggatcgccaggcgttttctgagcatacctggaaaatgcttctgtccgtttgccggtcgtgggcggcatggtgcaagttgaataaccggaaatggtttcccgcagaacctgaagatgttcgcgattatcttctatatcttcaggcgcgcggtctggcagtaaaaactatccagcaacatttgggccagctaaacatgcttcatcgtcggtccgggctgccacgaccaagtgacagcaatgctgtttcactggttatgcggcgtatccgaaaagaaaacgttgatgccggtgaacgtgcaaaacaggctctagcgttcgaacgcactgatttcgaccaggttcgttcactcatggaaaatagcgatcgctgccaggatatacgtaatctggcatttctggggattgcttataacaccctgttacgtatagccgaaattgccaggatcagggttaaagatatctcacgtactgacggtgggagaatgttaatccatattggcagaacgaaaacgctggttagcaccgcaggtgtagagaaggcacttagcctgggggtaactaaactggtcgagcgatggatttccgtctctggtgtagctgatgatccgaataactacctgttttgccgggtcagaaaaaatggtgttgccgcgccatctgccaccagccagctatcaactcgcgccctggaagggatttttgaagcaactcatcgattgatttacggcgctaaggatgactctggtcagagatacctggcctggtctggacacagtgcccgtgtcggagccgcgcgagatatggcccgcgctggagtttcaataccggagatcatgcaagctggtggctggaccaatgtaaatattgtcatgaactatatccgtaacctggatagtgaaacaggggcaatggtgcgcctgctggaagatggcgacggcggatcccatcaccaccaccatcac

SEQ ID NO: 269 - DNA, 4401 bp, synthetic construct
  misc_feature 1..4401: note = Synthetic Polynucleotide
  source 1..4401: mol_type = other DNA
atggataagaaatactcaataggcttagctatcggcacaaatagcgtcggatgggcggtgatcactgatgaatataaggttccgtctaaaaagttcaaggttctgggaaatacagaccgccacagtatcaaaaaaaatcttataggggctcttttatttgacagtggagagacagcggaagcgactcgtctcaaacggacagctcgtagaaggtatacacgtcggaagaatcgtatttgttatctacaggagattttttcaaatgagatggcgaaagtagatgatagtttctttcatcgacttgaagagtcttttttggtggaagaagacaagaagcatgaacgtcatcctatttttggaaatatagtagatgaagttgcttatcatgagaaatatccaactatctatcatctgcgaaaaaaattggtagattctactgataaagcggatttgcgcttaatctatttggccttagcgcatatgattaagtttcgtggtcattttttgattgagggagatttaaatcctgataatagtgatgtggacaaactatttatccagttggtacaaacctacaatcaattatttgaagaaaaccctattaacgcaagtggagtagatgctaaagcgattctttctgcacgattgagtaaatcaagacgattagaaaatctcattgctcagctccccggtgagaagaaaaatggcttatttgggaatctcattgctttgtcattgggtttgacccctaattttaaatcaaattttgatttggcagaagatgctaaattacagctttcaaaagatacttacgatgatgatttagataatttattggcgcaaattggagatcaatatgctgatttgtttttggcagctaagaatttatcagatgctattttactttcagatatcctaagagtaaatactgaaataactaaggctcccctatcagcttcaatgattaaacgctacgatgaacatcatcaagacttgactcttttaaaagctttagttcgacaacaacttccagaaaagtataaagaaatcttttttgatcaatcaaaaaacggatatgcaggttatattgatgggggagctagccaagaagaattttataaatttatcaaaccaattttagaaaaaatggatggtactgaggaattattggtgaaactaaatcgtgaagatttgctgcgcaagcaacggacctttgacaacggctctattccccatcaaattcacttgggtgagctgcatgctattttgagaagacaagaagacttttatccatttttaaaagacaatcgtgagaagattgaaaaaatcttgacttttcgaattccttattatgttggtccattggcgcgtggcaatagtcgttttgcatggatgactcggaagtctgaagaaacaattaccccatggaattttgaagaagttgtcgataaaggtgcttcagctcaatcatttattgaacgcatgacaaactttgataaaaatcttccaaatgaaaaagtactaccaaaacatagtttgctttatgagtattttacggtttataacgaattgacaaaggtcaaatatgttactgaaggaatgcgaaaaccagcatttctttcaggtgaacagaagaaagccattgttgatttactcttcaaaacaaatcgaaaagtaaccgttaagcaattaaaagaagattatttcaaaaaaatagaatgttttgatagtgttgaaatttcaggagttgaagatagatttaatgcttcattaggtacctaccatgatttgctaaaaattattaaagataaagattttttggataatgaagaaaatgaagatatcttagaggatattgttttaacattgaccttatttgaagatagggagatgattgaggaaagacttaaaacatatgctcacctctttgatgataaggtgatgaaacagcttaaacgtcgccgttatactggttggggacgtttgtctcgaaaattgattaatggtattagggataagcaatctggcaaaacaatattagattttttgaaatcagatggttttgccaatcgcaattttatgcagctgatccatgatgatagtttgacatttaaagaagacattcaaaaagcacaagtgtctggacaaggcgatagtttacatgaacatattgcaaatttagctggtagccctgctattaaaaaaggtattttacagactgtaaaagttgttgatgaattggtcaaagtaatggggcggcataagccagaaaatatcgttattgaaatggcacgtgaaaatcagacaactcaaaagggccagaaaaattcgcgagagcgtatgaaacgaatcgaagaaggtatcaaagaattaggaagtcagattcttaaagagcatcctgttgaaaatactcaattgcaaaatgaaaagctctatctctattatctccaaaatggaagagacatgtatgtggaccaagaattagatattaatcgtttaagtgattatgatgtcgatgccattgttccacaaagtttccttaaagacgattcaatagacaataaggtcttaacgcgttctgataaaaatcgtggtaaatcggataacgttccaagtgaagaagtagtcaaaaagatgaaaaactattggagacaacttctaaacgccaagttaatcactcaacgtaagtttgataatttaacgaaagctgaacgtggaggtttgagtgaacttgataaagctggttttatcaaacgccaattggttgaaactcgccaaatcactaagcatgtggcacaaattttggatagtcgcatgaatactaaatacgatgaaaatgataaacttattcgagaggttaaagtgattaccttaaaatctaaattagtttctgacttccgaaaagatttccaattctataaagtacgtgagattaacaattaccatcatgcccatgatgcgtatctaaatgccgtcgttggaactgctttgattaagaaatatccaaaacttgaatcggagtttgtctatggtgattataaagtttatgatgttcgtaaaatgattgctaagtctgagcaagaaataggcaaagcaaccgcaaaatatttcttttactctaatatcatgaacttcttcaaaacagaaattacacttgcaaatggagagattcgcaaacgccctctaatcgaaactaatggggaaactggagaaattgtctgggataaagggcgagattttgccacagtgcgcaaagtattgtccatgccccaagtcaatattgtcaagaaaacagaagtacagacaggcggattctccaaggagtcaattttaccaaaaagaaattcggacaagcttattgctcgtaaaaaagactgggatccaaaaaaatatggtggttttgatagtccaacggtagcttattcagtcctagtggttgctaaggtggaaaaagggaaatcgaagaagttaaaatccgttaaagagttactagggatcacaattatggaaagaagttcctttgaaaaaaatccgattgactttttagaagctaaaggatataaggaagttaaaaaagacttaatcattaaactacctaaatatagtctttttgagttagaaaacggtcgtaaacggatgctggctagtgccggagaattacaaaaaggaaatgagctggctctgccaagcaaatatgtgaattttttatatttagctagtcattatgaaaagttgaagggtagtccagaagataacgaacaaaaacaattgtttgtggagcagcataagcattatttagatgagattattgagcaaatcagtgaattttctaagcgtgttattttagcagatgccaatttagataaagttcttagtgcatataacaaacatagagacaaaccaatacgtgaacaagcagaaaatattattcatttatttacgttgacgaatcttggagctcccgctgcttttaaatattttgatacaacaattgatcgtaaacgatatacgtctacaaaagaagttttagatgccactcttatccatcaatccatcactggtctttatgaaacacgcattgatttgagtcagctaggaggtgacggttctcccaagaagaagaggaaagtctcgagcgactacaaagaccatgacggtgattataaagatcatgacatcgattacaaggatgacgatgacaaggctgcaggaggcggtggaagcgggcgcgccgacgcgctggacgatttcgatctcgacatgctgggttctgatgccctcgatgactttgacctggatatgttgggaagcgacgcattggatgactttgatctggacatgctcggctccgatgctctggacgatttcgatctcgatatgttacatcaccaccaccatcac

SEQ ID NO: 270 - protein, 1384 aa, synthetic construct
  REGION 1..1384: note = Synthetic Polypeptide
MDKKYSIGLAIGTNSVGWAVITDEYKVPSKKFKVLGNTDRHSIKKNLIGALLFDSGETAEATRLKRTARRRYTRRKNRICYLQEIFSNEMAKVDDSFFHRLEESFLVEEDKKHERHPIFGNIVDEVAYHEKYPTIYHLRKKLVDSTDKADLRLIYLALAHMIKFRGHFLIEGDLNPDNSDVDKLFIQLVQTYNQLFEENPINASGVDAKAILSARLSKSRRLENLIAQLPGEKKNGLFGNLIALSLGLTPNFKSNFDLAEDAKLQLSKDTYDDDLDNLLAQIGDQYADLFLAAKNLSDAILLSDILRVNTEITKAPLSASMIKRYDEHHQDLTLLKALVRQQLPEKYKEIFFDQSKNGYAGYIDGGASQEEFYKFIKPILEKMDGTEELLVKLNREDLLRKQRTFDNGSIPHQIHLGELHAILRRQEDFYPFLKDNREKIEKILTFRIPYYVGPLARGNSRFAWMTRKSEETITPWNFEEVVDKGASAQSFIERMTNFDKNLPNEKVLPKHSLLYEYFTVYNELTKVKYVTEGMRKPAFLSGEQKKAIVDLLFKTNRKVTVKQLKEDYFKKIECFDSVEISGVEDRFNASLGTYHDLLKIIKDKDFLDNEENEDILEDIVLTLTLFEDREMIEERLKTYAHLFDDKVMKQLKRRRYTGWGRLSRKLINGIRDKQSGKTILDFLKSDGFANRNFMQLIHDDSLTFKEDIQKAQVSGQGDSLHEHIANLAGSPAIKKGILQTVKVVDELVKVMGRHKPENIVIEMARENQTTQKGQKNSRERMKRIEEGIKELGSQILKEHPVENTQLQNEKLYLYYLQNGRDMYVDQELDINRLSDYDVDHIVPQSFLKDDSIDNKVLTRSDKNRGKSDNVPSEEVVKKMKNYWRQLLNAKLITQRKFDNLTKAERGGLSELDKAGFIKRQLVETRQITKHVAQILDSRMNTKYDENDKLIREVKVITLKSKLVSDFRKDFQFYKVREINNYHHAHDAYLNAVVGTALIKKYPKLESEFVYGDYKVYDVRKMIAKSEQEIGKATAKYFFYSNIMNFFKTEITLANGEIRKRPLIETNGETGEIVWDKGRDFATVRKVLSMPQVNIVKKTEVQTGGFSKESILPKRNSDKLIARKKDWDPKKYGGFDSPTVAYSVLVVAKVEKGKSKKLKSVKELLGITIMERSSFEKNPIDFLEAKGYKEVKKDLIIKLPKYSLFELENGRKRMLASAGELQKGNELALPSKYVNFLYLASHYEKLKGSPEDNEQKQLFVEQHKHYLDEIIEQISEFSKRVILADANLDKVLSAYNKHRDKPIREQAENIIHLFTLTNLGAPAAFKYFDTTIDRKRYTSTKEVLDATLIHQSITGLYETRIDLSQLGGDPKKKRKVMDKHHHHHH

SEQ ID NO: 271 - DNA, 4152 bp, synthetic construct
  misc_feature 1..4152: note = Synthetic Polynucleotide
  source 1..4152: mol_type = other DNA
atggataagaaatactcaataggcttagatatcggcacaaatagcgtcggatgggcggtgatcactgatgaatataaggttccgtctaaaaagttcaaggttctgggaaatacagaccgccacagtatcaaaaaaaatcttataggggctcttttatttgacagtggagagacagcggaagcgactcgtctcaaacggacagctcgtagaaggtatacacgtcggaagaatcgtatttgttatctacaggagattttttcaaatgagatggcgaaagtagatgatagtttctttcatcgacttgaagagtcttttttggtggaagaagacaagaagcatgaacgtcatcctatttttggaaatatagtagatgaagttgcttatcatgagaaatatccaactatctatcatctgcgaaaaaaattggtagattctactgataaagcggatttgcgcttaatctatttggccttagcgcatatgattaagtttcgtggtcattttttgattgagggagatttaaatcctgataatagtgatgtggacaaactatttatccagttggtacaaacctacaatcaattatttgaagaaaaccctattaacgcaagtggagtagatgctaaagcgattctttctgcacgattgagtaaatcaagacgattagaaaatctcattgctcagctccccggtgagaagaaaaatggcttatttgggaatctcattgctttgtcattgggtttgacccctaattttaaatcaaattttgatttggcagaagatgctaaattacagctttcaaaagatacttacgatgatgatttagataatttattggcgcaaattggagatcaatatgctgatttgtttttggcagctaagaatttatcagatgctattttactttcagatatcctaagagtaaatactgaaataactaaggctcccctatcagcttcaatgattaaacgctacgatgaacatcatcaagacttgactcttttaaaagctttagttcgacaacaacttccagaaaagtataaagaaatcttttttgatcaatcaaaaaacggatatgcaggttatattgatgggggagctagccaagaagaattttataaatttatcaaaccaattttagaaaaaatggatggtactgaggaattattggtgaaactaaatcgtgaagatttgctgcgcaagcaacggacctttgacaacggctctattccccatcaaattcacttgggtgagctgcatgctattttgagaagacaagaagacttttatccatttttaaaagacaatcgtgagaagattgaaaaaatcttgacttttcgaattccttattatgttggtccattggcgcgtggcaatagtcgttttgcatggatgactcggaagtctgaagaaacaattaccccatggaattttgaagaagttgtcgataaaggtgcttcagctcaatcatttattgaacgcatgacaaactttgataaaaatcttccaaatgaaaaagtactaccaaaacatagtttgctttatgagtattttacggtttataacgaattgacaaaggtcaaatatgttactgaaggaatgcgaaaaccagcatttctttcaggtgaacagaagaaagccattgttgatttactcttcaaaacaaatcgaaaagtaaccgttaagcaattaaaagaagattatttcaaaaaaatagaatgttttgatagtgttgaaatttcaggagttgaagatagatttaatgcttcattaggtacctaccatgatttgctaaaaattattaaagataaagattttttggataatgaagaaaatgaagatatcttagaggatattgttttaacattgaccttatttgaagatagggagatgattgaggaaagacttaaaacatatgctcacctctttgatgataaggtgatgaaacagcttaaacgtcgccgttatactggttggggacgtttgtctcgaaaattgattaatggtattagggataagcaatctggcaaaacaatattagattttttgaaatcagatggttttgccaatcgcaattttatgcagctgatccatgatgatagtttgacatttaaagaagacattcaaaaagcacaagtgtctggacaaggcgatagtttacatgaacatattgcaaatttagctggtagccctgctattaaaaaaggtattttacagactgtaaaagttgttgatgaattggtcaaagtaatggggcggcataagccagaaaatatcgttattgaaatggcacgtgaaaatcagacaactcaaaagggccagaaaaattcgcgagagcgtatgaaacgaatcgaagaaggtatcaaagaattaggaagtcagattcttaaagagcatcctgttgaaaatactcaattgcaaaatgaaaagctctatctctattatctccaaaatggaagagacatgtatgtggaccaagaattagatattaatcgtttaagtgattatgatgtcgatcacattgttccacaaagtttccttaaagacgattcaatagacaataaggtcttaacgcgttctgataaaaatcgtggtaaatcggataacgttccaagtgaagaagtagtcaaaaagatgaaaaactattggagacaacttctaaacgccaagttaatcactcaacgtaagtttgataatttaacgaaagctgaacgtggaggtttgagtgaacttgataaagctggttttatcaaacgccaattggttgaaactcgccaaatcactaagcatgtggcacaaattttggatagtcgcatgaatactaaatacgatgaaaatgataaacttattcgagaggttaaagtgattaccttaaaatctaaattagtttctgacttccgaaaagatttccaattctataaagtacgtgagattaacaattaccatcatgcccatgatgcgtatctaaatgccgtcgttggaactgctttgattaagaaatatccaaaacttgaatcggagtttgtctatggtgattataaagtttatgatgttcgtaaaatgattgctaagtctgagcaagaaataggcaaagcaaccgcaaaatatttcttttactctaatatcatgaacttcttcaaaacagaaattacacttgcaaatggagagattcgcaaacgccctctaatcgaaactaatggggaaactggagaaattgtctgggataaagggcgagattttgccacagtgcgcaaagtattgtccatgccccaagtcaatattgtcaagaaaacagaagtacagacaggcggattctccaaggagtcaattttaccaaaaagaaattcggacaagcttattgctcgtaaaaaagactgggatccaaaaaaatatggtggttttgatagtccaacggtagcttattcagtcctagtggttgctaaggtggaaaaagggaaatcgaagaagttaaaatccgttaaagagttactagggatcacaattatggaaagaagttcctttgaaaaaaatccgattgactttttagaagctaaaggatataaggaagttaaaaaagacttaatcattaaactacctaaatatagtctttttgagttagaaaacggtcgtaaacggatgctggctagtgccggagaattacaaaaaggaaatgagctggctctgccaagcaaatatgtgaattttttatatttagctagtcattatgaaaagttgaagggtagtccagaagataacgaacaaaaacaattgtttgtggagcagcataagcattatttagatgagattattgagcaaatcagtgaattttctaagcgtgttattttagcagatgccaatttagataaagttcttagtgcatataacaaacatagagacaaaccaatacgtgaacaagcagaaaatattattcatttatttacgttgacgaatcttggagctcccgctgcttttaaatattttgatacaacaattgatcgtaaacgatatacgtctacaaaagaagttttagatgccactcttatccatcaatccatcactggtctttatgaaacacgcattgatttgagtcagctaggaggtgaccccaagaagaagaggaaggtgatggataagcatcaccaccaccatcac

SEQ ID NO: 272 - protein, 1382 aa, synthetic construct
  REGION 1..1382: note = Synthetic Polypeptide
MPKKKRKVMDKKYSIGLAIGTNSVGWAVITDEYKVPSKKFKVLGNTDRHSIKKNLIGALLFDSGETAEATRLKRTARRRYTRRKNRICYLQEIFSNEMAKVDDSFFHRLEESFLVEEDKKHERHPIFGNIVDEVAYHEKYPTIYHLRKKLVDSTDKADLRLIYLALAHMIKFRGHFLIEGDLNPDNSDVDKLFIQLVQTYNQLFEENPINASGVDAKAILSARLSKSRRLENLIAQLPGEKKNGLFGNLIALSLGLTPNFKSNFDLAEDAKLQLSKDTYDDDLDNLLAQIGDQYADLFLAAKNLSDAILLSDILRVNTEITKAPLSASMIKRYDEHHQDLTLLKALVRQQLPEKYKEIFFDQSKNGYAGYIDGGASQEEFYKFIKPILEKMDGTEELLVKLNREDLLRKQRTFDNGSIPHQIHLGELHAILRRQEDFYPFLKDNREKIEKILTFRIPYYVGPLARGNSRFAWMTRKSEETITPWNFEEVVDKGASAQSFIERMTNFDKNLPNEKVLPKHSLLYEYFTVYNELTKVKYVTEGMRKPAFLSGEQKKAIVDLLFKTNRKVTVKQLKEDYFKKIECFDSVEISGVEDRFNASLGTYHDLLKIIKDKDFLDNEENEDILEDIVLTLTLFEDREMIEERLKTYAHLFDDKVMKQLKRRRYTGWGRLSRKLINGIRDKQSGKTILDFLKSDGFANRNFMQLIHDDSLTFKEDIQKAQVSGQGDSLHEHIANLAGSPAIKKGILQTVKVVDELVKVMGRHKPENIVIEMARENQTTQKGQKNSRERMKRIEEGIKELGSQILKEHPVENTQLQNEKLYLYYLQNGRDMYVDQELDINRLSDYDVDHIVPQSFLKDDSIDNKVLTRSDKNRGKSDNVPSEEVVKKMKNYWRQLLNAKLITQRKFDNLTKAERGGLSELDKAGFIKRQLVETRQITKHVAQILDSRMNTKYDENDKLIREVKVITLKSKLVSDFRKDFQFYKVREINNYHHAHDAYLNAVVGTALIKKYPKLESEFVYGDYKVYDVRKMIAKSEQEIGKATAKYFFYSNIMNFFKTEITLANGEIRKRPLIETNGETGEIVWDKGRDFATVRKVLSMPQVNIVKKTEVQTGGFSKESILPKRNSDKLIARKKDWDPKKYGGFDSPTVAYSVLVVAKVEKGKSKKLKSVKELLGITIMERSSFEKNPIDFLEAKGYKEVKKDLIIKLPKYSLFELENGRKRMLASAGELQKGNELALPSKYVNFLYLASHYEKLKGSPEDNEQKQLFVEQHKHYLDEIIEQISEFSKRVILADANLDKVLSAYNKHRDKPIREQAENIIHLFTLTNLGAPAAFKYFDTTIDRKRYTSTKEVLDATLIHQSITGLYETRIDLSQLGGDHHHHHH

SEQ ID NO: 273 - DNA, 53 bp, synthetic construct
  misc_feature 1..53: note = Synthetic Polynucleotide
  source 1..53: mol_type = other DNA
taatacgactcactataggggccactagggacaggatgaaaggacgaaacacc

SEQ ID NO: 274 - DNA, 200 bp, synthetic construct
  misc_feature 1..200: note = Synthetic Polynucleotide
  source 1..200: mol_type = other DNA
cgaccacatgaagcagcacgacttcttcaagtccgccatgcccgaaggctacgtccaggagcgcaccatcttcttcaaggacgacggcaactacaagacccgcgccgaggtgaagttcgagggcgacaccctggtgaaccgcatcgagctgaagggcatcgacttcaaggaggacggcaacatcctggggcacaagctgg

SEQ ID NO: 275 - protein, 248 aa, synthetic construct
  REGION 1..248: note = Synthetic Polypeptide
MGHHHHHHGGASKGEELFTGVVPILVELDGDVNGHKFSVRGEGEGDATNGKLTLKFICTTGKLPVPWPTLVTTLTYGVQCFSRYPDHMKQHDFFKSAMPEGYVQERTISFKDDGTYKTRAEVKFEGDTLVNRIELKGIDFKEDGNILGHKLEYNFNSHNVYITADKQKNGIKANFKIRHNVEDGSVQLADHYQQNTPIGDGPVLLPDNHYLSTQSALSKDPNEKRDHMVLLEFVTAAGITHGMDELYK

SEQ ID NO: 276 - protein, 248 aa, synthetic construct
  REGION 1..248: note = Synthetic Polypeptide
MGHHHHHHGGASKGEELFTGVVPILVELDGDVNGHEFSVRGEGEGDATEGELTLKFICTTGELPVPWPTLVTTLTYGVQCFSRYPDHMKQHDFFKSAMPEGYVQERTISFKDDGTYKTRAEVKFEGDTLVNRIELKGIDFKEDGNILGHKLEYNFNSHDVYITADKQENGIKAEFEIRHNVEDGSVQLADHYQQNTPIGDGPVLLPDDHYLSTESALSKDPNEDRDHMVLLEFVTAAGIDHGMDELYK

SEQ ID NO: 277 - protein, 248 aa, synthetic construct
  REGION 1..248: note = Synthetic Polypeptide
MGHHHHHHGGASKGEELFDGEVPILVELDGDVNGHEFSVRGEGEGDATEGELTLKFICTTGELPVPWPTLVTTLTYGVQCFSRYPDHMDQHDFFKSAMPEGYVQERTISFKDDGTYKTRAEVKFEGDTLVNRIELKGIDFKEDGNILGHKLEYNFNSHDVYITADKQENGIKAEFEIRHNVEDGSVQLADHYQQNTPIGDGPVLLPDDHYLSTESALSKDPNEDRDHMVLLEFVTAAGIDHGMDELYK

SEQ ID NO: 278 - protein, 128 aa, synthetic construct
  REGION 1..128: note = Synthetic Polypeptide
AAEAGITGTWYNQLGSTFIVTAGADGALTGTYESAVGNAESRYVLTGRYDSAPATDGSGTALGWTVAWKNNYRNAHSATTWSGQYVGGAEARINTQWLLTSGTTEANAWKSTLVGHDTFTKVKPSAAS

SEQ ID NO: 279 - protein, 137 aa, synthetic construct
  REGION 1..137: note = Synthetic Polypeptide
MGHHHHHHGGAEAGITGTWYNQLGSTFIVTAGADGALTGTYESAVGDAESEYVLTGRYDSAPATDGSGTALGWTVAWKNDYENAHSATTWSGQYVGGAEARINTQWLLTSGTTEADAWKSTLVGHDTFTKVEPSAAS

SEQ ID NO: 280 - protein, 137 aa, synthetic construct
  REGION 1..137: note = Synthetic Polypeptide
MGHHHHHHGGAKAGITGTWYNQLGSTFIVTAGAKGALTGTYESAVGNAKSRYVLTGRYDSAPATKGSGTALGWTVAWKNKYRNAHSALTWSGQYVGGAKARINTQWLLTSGTTKAKAWKSTLVGHDTFTKVKPSAAS